European Patent Specification EP 4 229 221 B1, published March 4, 2026. Title: Method for parallel nucleic acid analysis. Applicant: IMBA - INSTITUT FÜR MOLEKULARE BIOTECHNOLOGIE GMBH. The sequence listing filed with the application follows.

SEQUENCE LISTING (1046 sequences)

SEQ ID NO: 1 - DNA, 51 bp, Artificial Sequence
  primer
  misc_feature 23: n is a, c, g, or t
ctacacgacgctcttccgatctnccaatactgaccccaaaatcagcgaaat

SEQ ID NO: 2 - DNA, 52 bp, Artificial Sequence
  primer
  misc_feature (23)..(24): n is a, c, g, or t
ctacacgacgctcttccgatctnntcgcgcatgaccccaaaatcagcgaaat

SEQ ID NO: 3 - DNA, 53 bp, Artificial Sequence
  primer
  misc_feature (23)..(25): n is a, c, g, or t
ctacacgacgctcttccgatctnnngtgtgaacgaccccaaaatcagcgaaat

SEQ ID NO: 4 - DNA, 54 bp, Artificial Sequence
  primer
  misc_feature (23)..(26): n is a, c, g, or t
ctacacgacgctcttccgatctnnnnggtggcacgaccccaaaatcagcgaaat

SEQ ID NO: 5 - DNA, 51 bp, Artificial Sequence
  primer
  misc_feature 23: n is a, c, g, or t
ctacacgacgctcttccgatctntaggtgctgaccccaaaatcagcgaaat

SEQ ID NO: 6 - DNA, 52 bp, Artificial Sequence
  primer
  misc_feature (23)..(24): n is a, c, g, or t
ctacacgacgctcttccgatctnngagcggttgaccccaaaatcagcgaaat

SEQ ID NO: 7 - DNA, 53 bp, Artificial Sequence
  primer
  misc_feature (23)..(25): n is a, c, g, or t
ctacacgacgctcttccgatctnnnaggattaggaccccaaaatcagcgaaat

SEQ ID NO: 8 - DNA, 54 bp, Artificial Sequence
  primer
  misc_feature (23)..(26): n is a, c, g, or t
ctacacgacgctcttccgatctnnnngtgagccagaccccaaaatcagcgaaat

SEQ ID NO: 9 - DNA, 51 bp, Artificial Sequence
  primer
  misc_feature 23: n is a, c, g, or t
ctacacgacgctcttccgatctnaattatgcgaccccaaaatcagcgaaat

SEQ ID NO: 10 - DNA, 52 bp, Artificial Sequence
  primer
  misc_feature (23)..(24): n is a, c, g, or t
ctacacgacgctcttccgatctnnttacgccggaccccaaaatcagcgaaat

SEQ ID NO: 11 - DNA, 53 bp, Artificial Sequence
  primer
  misc_feature (23)..(25): n is a, c, g, or t
ctacacgacgctcttccgatctnnngtagtgatgaccccaaaatcagcgaaat

SEQ ID NO: 12 - DNA, 54 bp, Artificial Sequence
  primer
  misc_feature (23)..(26): n is a, c, g, or t
ctacacgacgctcttccgatctnnnntggttgcagaccccaaaatcagcgaaat

SEQ ID NO: 13 - DNA, 51 bp, Artificial Sequence
  primer
  misc_feature 23: n is a, c, g, or t
ctacacgacgctcttccgatctngtccgaccgaccccaaaatcagcgaaat

SEQ ID NO: 14 - DNA, 52 bp, Artificial Sequence
  primer
  misc_feature (23)..(24): n is a, c, g, or t
ctacacgacgctcttccgatctnngccagccggaccccaaaatcagcgaaat

SEQ ID NO: 15 - DNA, 53 bp, Artificial Sequence
  primer
  misc_feature (23)..(25): n is a, c, g, or t
ctacacgacgctcttccgatctnnnctcgtgtcgaccccaaaatcagcgaaat

SEQ ID NO: 16 - DNA, 54 bp, Artificial Sequence
  primer
  misc_feature (23)..(26): n is a, c, g, or t
ctacacgacgctcttccgatctnnnngccgtggcgaccccaaaatcagcgaaat

SEQ ID NO: 17 - DNA, 51 bp, Artificial Sequence
  primer
  misc_feature 23: n is a, c, g, or t
ctacacgacgctcttccgatctngtagccacgaccccaaaatcagcgaaat

SEQ ID NO: 18 - DNA, 52 bp, Artificial Sequence
  primer
  misc_feature (23)..(24): n is a, c, g, or t
ctacacgacgctcttccgatctnngacttatagaccccaaaatcagcgaaat

SEQ ID NO: 19 - DNA, 53 bp, Artificial Sequence
  primer
  misc_feature (23)..(25): n is a, c, g, or t
ctacacgacgctcttccgatctnnngaacgtcggaccccaaaatcagcgaaat

SEQ ID NO: 20 - DNA, 54 bp, Artificial Sequence
  primer
  misc_feature (23)..(26): n is a, c, g, or t
ctacacgacgctcttccgatctnnnnatgcgtaggaccccaaaatcagcgaaat

SEQ ID NO: 21 - DNA, 51 bp, Artificial Sequence
  primer
  misc_feature 23: n is a, c, g, or t
ctacacgacgctcttccgatctnaattagatgaccccaaaatcagcgaaat

SEQ ID NO: 22 - DNA, 52 bp, Artificial Sequence
  primer
  misc_feature (23)..(24): n is a, c, g, or t
ctacacgacgctcttccgatctnnttacgatagaccccaaaatcagcgaaat

SEQ ID NO: 23 - DNA, 53 bp, Artificial Sequence
  primer
  misc_feature (23)..(25): n is a, c, g, or t
ctacacgacgctcttccgatctnnnctgtacaagaccccaaaatcagcgaaat

SEQ ID NO: 24 - DNA, 54 bp, Artificial Sequence
  primer
  misc_feature (23)..(26): n is a, c, g, or t
ctacacgacgctcttccgatctnnnncgtggttggaccccaaaatcagcgaaat

SEQ ID NO: 25 - DNA, 51 bp, Artificial Sequence
  primer
  misc_feature 23: n is a, c, g, or t
ctacacgacgctcttccgatctnaataacgtgaccccaaaatcagcgaaat

SEQ ID NO: 26 - DNA, 52 bp, Artificial Sequence
  primer
  misc_feature (23)..(24): n is a, c, g, or t
ctacacgacgctcttccgatctnnttcttgaagaccccaaaatcagcgaaat

SEQ ID NO: 27 - DNA, 53 bp, Artificial Sequence
  primer
  misc_feature (23)..(25): n is a, c, g, or t
ctacacgacgctcttccgatctnnnggcagatcgaccccaaaatcagcgaaat

SEQ ID NO: 28 - DNA, 54 bp, Artificial Sequence
  primer
  misc_feature (23)..(26): n is a, c, g, or t
ctacacgacgctcttccgatctnnnnctatgttagaccccaaaatcagcgaaat

SEQ ID NO: 29 - DNA, 51 bp, Artificial Sequence
  primer
  misc_feature 23: n is a, c, g, or t
ctacacgacgctcttccgatctngttgacgcgaccccaaaatcagcgaaat

SEQ ID NO: 30 - DNA, 52 bp, Artificial Sequence
  primer
  misc_feature (23)..(24): n is a, c, g, or t
ctacacgacgctcttccgatctnnatctacgagaccccaaaatcagcgaaat

SEQ ID NO: 31 - DNA, 53 bp, Artificial Sequence
  primer
  misc_feature (23)..(25): n is a, c, g, or t
ctacacgacgctcttccgatctnnnctcgacaggaccccaaaatcagcgaaat

SEQ ID NO: 32 - DNA, 54 bp, Artificial Sequence
  primer
  misc_feature (23)..(26): n is a, c, g, or t
ctacacgacgctcttccgatctnnnngaggctgcgaccccaaaatcagcgaaat

SEQ ID NO: 33 - DNA, 51 bp, Artificial Sequence
  primer
  misc_feature 23: n is a, c, g, or t
ctacacgacgctcttccgatctncctcgtaggaccccaaaatcagcgaaat

SEQ ID NO: 34 - DNA, 52 bp, Artificial Sequence
  primer
  misc_feature (23)..(24): n is a, c, g, or t
ctacacgacgctcttccgatctnncataggcagaccccaaaatcagcgaaat

SEQ ID NO: 35 - DNA, 53 bp, Artificial Sequence
  primer
  misc_feature (23)..(25): n is a, c, g, or t
ctacacgacgctcttccgatctnnnagatgaacgaccccaaaatcagcgaaat

SEQ ID NO: 36 - DNA, 54 bp, Artificial Sequence
  primer
  misc_feature (23)..(26): n is a, c, g, or t
ctacacgacgctcttccgatctnnnnccgagtatgaccccaaaatcagcgaaat

SEQ ID NO: 37 - DNA, 51 bp, Artificial Sequence
  primer
  misc_feature 23: n is a, c, g, or t
ctacacgacgctcttccgatctnaatattgagaccccaaaatcagcgaaat

SEQ ID NO: 38 - DNA, 52 bp, Artificial Sequence
  primer
  misc_feature (23)..(24): n is a, c, g, or t
ctacacgacgctcttccgatctnngtataccggaccccaaaatcagcgaaat

SEQ ID NO: 39 - DNA, 53 bp, Artificial Sequence
  primer
  misc_feature (23)..(25): n is a, c, g, or t
ctacacgacgctcttccgatctnnngatccaacgaccccaaaatcagcgaaat

SEQ ID NO: 40 - DNA, 54 bp, Artificial Sequence
  primer
  misc_feature (23)..(26): n is a, c, g, or t
ctacacgacgctcttccgatctnnnnagatacgcgaccccaaaatcagcgaaat

SEQ ID NO: 41 - DNA, 51 bp, Artificial Sequence
  primer
  misc_feature 23: n is a, c, g, or t
ctacacgacgctcttccgatctnggtatcttgaccccaaaatcagcgaaat

SEQ ID NO: 42 - DNA, 52 bp, Artificial Sequence
  primer
  misc_feature (23)..(24): n is a, c, g, or t
ctacacgacgctcttccgatctnncctctggcgaccccaaaatcagcgaaat

SEQ ID NO: 43 - DNA, 51 bp, Artificial Sequence
  primer
  misc_feature 23: n is a, c, g, or t
ctacacgacgctcttccgatctnccattgtggaccccaaaatcagcgaaat

SEQ ID NO: 44 - DNA, 52 bp, Artificial Sequence
  primer
  misc_feature (23)..(24): n is a, c, g, or t
ctacacgacgctcttccgatctnnactacggtgaccccaaaatcagcgaaat

SEQ ID NO: 45 - DNA, 53 bp, Artificial Sequence
  primer
  misc_feature (23)..(25): n is a, c, g, or t
ctacacgacgctcttccgatctnnnaagtgctagaccccaaaatcagcgaaat

SEQ ID NO: 46 - DNA, 54 bp, Artificial Sequence
  primer
  misc_feature (23)..(26): n is a, c, g, or t
ctacacgacgctcttccgatctnnnngccgaacggaccccaaaatcagcgaaat

SEQ ID NO: 47 - DNA, 51 bp, Artificial Sequence
  primer
  misc_feature 23: n is a, c, g, or t
ctacacgacgctcttccgatctntgtccacggaccccaaaatcagcgaaat

SEQ ID NO: 48 - DNA, 52 bp, Artificial Sequence
  primer
  misc_feature (23)..(24): n is a, c, g, or t
ctacacgacgctcttccgatctnngacacactgaccccaaaatcagcgaaat

SEQ ID NO: 49 - DNA, 53 bp, Artificial Sequence
  primer
  misc_feature (23)..(25): n is a, c, g, or t
ctacacgacgctcttccgatctnnnaatatgctgaccccaaaatcagcgaaat

SEQ ID NO: 50 - DNA, 54 bp, Artificial Sequence
  primer
  misc_feature (23)..(26): n is a, c, g, or t
ctacacgacgctcttccgatctnnnnttctcatagaccccaaaatcagcgaaat

SEQ ID NO: 51 - DNA, 51 bp, Artificial Sequence
  primer
  misc_feature 23: n is a, c, g, or t
ctacacgacgctcttccgatctntctgtgatgaccccaaaatcagcgaaat

SEQ ID NO: 52 - DNA, 52 bp, Artificial Sequence
  primer
  misc_feature (23)..(24): n is a, c, g, or t
ctacacgacgctcttccgatctnnccgaacttgaccccaaaatcagcgaaat

SEQ ID NO: 53 - DNA, 53 bp, Artificial Sequence
  primer
  misc_feature (23)..(25): n is a, c, g, or t
ctacacgacgctcttccgatctnnngtctaacagaccccaaaatcagcgaaat

SEQ ID NO: 54 - DNA, 54 bp, Artificial Sequence
  primer
  misc_feature (23)..(26): n is a, c, g, or t
ctacacgacgctcttccgatctnnnngacgccatgaccccaaaatcagcgaaat

SEQ ID NO: 55 - DNA, 51 bp, Artificial Sequence
  primer
  misc_feature 23: n is a, c, g, or t
ctacacgacgctcttccgatctngccaatgtgaccccaaaatcagcgaaat

SEQ ID NO: 56 - DNA, 52 bp, Artificial Sequence
  primer
  misc_feature (23)..(24): n is a, c, g, or t
ctacacgacgctcttccgatctnnccaacgtcgaccccaaaatcagcgaaat

SEQ ID NO: 57 - DNA, 53 bp, Artificial Sequence
  primer
  misc_feature (23)..(25): n is a, c, g, or t
ctacacgacgctcttccgatctnnngtagataagaccccaaaatcagcgaaat

SEQ ID NO: 58 - DNA, 54 bp, Artificial Sequence
  primer
  misc_feature (23)..(26): n is a, c, g, or t
ctacacgacgctcttccgatctnnnncttacggcgaccccaaaatcagcgaaat

SEQ ID NO: 59 - DNA, 51 bp, Artificial Sequence
  primer
  misc_feature 23: n is a, c, g, or t
ctacacgacgctcttccgatctnccaagtgcgaccccaaaatcagcgaaat

SEQ ID NO: 60 - DNA, 52 bp, Artificial Sequence
  primer
  misc_feature (23)..(24): n is a, c, g, or t
ctacacgacgctcttccgatctnnctaactcagaccccaaaatcagcgaaat

SEQ ID NO: 61 - DNA, 53 bp, Artificial Sequence
  primer
  misc_feature (23)..(25): n is a, c, g, or t
ctacacgacgctcttccgatctnnnaatatctggaccccaaaatcagcgaaat

SEQ ID NO: 62 - DNA, 54 bp, Artificial Sequence
  primer
  misc_feature (23)..(26): n is a, c, g, or t
ctacacgacgctcttccgatctnnnnttatatcagaccccaaaatcagcgaaat

SEQ ID NO: 63 - DNA, 51 bp, Artificial Sequence
  primer
  misc_feature 23: n is a, c, g, or t
ctacacgacgctcttccgatctnctgcggatgaccccaaaatcagcgaaat

SEQ ID NO: 64 - DNA, 52 bp, Artificial Sequence
  primer
  misc_feature (23)..(24): n is a, c, g, or t
ctacacgacgctcttccgatctnngcggcttggaccccaaaatcagcgaaat

SEQ ID NO: 65 - DNA, 53 bp, Artificial Sequence
  primer
  misc_feature (23)..(25): n is a, c, g, or t
ctacacgacgctcttccgatctnnngagttgatgaccccaaaatcagcgaaat

SEQ ID NO: 66 - DNA, 54 bp, Artificial Sequence
  primer
  misc_feature (23)..(26): n is a, c, g, or t
ctacacgacgctcttccgatctnnnngcactgaggaccccaaaatcagcgaaat

SEQ ID NO: 67 - DNA, 51 bp, Artificial Sequence
  primer
  misc_feature 23: n is a, c, g, or t
ctacacgacgctcttccgatctngaccacctgaccccaaaatcagcgaaat

SEQ ID NO: 68 - DNA, 51 bp, Artificial Sequence
  primer
  misc_feature 23: n is a, c, g, or t
ctacacgacgctcttccgatctnaatagcaagaccccaaaatcagcgaaat

SEQ ID NO: 69 - DNA, 51 bp, Artificial Sequence
  primer
  misc_feature 23: n is a, c, g, or t
ctacacgacgctcttccgatctncctaccgggaccccaaaatcagcgaaat

SEQ ID NO: 70 - DNA, 52 bp, Artificial Sequence
  primer
  misc_feature (23)..(24): n is a, c, g, or t
ctacacgacgctcttccgatctnnggaggatggaccccaaaatcagcgaaat

SEQ ID NO: 71 - DNA, 53 bp, Artificial Sequence
  primer
  misc_feature (23)..(25): n is a, c, g, or t
ctacacgacgctcttccgatctnnncgctgaatgaccccaaaatcagcgaaat

SEQ ID NO: 72 - DNA, 54 bp, Artificial Sequence
  primer
  misc_feature (23)..(26): n is a, c, g, or t
ctacacgacgctcttccgatctnnnntgtgacgagaccccaaaatcagcgaaat

SEQ ID NO: 73 - DNA, 51 bp, Artificial Sequence
  primer
  misc_feature 23: n is a, c, g, or t
ctacacgacgctcttccgatctnaatagattgaccccaaaatcagcgaaat

SEQ ID NO: 74 - DNA, 52 bp, Artificial Sequence
  primer
  misc_feature (23)..(24): n is a, c, g, or t
ctacacgacgctcttccgatctnnttagcgcagaccccaaaatcagcgaaat

SEQ ID NO: 75 - DNA, 53 bp, Artificial Sequence
  primer
  misc_feature (23)..(25): n is a, c, g, or t
ctacacgacgctcttccgatctnnngcggccgtgaccccaaaatcagcgaaat

SEQ ID NO: 76 - DNA, 54 bp, Artificial Sequence
  primer
  misc_feature (23)..(26): n is a, c, g, or t
ctacacgacgctcttccgatctnnnncagtaaccgaccccaaaatcagcgaaat

SEQ ID NO: 77 - DNA, 51 bp, Artificial Sequence
  primer
  misc_feature 23: n is a, c, g, or t
ctacacgacgctcttccgatctngcctagtagaccccaaaatcagcgaaat

SEQ ID NO: 78 - DNA, 52 bp, Artificial Sequence
  primer
  misc_feature (23)..(24): n is a, c, g, or t
ctacacgacgctcttccgatctnncacggcgcgaccccaaaatcagcgaaat

SEQ ID NO: 79 - DNA, 53 bp, Artificial Sequence
  primer
  misc_feature (23)..(25): n is a, c, g, or t
ctacacgacgctcttccgatctnnnggtgcagagaccccaaaatcagcgaaat

SEQ ID NO: 80 - DNA, 54 bp, Artificial Sequence
  primer
  misc_feature (23)..(26): n is a, c, g, or t
ctacacgacgctcttccgatctnnnntcgctgacgaccccaaaatcagcgaaat

SEQ ID NO: 81 - DNA, 51 bp, Artificial Sequence
  primer
  misc_feature 23: n is a, c, g, or t
ctacacgacgctcttccgatctncagccagtgaccccaaaatcagcgaaat

SEQ ID NO: 82 - DNA, 52 bp, Artificial Sequence
  primer
  misc_feature (23)..(24): n is a, c, g, or t
ctacacgacgctcttccgatctnncgtcaaccgaccccaaaatcagcgaaat

SEQ ID NO: 83 - DNA, 51 bp, Artificial Sequence
  primer
  misc_feature 23: n is a, c, g, or t
ctacacgacgctcttccgatctngccggcgagaccccaaaatcagcgaaat

SEQ ID NO: 84 - DNA, 52 bp, Artificial Sequence
  primer
  misc_feature (23)..(24): n is a, c, g, or t
ctacacgacgctcttccgatctnngcctccgggaccccaaaatcagcgaaat

SEQ ID NO: 85 - DNA, 53 bp, Artificial Sequence
  primer
  misc_feature (23)..(25): n is a, c, g, or t
ctacacgacgctcttccgatctnnnaatagtccgaccccaaaatcagcgaaat

SEQ ID NO: 86 - DNA, 54 bp, Artificial Sequence
  primer
  misc_feature (23)..(26): n is a, c, g, or t
ctacacgacgctcttccgatctnnnnttagacgtgaccccaaaatcagcgaaat

SEQ ID NO: 87 - DNA, 51 bp, Artificial Sequence
  primer
  misc_feature 23: n is a, c, g, or t
ctacacgacgctcttccgatctngtggactagaccccaaaatcagcgaaat

SEQ ID NO: 88 - DNA, 52 bp, Artificial Sequence
  primer
  misc_feature (23)..(24): n is a, c, g, or t
ctacacgacgctcttccgatctnncacggacggaccccaaaatcagcgaaat

SEQ ID NO: 89 - DNA, 53 bp, Artificial Sequence
  primer
  misc_feature (23)..(25): n is a, c, g, or t
ctacacgacgctcttccgatctnnncactagaggaccccaaaatcagcgaaat

SEQ ID NO: 90 - DNA, 54 bp, Artificial Sequence
  primer
  misc_feature (23)..(26): n is a, c, g, or t
ctacacgacgctcttccgatctnnnngcagatgggaccccaaaatcagcgaaat

SEQ ID NO: 91 - DNA, 51 bp, Artificial Sequence
  primer
  misc_feature 23: n is a, c, g, or t
ctacacgacgctcttccgatctnctctcacggaccccaaaatcagcgaaat

SEQ ID NO: 92 - DNA, 52 bp, Artificial Sequence
  primer
  misc_feature (23)..(24): n is a, c, g, or t
ctacacgacgctcttccgatctnnggaatcacgaccccaaaatcagcgaaat

SEQ ID NO: 93 - DNA, 53 bp, Artificial Sequence
  primer
  misc_feature (23)..(25): n is a, c, g, or t
ctacacgacgctcttccgatctnnncgttgacggaccccaaaatcagcgaaat

SEQ ID NO: 94 - DNA, 54 bp, Artificial Sequence
  primer
  misc_feature (23)..(26): n is a, c, g, or t
ctacacgacgctcttccgatctnnnncatcaggtgaccccaaaatcagcgaaat

SEQ ID NO: 95 - DNA, 51 bp, Artificial Sequence
  primer
  misc_feature 23: n is a, c, g, or t
ctacacgacgctcttccgatctncgttgtaagaccccaaaatcagcgaaat

SEQ ID NO: 96 - DNA, 52 bp, Artificial Sequence
  primer
  misc_feature (23)..(24): n is a, c, g, or t
ctacacgacgctcttccgatctnnggcacggtgaccccaaaatcagcgaaat

SEQ ID NO: 97 - DNA, 53 bp, Artificial Sequence
  primer
  misc_feature 23: n is a, c, g, or t
ctacacgacgctcttccgatctnccaatactgggagccttgaatacaccaaaa

SEQ ID NO: 98 - DNA, 54 bp, Artificial Sequence
  primer
  misc_feature (23)..(24): n is a, c, g, or t
ctacacgacgctcttccgatctnntcgcgcatgggagccttgaatacaccaaaa

SEQ ID NO: 99 - DNA, 55 bp, Artificial Sequence
  primer
  misc_feature (23)..(25): n is a, c, g, or t
ctacacgacgctcttccgatctnnngtgtgaacgggagccttgaatacaccaaaa

SEQ ID NO: 100 - DNA, 56 bp, Artificial Sequence
  primer
  misc_feature (23)..(26): n is a, c, g, or t
ctacacgacgctcttccgatctnnnnggtggcacgggagccttgaatacaccaaaa

SEQ ID NO: 101 - DNA, 53 bp, Artificial Sequence
  primer
  misc_feature 23: n is a, c, g, or t
ctacacgacgctcttccgatctntaggtgctgggagccttgaatacaccaaaa

SEQ ID NO: 102 - DNA, 54 bp, Artificial Sequence
  primer
  misc_feature (23)..(24): n is a, c, g, or t
ctacacgacgctcttccgatctnngagcggttgggagccttgaatacaccaaaa

SEQ ID NO: 103 - DNA, 55 bp, Artificial Sequence
  primer
  misc_feature (23)..(25): n is a, c, g, or t
ctacacgacgctcttccgatctnnnaggattaggggagccttgaatacaccaaaa

SEQ ID NO: 104 - DNA, 56 bp, Artificial Sequence
  primer
  misc_feature (23)..(26): n is a, c, g, or t
ctacacgacgctcttccgatctnnnngtgagccagggagccttgaatacaccaaaa

SEQ ID NO: 105 - DNA, 53 bp, Artificial Sequence
  primer
  misc_feature 23: n is a, c, g, or t
ctacacgacgctcttccgatctnaattatgcgggagccttgaatacaccaaaa

SEQ ID NO: 106 - DNA, 54 bp, Artificial Sequence
  primer
  misc_feature (23)..(24): n is a, c, g, or t
ctacacgacgctcttccgatctnnttacgccggggagccttgaatacaccaaaa

SEQ ID NO: 107 - DNA, 55 bp, Artificial Sequence
  primer
  misc_feature (23)..(25): n is a, c, g, or t
ctacacgacgctcttccgatctnnngtagtgatgggagccttgaatacaccaaaa

SEQ ID NO: 108 - DNA, 56 bp, Artificial Sequence
  primer
  misc_feature (23)..(26): n is a, c, g, or t
ctacacgacgctcttccgatctnnnntggttgcagggagccttgaatacaccaaaa

SEQ ID NO: 109 - DNA, 53 bp, Artificial Sequence
  primer
  misc_feature 23: n is a, c, g, or t
ctacacgacgctcttccgatctngtccgaccgggagccttgaatacaccaaaa

SEQ ID NO: 110 - DNA, 54 bp, Artificial Sequence
  primer
  misc_feature (23)..(24): n is a, c, g, or t
ctacacgacgctcttccgatctnngccagccggggagccttgaatacaccaaaa

SEQ ID NO: 111 - DNA, 55 bp, Artificial Sequence
  primer
  misc_feature (23)..(25): n is a, c, g, or t
ctacacgacgctcttccgatctnnnctcgtgtcgggagccttgaatacaccaaaa

SEQ ID NO: 112 - DNA, 56 bp, Artificial Sequence
  primer
  misc_feature (23)..(26): n is a, c, g, or t
ctacacgacgctcttccgatctnnnngccgtggcgggagccttgaatacaccaaaa

SEQ ID NO: 113 - DNA, 53 bp, Artificial Sequence
  primer
  misc_feature 23: n is a, c, g, or t
ctacacgacgctcttccgatctngtagccacgggagccttgaatacaccaaaa

SEQ ID NO: 114 - DNA, 54 bp, Artificial Sequence
  primer
  misc_feature (23)..(24): n is a, c, g, or t
ctacacgacgctcttccgatctnngacttatagggagccttgaatacaccaaaa

SEQ ID NO: 115 - DNA, 55 bp, Artificial Sequence
  primer
  misc_feature (23)..(25): n is a, c, g, or t
ctacacgacgctcttccgatctnnngaacgtcggggagccttgaatacaccaaaa

SEQ ID NO: 116 - DNA, 56 bp, Artificial Sequence
  primer
  misc_feature (23)..(26): n is a, c, g, or t
ctacacgacgctcttccgatctnnnnatgcgtaggggagccttgaatacaccaaaa

SEQ ID NO: 117 - DNA, 53 bp, Artificial Sequence
  primer
  misc_feature 23: n is a, c, g, or t
ctacacgacgctcttccgatctnaattagatgggagccttgaatacaccaaaa

SEQ ID NO: 118 - DNA, 54 bp, Artificial Sequence
  primer
  misc_feature (23)..(24): n is a, c, g, or t
ctacacgacgctcttccgatctnnttacgatagggagccttgaatacaccaaaa

SEQ ID NO: 119 - DNA, 55 bp, Artificial Sequence
  primer
  misc_feature (23)..(25): n is a, c, g, or t
ctacacgacgctcttccgatctnnnctgtacaagggagccttgaatacaccaaaa

SEQ ID NO: 120 - DNA, 56 bp, Artificial Sequence
  primer
  misc_feature (23)..(26): n is a, c, g, or t
ctacacgacgctcttccgatctnnnncgtggttggggagccttgaatacaccaaaa

SEQ ID NO: 121 - DNA, 53 bp, Artificial Sequence
  primer
  misc_feature 23: n is a, c, g, or t
ctacacgacgctcttccgatctnaataacgtgggagccttgaatacaccaaaa

SEQ ID NO: 122 - DNA, 54 bp, Artificial Sequence
  primer
  misc_feature (23)..(24): n is a, c, g, or t
ctacacgacgctcttccgatctnnttcttgaagggagccttgaatacaccaaaa

SEQ ID NO: 123 - DNA, 55 bp, Artificial Sequence
  primer
  misc_feature (23)..(25): n is a, c, g, or t
ctacacgacgctcttccgatctnnnggcagatcgggagccttgaatacaccaaaa

SEQ ID NO: 124 - DNA, 56 bp, Artificial Sequence
  primer
  misc_feature (23)..(26): n is a, c, g, or t
ctacacgacgctcttccgatctnnnnctatgttagggagccttgaatacaccaaaa

SEQ ID NO: 125 - DNA, 53 bp, Artificial Sequence
  primer
  misc_feature 23: n is a, c, g, or t
ctacacgacgctcttccgatctngttgacgcgggagccttgaatacaccaaaa

SEQ ID NO: 126 - DNA, 54 bp, Artificial Sequence
  primer
  misc_feature (23)..(24): n is a, c, g, or t
ctacacgacgctcttccgatctnnatctacgagggagccttgaatacaccaaaa

SEQ ID NO: 127 - DNA, 55 bp, Artificial Sequence
  primer
  misc_feature (23)..(25): n is a, c, g, or t
ctacacgacgctcttccgatctnnnctcgacaggggagccttgaatacaccaaaa

SEQ ID NO: 128 - DNA, 56 bp, Artificial Sequence
  primer
  misc_feature (23)..(26): n is a, c, g, or t
ctacacgacgctcttccgatctnnnngaggctgcgggagccttgaatacaccaaaa

SEQ ID NO: 129 - DNA, 53 bp, Artificial Sequence
  primer
  misc_feature 23: n is a, c, g, or t
ctacacgacgctcttccgatctncctcgtaggggagccttgaatacaccaaaa

SEQ ID NO: 130 - DNA, 54 bp, Artificial Sequence
  primer
  misc_feature (23)..(24): n is a, c, g, or t
ctacacgacgctcttccgatctnncataggcagggagccttgaatacaccaaaa

SEQ ID NO: 131 - DNA, 55 bp, Artificial Sequence
  primer
  misc_feature (23)..(25): n is a, c, g, or t
ctacacgacgctcttccgatctnnnagatgaacgggagccttgaatacaccaaaa

SEQ ID NO: 132 - DNA, 56 bp, Artificial Sequence
  primer
  misc_feature (23)..(26): n is a, c, g, or t
ctacacgacgctcttccgatctnnnnccgagtatgggagccttgaatacaccaaaa

SEQ ID NO: 133 - DNA, 53 bp, Artificial Sequence
  primer
  misc_feature 23: n is a, c, g, or t
ctacacgacgctcttccgatctnaatattgagggagccttgaatacaccaaaa

SEQ ID NO: 134 - DNA, 54 bp, Artificial Sequence
  primer
  misc_feature (23)..(24): n is a, c, g, or t
ctacacgacgctcttccgatctnngtataccggggagccttgaatacaccaaaa

SEQ ID NO: 135 - DNA, 55 bp, Artificial Sequence
  primer
  misc_feature (23)..(25): n is a, c, g, or t
ctacacgacgctcttccgatctnnngatccaacgggagccttgaatacaccaaaa

SEQ ID NO: 136 - DNA, 56 bp, Artificial Sequence
  primer
  misc_feature (23)..(26): n is a, c, g, or t
ctacacgacgctcttccgatctnnnnagatacgcgggagccttgaatacaccaaaa

SEQ ID NO: 137 - DNA, 53 bp, Artificial Sequence
  primer
  misc_feature 23: n is a, c, g, or t
ctacacgacgctcttccgatctnggtatcttgggagccttgaatacaccaaaa

SEQ ID NO: 138 - DNA, 54 bp, Artificial Sequence
  primer
  misc_feature (23)..(24): n is a, c, g, or t
ctacacgacgctcttccgatctnncctctggcgggagccttgaatacaccaaaa

SEQ ID NO: 139 - DNA, 53 bp, Artificial Sequence
  primer
  misc_feature 23: n is a, c, g, or t
ctacacgacgctcttccgatctnccattgtggggagccttgaatacaccaaaa

SEQ ID NO: 140 - DNA, 54 bp, Artificial Sequence
  primer
  misc_feature (23)..(24): n is a, c, g, or t
ctacacgacgctcttccgatctnnactacggtgggagccttgaatacaccaaaa

SEQ ID NO: 141 - DNA, 55 bp, Artificial Sequence
  primer
  misc_feature (23)..(25): n is a, c, g, or t
ctacacgacgctcttccgatctnnnaagtgctagggagccttgaatacaccaaaa

SEQ ID NO: 142 - DNA, 56 bp, Artificial Sequence
  primer
  misc_feature (23)..(26): n is a, c, g, or t
ctacacgacgctcttccgatctnnnngccgaacggggagccttgaatacaccaaaa

SEQ ID NO: 143 - DNA, 53 bp, Artificial Sequence
  primer
  misc_feature 23: n is a, c, g, or t
ctacacgacgctcttccgatctntgtccacggggagccttgaatacaccaaaa

SEQ ID NO: 144 - DNA, 54 bp, Artificial Sequence
  primer
  misc_feature (23)..(24): n is a, c, g, or t
ctacacgacgctcttccgatctnngacacactgggagccttgaatacaccaaaa

SEQ ID NO: 145 - DNA, 55 bp, Artificial Sequence
  primer
  misc_feature (23)..(25): n is a, c, g, or t
ctacacgacgctcttccgatctnnnaatatgctgggagccttgaatacaccaaaa

SEQ ID NO: 146 - DNA, 56 bp, Artificial Sequence
  primer
  misc_feature (23)..(26): n is a, c, g, or t
ctacacgacgctcttccgatctnnnnttctcatagggagccttgaatacaccaaaa

SEQ ID NO: 147 - DNA, 53 bp, Artificial Sequence
  primer
  misc_feature 23: n is a, c, g, or t
ctacacgacgctcttccgatctntctgtgatgggagccttgaatacaccaaaa

SEQ ID NO: 148 - DNA, 54 bp, Artificial Sequence
  primer
  misc_feature (23)..(24): n is a, c, g, or t
ctacacgacgctcttccgatctnnccgaacttgggagccttgaatacaccaaaa

SEQ ID NO: 149 - DNA, 55 bp, Artificial Sequence
  primer
  misc_feature (23)..(25): n is a, c, g, or t
ctacacgacgctcttccgatctnnngtctaacagggagccttgaatacaccaaaa

SEQ ID NO: 150 - DNA, 56 bp, Artificial Sequence
  primer
  misc_feature (23)..(26): n is a, c, g, or t
ctacacgacgctcttccgatctnnnngacgccatgggagccttgaatacaccaaaa

SEQ ID NO: 151 - DNA, 53 bp, Artificial Sequence
  primer
  misc_feature 23: n is a, c, g, or t
ctacacgacgctcttccgatctngccaatgtgggagccttgaatacaccaaaa

SEQ ID NO: 152 - DNA, 54 bp, Artificial Sequence
  primer
  misc_feature (23)..(24): n is a, c, g, or t
ctacacgacgctcttccgatctnnccaacgtcgggagccttgaatacaccaaaa

SEQ ID NO: 153 - DNA, 55 bp, Artificial Sequence
  primer
  misc_feature (23)..(25): n is a, c, g, or t
ctacacgacgctcttccgatctnnngtagataagggagccttgaatacaccaaaa

SEQ ID NO: 154 - DNA, 56 bp, Artificial Sequence
  primer
  misc_feature (23)..(26): n is a, c, g, or t
ctacacgacgctcttccgatctnnnncttacggcgggagccttgaatacaccaaaa

SEQ ID NO: 155 - DNA, 53 bp, Artificial Sequence
  primer
  misc_feature 23: n is a, c, g, or t
ctacacgacgctcttccgatctnccaagtgcgggagccttgaatacaccaaaa

SEQ ID NO: 156 - DNA, 54 bp, Artificial Sequence
  primer
  misc_feature (23)..(24): n is a, c, g, or t
ctacacgacgctcttccgatctnnctaactcagggagccttgaatacaccaaaa

SEQ ID NO: 157 - DNA, 55 bp, Artificial Sequence
  primer
  misc_feature (23)..(25): n is a, c, g, or t
ctacacgacgctcttccgatctnnnaatatctggggagccttgaatacaccaaaa

SEQ ID NO: 158 - DNA, 56 bp, Artificial Sequence
  primer
  misc_feature (23)..(26): n is a, c, g, or t
ctacacgacgctcttccgatctnnnnttatatcagggagccttgaatacaccaaaa

SEQ ID NO: 159 - DNA, 53 bp, Artificial Sequence
  primer
  misc_feature 23: n is a, c, g, or t
ctacacgacgctcttccgatctnctgcggatgggagccttgaatacaccaaaa

SEQ ID NO: 160 - DNA, 54 bp, Artificial Sequence
  primer
  misc_feature (23)..(24): n is a, c, g, or t
ctacacgacgctcttccgatctnngcggcttggggagccttgaatacaccaaaa

SEQ ID NO: 161 - DNA, 55 bp, Artificial Sequence
  primer
  misc_feature (23)..(25): n is a, c, g, or t
ctacacgacgctcttccgatctnnngagttgatgggagccttgaatacaccaaaa

SEQ ID NO: 162 - DNA, 56 bp, Artificial Sequence
  primer
  misc_feature (23)..(26): n is a, c, g, or t
ctacacgacgctcttccgatctnnnngcactgaggggagccttgaatacaccaaaa

SEQ ID NO: 163 - DNA, 53 bp, Artificial Sequence
  primer
  misc_feature 23: n is a, c, g, or t
ctacacgacgctcttccgatctngaccacctgggagccttgaatacaccaaaa

SEQ ID NO: 164 - DNA, 53 bp, Artificial Sequence
  primer
  misc_feature 23: n is a, c, g, or t
ctacacgacgctcttccgatctnaatagcaagggagccttgaatacaccaaaa

SEQ ID NO: 165 - DNA, 53 bp, Artificial Sequence
  primer
  misc_feature 23: n is a, c, g, or t
ctacacgacgctcttccgatctncctaccgggggagccttgaatacaccaaaa

SEQ ID NO: 166 - DNA, 54 bp, Artificial Sequence
  primer
  misc_feature (23)..(24): n is a, c, g, or t
ctacacgacgctcttccgatctnnggaggatggggagccttgaatacaccaaaa

SEQ ID NO: 167 - DNA, 55 bp, Artificial Sequence
  primer
  misc_feature (23)..(25): n is a, c, g, or t
ctacacgacgctcttccgatctnnncgctgaatgggagccttgaatacaccaaaa

SEQ ID NO: 168 - DNA, 56 bp, Artificial Sequence
  primer
  misc_feature (23)..(26): n is a, c, g, or t
ctacacgacgctcttccgatctnnnntgtgacgagggagccttgaatacaccaaaa

SEQ ID NO: 169 - DNA, 53 bp, Artificial Sequence
  primer
  misc_feature 23: n is a, c, g, or t
ctacacgacgctcttccgatctnaatagattgggagccttgaatacaccaaaa

SEQ ID NO: 170 - DNA, 54 bp, Artificial Sequence
  primer
  misc_feature (23)..(24): n is a, c, g, or t
ctacacgacgctcttccgatctnnttagcgcagggagccttgaatacaccaaaa

SEQ ID NO: 171 - DNA, 55 bp, Artificial Sequence
  primer
  misc_feature (23)..(25): n is a, c, g, or t
ctacacgacgctcttccgatctnnngcggccgtgggagccttgaatacaccaaaa

SEQ ID NO: 172 - DNA, 56 bp, Artificial Sequence
  primer
  misc_feature (23)..(26): n is a, c, g, or t
ctacacgacgctcttccgatctnnnncagtaaccgggagccttgaatacaccaaaa

SEQ ID NO: 173 - DNA, 53 bp, Artificial Sequence
  primer
  misc_feature 23: n is a, c, g, or t
ctacacgacgctcttccgatctngcctagtagggagccttgaatacaccaaaa

SEQ ID NO: 174 - DNA, 54 bp, Artificial Sequence
  primer
  misc_feature (23)..(24): n is a, c, g, or t
ctacacgacgctcttccgatctnncacggcgcgggagccttgaatacaccaaaa

SEQ ID NO: 175 - DNA, 55 bp, Artificial Sequence
  primer
  misc_feature (23)..(25): n is a, c, g, or t
ctacacgacgctcttccgatctnnnggtgcagagggagccttgaatacaccaaaa

SEQ ID NO: 176 - DNA, 56 bp, Artificial Sequence
  primer
  misc_feature (23)..(26): n is a, c, g, or t
ctacacgacgctcttccgatctnnnntcgctgacgggagccttgaatacaccaaaa

SEQ ID NO: 177 - DNA, 53 bp, Artificial Sequence
  primer
  misc_feature 23: n is a, c, g, or t
ctacacgacgctcttccgatctncagccagtgggagccttgaatacaccaaaa

SEQ ID NO: 178 - DNA, 54 bp, Artificial Sequence
  primer
  misc_feature (23)..(24): n is a, c, g, or t
ctacacgacgctcttccgatctnncgtcaaccgggagccttgaatacaccaaaa

SEQ ID NO: 179 - DNA, 53 bp, Artificial Sequence
  primer
  misc_feature 23: n is a, c, g, or t
ctacacgacgctcttccgatctngccggcgagggagccttgaatacaccaaaa

SEQ ID NO: 180 - DNA, 54 bp, Artificial Sequence
  primer
  misc_feature (23)..(24): n is a, c, g, or t
ctacacgacgctcttccgatctnngcctccgggggagccttgaatacaccaaaa

SEQ ID NO: 181 - DNA, 55 bp, Artificial Sequence
  primer
  misc_feature (23)..(25): n is a, c, g, or t
ctacacgacgctcttccgatctnnnaatagtccgggagccttgaatacaccaaaa

SEQ ID NO: 182 - DNA, 56 bp, Artificial Sequence
  primer
  misc_feature (23)..(26): n is a, c, g, or t
ctacacgacgctcttccgatctnnnnttagacgtgggagccttgaatacaccaaaa

SEQ ID NO: 183 - DNA, 53 bp, Artificial Sequence
  primer
  misc_feature 23: n is a, c, g, or t
ctacacgacgctcttccgatctngtggactagggagccttgaatacaccaaaa

SEQ ID NO: 184 - DNA, 54 bp, Artificial Sequence
  primer
  misc_feature (23)..(24): n is a, c, g, or t
ctacacgacgctcttccgatctnncacggacggggagccttgaatacaccaaaa

SEQ ID NO: 185 - DNA, 55 bp, Artificial Sequence
  primer
  misc_feature (23)..(25): n is a, c, g, or t
ctacacgacgctcttccgatctnnncactagaggggagccttgaatacaccaaaa

SEQ ID NO: 186 - DNA, 56 bp, Artificial Sequence
  primer
  misc_feature (23)..(26): n is a, c, g, or t
ctacacgacgctcttccgatctnnnngcagatgggggagccttgaatacaccaaaa

SEQ ID NO: 187 - DNA, 53 bp, Artificial Sequence
  primer
  misc_feature 23: n is a, c, g, or t
ctacacgacgctcttccgatctnctctcacggggagccttgaatacaccaaaa

SEQ ID NO: 188 - DNA, 54 bp, Artificial Sequence
  primer
  misc_feature (23)..(24): n is a, c, g, or t
ctacacgacgctcttccgatctnnggaatcacgggagccttgaatacaccaaaa

SEQ ID NO: 189 - DNA, 55 bp, Artificial Sequence
  primer
  misc_feature (23)..(25): n is a, c, g, or t
ctacacgacgctcttccgatctnnncgttgacggggagccttgaatacaccaaaa

SEQ ID NO: 190 - DNA, 56 bp, Artificial Sequence
  primer
  misc_feature (23)..(26): n is a, c, g, or t
ctacacgacgctcttccgatctnnnncatcaggtgggagccttgaatacaccaaaa

SEQ ID NO: 191 - DNA, 53 bp, Artificial Sequence
  primer
  misc_feature 23: n is a, c, g, or t
ctacacgacgctcttccgatctncgttgtaagggagccttgaatacaccaaaa

SEQ ID NO: 192 - DNA, 54 bp, Artificial Sequence
  primer
  misc_feature (23)..(24): n is a, c, g, or t
ctacacgacgctcttccgatctnnggcacggtgggagccttgaatacaccaaaa

SEQ ID NO: 193 - DNA, 52 bp, Artificial Sequence
  primer
  misc_feature 23: n is a, c, g, or t
ctacacgacgctcttccgatctnccaatactggcattcgtattgcgccgcta

SEQ ID NO: 194 - DNA, 53 bp, Artificial Sequence
  primer
  misc_feature (23)..(24): n is a, c, g, or t
ctacacgacgctcttccgatctnntcgcgcatggcattcgtattgcgccgcta

SEQ ID NO: 195 - DNA, 54 bp, Artificial Sequence
  primer
  misc_feature (23)..(25): n is a, c, g, or t
ctacacgacgctcttccgatctnnngtgtgaacggcattcgtattgcgccgcta

SEQ ID NO: 196 - DNA, 55 bp, Artificial Sequence
  primer
  misc_feature (23)..(26): n is a, c, g, or t
ctacacgacgctcttccgatctnnnnggtggcacggcattcgtattgcgccgcta

SEQ ID NO: 197 - DNA, 52 bp, Artificial Sequence
  primer
  misc_feature 23: n is a, c, g, or t
ctacacgacgctcttccgatctntaggtgctggcattcgtattgcgccgcta

SEQ ID NO: 198 - DNA, 53 bp, Artificial Sequence
  primer
  misc_feature (23)..(24): n is a, c, g, or t
ctacacgacgctcttccgatctnngagcggttggcattcgtattgcgccgcta

SEQ ID NO: 199 - DNA, 54 bp, Artificial Sequence
  primer
  misc_feature (23)..(25): n is a, c, g, or t
ctacacgacgctcttccgatctnnnaggattagggcattcgtattgcgccgcta

SEQ ID NO: 200 - DNA, 55 bp, Artificial Sequence
  primer
  misc_feature (23)..(26): n is a, c, g, or t
ctacacgacgctcttccgatctnnnngtgagccaggcattcgtattgcgccgcta

SEQ ID NO: 201 - DNA, 52 bp, Artificial Sequence
  primer
  misc_feature 23: n is a, c, g, or t
ctacacgacgctcttccgatctnaattatgcggcattcgtattgcgccgcta

SEQ ID NO: 202 - DNA, 53 bp, Artificial Sequence
  primer
  misc_feature (23)..(24): n is a, c, g, or t
ctacacgacgctcttccgatctnnttacgccgggcattcgtattgcgccgcta

SEQ ID NO: 203 - DNA, 54 bp, Artificial Sequence
  primer
  misc_feature (23)..(25): n is a, c, g, or t
ctacacgacgctcttccgatctnnngtagtgatggcattcgtattgcgccgcta

SEQ ID NO: 204 - DNA, 55 bp, Artificial Sequence
  primer
  misc_feature (23)..(26): n is a, c, g, or t
ctacacgacgctcttccgatctnnnntggttgcaggcattcgtattgcgccgcta

SEQ ID NO: 205 - DNA, 52 bp, Artificial Sequence
  primer
  misc_feature 23: n is a, c, g, or t
ctacacgacgctcttccgatctngtccgaccggcattcgtattgcgccgcta

SEQ ID NO: 206 - DNA, 53 bp, Artificial Sequence
  primer
  misc_feature (23)..(24): n is a, c, g, or t
ctacacgacgctcttccgatctnngccagccgggcattcgtattgcgccgcta

SEQ ID NO: 207 - DNA, 54 bp, Artificial Sequence
  primer
  misc_feature (23)..(25): n is a, c, g, or t
ctacacgacgctcttccgatctnnnctcgtgtcggcattcgtattgcgccgcta

SEQ ID NO: 208 - DNA, 55 bp, Artificial Sequence
  primer
  misc_feature (23)..(26): n is a, c, g, or t
ctacacgacgctcttccgatctnnnngccgtggcggcattcgtattgcgccgcta

SEQ ID NO: 209 - DNA, 52 bp, Artificial Sequence
  primer
  misc_feature 23: n is a, c, g, or t
ctacacgacgctcttccgatctngtagccacggcattcgtattgcgccgcta

SEQ ID NO: 210 - DNA, 53 bp, Artificial Sequence
  primer
  misc_feature (23)..(24): n is a, c, g, or t
ctacacgacgctcttccgatctnngacttataggcattcgtattgcgccgcta

SEQ ID NO: 211 - DNA, 54 bp, Artificial Sequence
  primer
  misc_feature (23)..(25): n is a, c, g, or t
ctacacgacgctcttccgatctnnngaacgtcgggcattcgtattgcgccgcta

SEQ ID NO: 212 - DNA, 55 bp, Artificial Sequence
  primer
  misc_feature (23)..(26): n is a, c, g, or t
ctacacgacgctcttccgatctnnnnatgcgtagggcattcgtattgcgccgcta

SEQ ID NO: 213 - DNA, 52 bp, Artificial Sequence
  primer
  misc_feature 23: n is a, c, g, or t
ctacacgacgctcttccgatctnaattagatggcattcgtattgcgccgcta

SEQ ID NO: 214 - DNA, 53 bp, Artificial Sequence
  primer
  misc_feature (23)..(24): n is a, c, g, or t
ctacacgacgctcttccgatctnnttacgataggcattcgtattgcgccgcta

SEQ ID NO: 215 - DNA, 54 bp, Artificial Sequence
  primer
  misc_feature (23)..(25): n is a, c, g, or t
ctacacgacgctcttccgatctnnnctgtacaaggcattcgtattgcgccgcta

SEQ ID NO: 216 - DNA, 55 bp, Artificial Sequence
  primer
  misc_feature (23)..(26): n is a, c, g, or t
ctacacgacgctcttccgatctnnnncgtggttgggcattcgtattgcgccgcta

SEQ ID NO: 217 - DNA, 52 bp, Artificial Sequence
  primer
  misc_feature 23: n is a, c, g, or t
ctacacgacgctcttccgatctnaataacgtggcattcgtattgcgccgcta

SEQ ID NO: 218 - DNA, 53 bp, Artificial Sequence
  primer
  misc_feature (23)..(24): n is a, c, g, or t
ctacacgacgctcttccgatctnnttcttgaaggcattcgtattgcgccgcta

SEQ ID NO: 219 - DNA, 54 bp, Artificial Sequence
  primer
  misc_feature (23)..(25): n is a, c, g, or t
ctacacgacgctcttccgatctnnnggcagatcggcattcgtattgcgccgcta

SEQ ID NO: 220 - DNA, 55 bp, Artificial Sequence
  primer
  misc_feature (23)..(26): n is a, c, g, or t
ctacacgacgctcttccgatctnnnnctatgttaggcattcgtattgcgccgcta

SEQ ID NO: 221 - DNA, 52 bp, Artificial Sequence
  primer
  misc_feature 23: n is a, c, g, or t
ctacacgacgctcttccgatctngttgacgcggcattcgtattgcgccgcta

SEQ ID NO: 222 - DNA, 53 bp, Artificial Sequence
  primer
  misc_feature (23)..(24): n is a, c, g, or t
ctacacgacgctcttccgatctnnatctacgaggcattcgtattgcgccgcta

SEQ ID NO: 223 - DNA, 54 bp, Artificial Sequence
  primer
  misc_feature (23)..(25): n is a, c, g, or t
ctacacgacgctcttccgatctnnnctcgacagggcattcgtattgcgccgcta

SEQ ID NO: 224 - DNA, 55 bp, Artificial Sequence
  primer
  misc_feature (23)..(26): n is a, c, g, or t
ctacacgacgctcttccgatctnnnngaggctgcggcattcgtattgcgccgcta

SEQ ID NO: 225 - DNA, 52 bp, Artificial Sequence
  primer
  misc_feature 23: n is a, c, g, or t
ctacacgacgctcttccgatctncctcgtagggcattcgtattgcgccgcta

SEQ ID NO: 226 - DNA, 53 bp, Artificial Sequence
  primer
  misc_feature (23)..(24): n is a, c, g, or t
ctacacgacgctcttccgatctnncataggcaggcattcgtattgcgccgcta

SEQ ID NO: 227 - DNA, 54 bp, Artificial Sequence
  primer
  misc_feature (23)..(25): n is a, c, g, or t
ctacacgacgctcttccgatctnnnagatgaacggcattcgtattgcgccgcta

SEQ ID NO: 228 - DNA, 55 bp, Artificial Sequence
  primer
  misc_feature (23)..(26): n is a, c, g, or t
ctacacgacgctcttccgatctnnnnccgagtatggcattcgtattgcgccgcta

SEQ ID NO: 229 - DNA, 52 bp, Artificial Sequence
  primer
  misc_feature 23: n is a, c, g, or t
ctacacgacgctcttccgatctnaatattgaggcattcgtattgcgccgcta

SEQ ID NO: 230 - DNA, 53 bp, Artificial Sequence
  primer
  misc_feature (23)..(24): n is a, c, g, or t
ctacacgacgctcttccgatctnngtataccgggcattcgtattgcgccgcta

SEQ ID NO: 231 - DNA, 54 bp, Artificial Sequence
  primer
  misc_feature (23)..(25): n is a, c, g, or t
ctacacgacgctcttccgatctnnngatccaacggcattcgtattgcgccgcta

SEQ ID NO: 232 - DNA, 55 bp, Artificial Sequence
  primer
  misc_feature (23)..(26): n is a, c, g, or t
ctacacgacgctcttccgatctnnnnagatacgcggcattcgtattgcgccgcta

SEQ ID NO: 233 - DNA, 52 bp, Artificial Sequence
  primer
  misc_feature 23: n is a, c, g, or t
ctacacgacgctcttccgatctnggtatcttggcattcgtattgcgccgcta

SEQ ID NO: 234 - DNA, 53 bp, Artificial Sequence
  primer
  misc_feature (23)..(24): n is a, c, g, or t
ctacacgacgctcttccgatctnncctctggcggcattcgtattgcgccgcta

SEQ ID NO: 235 - DNA, 52 bp, Artificial Sequence
  primer
  misc_feature 23: n is a, c, g, or t
ctacacgacgctcttccgatctnccattgtgggcattcgtattgcgccgcta

SEQ ID NO: 236 - DNA, 53 bp, Artificial Sequence
  primer
  misc_feature (23)..(24): n is a, c, g, or t
ctacacgacgctcttccgatctnnactacggtggcattcgtattgcgccgcta

SEQ ID NO: 237 - DNA, 54 bp, Artificial Sequence
  primer
  misc_feature (23)..(25): n is a, c, g, or t
ctacacgacgctcttccgatctnnnaagtgctaggcattcgtattgcgccgcta

SEQ ID NO: 238 - DNA, 55 bp, Artificial Sequence
  primer
  misc_feature (23)..(26): n is a, c, g, or t
ctacacgacgctcttccgatctnnnngccgaacgggcattcgtattgcgccgcta

SEQ ID NO: 239 - DNA, 52 bp, Artificial Sequence
  primer
  misc_feature 23: n is a, c, g, or t
ctacacgacgctcttccgatctntgtccacgggcattcgtattgcgccgcta

SEQ ID NO: 240 - DNA, 53 bp, Artificial Sequence
  primer
  misc_feature (23)..(24): n is a, c, g, or t
ctacacgacgctcttccgatctnngacacactggcattcgtattgcgccgcta

SEQ ID NO: 241 - DNA, 54 bp, Artificial Sequence
  primer
  misc_feature (23)..(25): n is a, c, g, or t
ctacacgacgctcttccgatctnnnaatatgctggcattcgtattgcgccgcta

SEQ ID NO: 242 - DNA, 55 bp, Artificial Sequence
  primer
  misc_feature (23)..(26): n is a, c, g, or t
ctacacgacgctcttccgatctnnnnttctcataggcattcgtattgcgccgcta

SEQ ID NO: 243 - DNA, 52 bp, Artificial Sequence
  primer
  misc_feature 23: n is a, c, g, or t
ctacacgacgctcttccgatctntctgtgatggcattcgtattgcgccgcta

SEQ ID NO: 244 - DNA, 53 bp, Artificial Sequence
  primer
  misc_feature (23)..(24): n is a, c, g, or t
ctacacgacgctcttccgatctnnccgaacttggcattcgtattgcgccgcta

SEQ ID NO: 245 - DNA, 54 bp, Artificial Sequence
  primer
  misc_feature (23)..(25): n is a, c, g, or t
ctacacgacgctcttccgatctnnngtctaacaggcattcgtattgcgccgcta

SEQ ID NO: 246 - DNA, 55 bp, Artificial Sequence
  primer
  misc_feature (23)..(26): n is a, c, g, or t
ctacacgacgctcttccgatctnnnngacgccatggcattcgtattgcgccgcta

SEQ ID NO: 247 - DNA, 52 bp, Artificial Sequence
  primer
  misc_feature 23: n is a, c, g, or t
ctacacgacgctcttccgatctngccaatgtggcattcgtattgcgccgcta

SEQ ID NO: 248 - DNA, 53 bp, Artificial Sequence
  primer
  misc_feature (23)..(24): n is a, c, g, or t
ctacacgacgctcttccgatctnnccaacgtcggcattcgtattgcgccgcta

SEQ ID NO: 249 - DNA, 54 bp, Artificial Sequence
  primer
  misc_feature (23)..(25): n is a, c, g, or t
ctacacgacgctcttccgatctnnngtagataaggcattcgtattgcgccgcta

SEQ ID NO: 250 - DNA, 55 bp, Artificial Sequence
  primer
  misc_feature (23)..(26): n is a, c, g, or t
ctacacgacgctcttccgatctnnnncttacggcggcattcgtattgcgccgcta

SEQ ID NO: 251 - DNA, 52 bp, Artificial Sequence
  primer
  misc_feature 23: n is a, c, g, or t
ctacacgacgctcttccgatctnccaagtgcggcattcgtattgcgccgcta

SEQ ID NO: 252 - DNA, 53 bp, Artificial Sequence
  primer
  misc_feature (23)..(24): n is a, c, g, or t
ctacacgacgctcttccgatctnnctaactcaggcattcgtattgcgccgcta

SEQ ID NO: 253 - DNA, 54 bp, Artificial Sequence
  primer
  misc_feature (23)..(25): n is a, c, g, or t
ctacacgacgctcttccgatctnnnaatatctgggcattcgtattgcgccgcta

SEQ ID NO: 254 - DNA, 55 bp, Artificial Sequence
  primer
  misc_feature (23)..(26): n is a, c, g, or t
ctacacgacgctcttccgatctnnnnttatatcaggcattcgtattgcgccgcta

SEQ ID NO: 255 - DNA, 52 bp, Artificial Sequence
  primer
  misc_feature 23: n is a, c, g, or t
ctacacgacgctcttccgatctnctgcggatggcattcgtattgcgccgcta

SEQ ID NO: 256 - DNA, 53 bp, Artificial Sequence
  primer
  misc_feature (23)..(24): n is a, c, g, or t
ctacacgacgctcttccgatctnngcggcttgggcattcgtattgcgccgcta

SEQ ID NO: 257 - DNA, 54 bp, Artificial Sequence
  primer
  misc_feature (23)..(25): n is a, c, g, or t
ctacacgacgctcttccgatctnnngagttgatggcattcgtattgcgccgcta

SEQ ID NO: 258 - DNA, 55 bp, Artificial Sequence
  primer
  misc_feature (23)..(26): n is a, c, g, or t
ctacacgacgctcttccgatctnnnngcactgagggcattcgtattgcgccgcta

SEQ ID NO: 259 - DNA, 52 bp, Artificial Sequence
  primer
  misc_feature 23: n is a, c, g, or t
ctacacgacgctcttccgatctngaccacctggcattcgtattgcgccgcta

SEQ ID NO: 260 - DNA, 52 bp, Artificial Sequence
  primer
  misc_feature 23: n is a, c, g, or t
ctacacgacgctcttccgatctnaatagcaaggcattcgtattgcgccgcta

SEQ ID NO: 261 - DNA, 52 bp, Artificial Sequence
  primer
  misc_feature 23: n is a, c, g, or t
ctacacgacgctcttccgatctncctaccggggcattcgtattgcgccgcta

SEQ ID NO: 262 - DNA, 53 bp, Artificial Sequence
  primer
  misc_feature (23)..(24): n is a, c, g, or t
ctacacgacgctcttccgatctnnggaggatgggcattcgtattgcgccgcta

SEQ ID NO: 263 - DNA, 54 bp, Artificial Sequence
  primer
  misc_feature (23)..(25): n is a, c, g, or t
ctacacgacgctcttccgatctnnncgctgaatggcattcgtattgcgccgcta

SEQ ID NO: 264 - DNA, 55 bp, Artificial Sequence
  primer
  misc_feature (23)..(26): n is a, c, g, or t
ctacacgacgctcttccgatctnnnntgtgacgaggcattcgtattgcgccgcta

SEQ ID NO: 265 - DNA, 52 bp, Artificial Sequence
  primer
  misc_feature 23: n is a, c, g, or t
ctacacgacgctcttccgatctnaatagattggcattcgtattgcgccgcta

SEQ ID NO: 266 - DNA, 53 bp, Artificial Sequence
  primer
  misc_feature (23)..(24): n is a, c, g, or t
ctacacgacgctcttccgatctnnttagcgcaggcattcgtattgcgccgcta

SEQ ID NO: 267 - DNA, 54 bp, Artificial Sequence
  primer
  misc_feature (23)..(25): n is a, c, g, or t
ctacacgacgctcttccgatctnnngcggccgtggcattcgtattgcgccgcta

SEQ ID NO: 268 - DNA, 55 bp, Artificial Sequence
  primer
  misc_feature (23)..(26): n is a, c, g, or t
ctacacgacgctcttccgatctnnnncagtaaccggcattcgtattgcgccgcta

SEQ ID NO: 269 - DNA, 52 bp, Artificial Sequence
  primer
  misc_feature 23: n is a, c, g, or t
ctacacgacgctcttccgatctngcctagtaggcattcgtattgcgccgcta

SEQ ID NO: 270 - DNA, 53 bp, Artificial Sequence
  primer
  misc_feature (23)..(24): n is a, c, g, or t
ctacacgacgctcttccgatctnncacggcgcggcattcgtattgcgccgcta

SEQ ID NO: 271 - DNA, 54 bp, Artificial Sequence
  primer
  misc_feature (23)..(25): n is a, c, g, or t
ctacacgacgctcttccgatctnnnggtgcagaggcattcgtattgcgccgcta

SEQ ID NO: 272 - DNA, 55 bp, Artificial Sequence
  primer
  misc_feature (23)..(26): n is a, c, g, or t
ctacacgacgctcttccgatctnnnntcgctgacggcattcgtattgcgccgcta

SEQ ID NO: 273 - DNA, 52 bp, Artificial Sequence
  primer
  misc_feature 23: n is a, c, g, or t
ctacacgacgctcttccgatctncagccagtggcattcgtattgcgccgcta

SEQ ID NO: 274 - DNA, 53 bp, Artificial Sequence
  primer
  misc_feature (23)..(24): n is a, c, g, or t
ctacacgacgctcttccgatctnncgtcaaccggcattcgtattgcgccgcta

SEQ ID NO: 275 - DNA, 52 bp, Artificial Sequence
  primer
  misc_feature 23: n is a, c, g, or t
ctacacgacgctcttccgatctngccggcgaggcattcgtattgcgccgcta

SEQ ID NO: 276 - DNA, 53 bp, Artificial Sequence
  primer
  misc_feature (23)..(24): n is a, c, g, or t
ctacacgacgctcttccgatctnngcctccggggcattcgtattgcgccgcta

SEQ ID NO: 277 - DNA, 54 bp, Artificial Sequence
  primer
  misc_feature (23)..(25): n is a, c, g, or t
ctacacgacgctcttccgatctnnnaatagtccggcattcgtattgcgccgcta

SEQ ID NO: 278 - DNA, 55 bp, Artificial Sequence
  primer
  misc_feature (23)..(26): n is a, c, g, or t
ctacacgacgctcttccgatctnnnnttagacgtggcattcgtattgcgccgcta

SEQ ID NO: 279 - DNA, 52 bp, Artificial Sequence
  primer
  misc_feature 23: n is a, c, g, or t
ctacacgacgctcttccgatctngtggactaggcattcgtattgcgccgcta

SEQ ID NO: 280 - DNA, 53 bp, Artificial Sequence
  primer
  misc_feature (23)..(24): n is a, c, g, or t
ctacacgacgctcttccgatctnncacggacgggcattcgtattgcgccgcta

SEQ ID NO: 281 - DNA, 54 bp, Artificial Sequence
  primer
  misc_feature (23)..(25): n is a, c, g, or t
ctacacgacgctcttccgatctnnncactagagggcattcgtattgcgccgcta

SEQ ID NO: 282 - DNA, 55 bp, Artificial Sequence
  primer
  misc_feature (23)..(26): n is a, c, g, or t
ctacacgacgctcttccgatctnnnngcagatggggcattcgtattgcgccgcta

SEQ ID NO: 283 - DNA, 52 bp, Artificial Sequence
  primer
  misc_feature 23: n is a, c, g, or t
ctacacgacgctcttccgatctnctctcacgggcattcgtattgcgccgcta

SEQ ID NO: 284 - DNA, 53 bp, Artificial Sequence
  primer
  misc_feature (23)..(24): n is a, c, g, or t
ctacacgacgctcttccgatctnnggaatcacggcattcgtattgcgccgcta

SEQ ID NO: 285 - DNA, 54 bp, Artificial Sequence
  primer
  misc_feature (23)..(25): n is a, c, g, or t
ctacacgacgctcttccgatctnnncgttgacgggcattcgtattgcgccgcta

SEQ ID NO: 286 - DNA, 55 bp, Artificial Sequence
  primer
  misc_feature (23)..(26): n is a, c, g, or t
ctacacgacgctcttccgatctnnnncatcaggtggcattcgtattgcgccgcta

SEQ ID NO: 287 - DNA, 52 bp, Artificial Sequence
  primer
  misc_feature 23: n is a, c, g, or t
ctacacgacgctcttccgatctncgttgtaaggcattcgtattgcgccgcta

SEQ ID NO: 288 - DNA, 53 bp, Artificial Sequence
  primer
  misc_feature (23)..(24): n is a, c, g, or t
ctacacgacgctcttccgatctnnggcacggtggcattcgtattgcgccgcta

SEQ ID NO: 289 - DNA, 49 bp, Artificial Sequence
  primer
  misc_feature 23: n is a, c, g, or t
ctacacgacgctcttccgatctnccaatactctcatggartggctaaag

SEQ ID NO: 290 - DNA, 50 bp, Artificial Sequence
  primer
  misc_feature (23)..(24): n is a, c, g, or t
ctacacgacgctcttccgatctnntcgcgcatctcatggartggctaaag

SEQ ID NO: 291 - DNA, 51 bp, Artificial Sequence
  primer
  misc_feature (23)..(25): n is a, c, g, or t
ctacacgacgctcttccgatctnnngtgtgaacctcatggartggctaaag

SEQ ID NO: 292 - DNA, 52 bp, Artificial Sequence
  primer
  misc_feature (23)..(26): n is a, c, g, or t
ctacacgacgctcttccgatctnnnnggtggcacctcatggartggctaaag

SEQ ID NO: 293 - DNA, 49 bp, Artificial Sequence
  primer
  misc_feature 23: n is a, c, g, or t
ctacacgacgctcttccgatctntaggtgctctcatggartggctaaag

SEQ ID NO: 294 - DNA, 50 bp, Artificial Sequence
  primer
  misc_feature (23)..(24): n is a, c, g, or t
ctacacgacgctcttccgatctnngagcggttctcatggartggctaaag

SEQ ID NO: 295 - DNA, 51 bp, Artificial Sequence
  primer
  misc_feature (23)..(25): n is a, c, g, or t
ctacacgacgctcttccgatctnnnaggattagctcatggartggctaaag

SEQ ID NO: 296 - DNA, 52 bp, Artificial Sequence
  primer
  misc_feature (23)..(26): n is a, c, g, or t
ctacacgacgctcttccgatctnnnngtgagccactcatggartggctaaag

SEQ ID NO: 297 - DNA, 49 bp, Artificial Sequence
  primer
  misc_feature 23: n is a, c, g, or t
ctacacgacgctcttccgatctnaattatgcctcatggartggctaaag

SEQ ID NO: 298 - DNA, 50 bp, Artificial Sequence
  primer
  misc_feature (23)..(24): n is a, c, g, or t
ctacacgacgctcttccgatctnnttacgccgctcatggartggctaaag

SEQ ID NO: 299 - DNA, 51 bp, Artificial Sequence
  primer
  misc_feature (23)..(25): n is a, c, g, or t
ctacacgacgctcttccgatctnnngtagtgatctcatggartggctaaag

SEQ ID NO: 300 - DNA, 52 bp, Artificial Sequence
  primer
  misc_feature (23)..(26): n is a, c, g, or t
ctacacgacgctcttccgatctnnnntggttgcactcatggartggctaaag

SEQ ID NO: 301 - DNA, 49 bp, Artificial Sequence
  primer
  misc_feature 23: n is a, c, g, or t
ctacacgacgctcttccgatctngtccgaccctcatggartggctaaag

SEQ ID NO: 302 - DNA, 50 bp, Artificial Sequence
  primer
  misc_feature (23)..(24): n is a, c, g, or t
ctacacgacgctcttccgatctnngccagccgctcatggartggctaaag

SEQ ID NO: 303 - DNA, 51 bp, Artificial Sequence
  primer
  misc_feature (23)..(25): n is a, c, g, or t
ctacacgacgctcttccgatctnnnctcgtgtcctcatggartggctaaag

SEQ ID NO: 304 - DNA, 52 bp, Artificial Sequence
  primer
  misc_feature (23)..(26): n is a, c, g, or t
ctacacgacgctcttccgatctnnnngccgtggcctcatggartggctaaag

SEQ ID NO: 305 - DNA, 49 bp, Artificial Sequence
  primer
  misc_feature 23: n is a, c, g, or t
ctacacgacgctcttccgatctngtagccacctcatggartggctaaag

SEQ ID NO: 306 - DNA, 50 bp, Artificial Sequence
  primer
  misc_feature (23)..(24): n is a, c, g, or t
ctacacgacgctcttccgatctnngacttatactcatggartggctaaag

SEQ ID NO: 307 - DNA, 51 bp, Artificial Sequence
  primer
  misc_feature (23)..(25): n is a, c, g, or t
ctacacgacgctcttccgatctnnngaacgtcgctcatggartggctaaag

SEQ ID NO: 308 - DNA, 52 bp, Artificial Sequence
  primer
  misc_feature (23)..(26): n is a, c, g, or t
ctacacgacgctcttccgatctnnnnatgcgtagctcatggartggctaaag

SEQ ID NO: 309 - DNA, 49 bp, Artificial Sequence
  primer
  misc_feature 23: n is a, c, g, or t
ctacacgacgctcttccgatctnaattagatctcatggartggctaaag

SEQ ID NO: 310 - DNA, 50 bp, Artificial Sequence
  primer
  misc_feature (23)..(24): n is a, c, g, or t
ctacacgacgctcttccgatctnnttacgatactcatggartggctaaag

SEQ ID NO: 311 - DNA, 51 bp, Artificial Sequence
  primer
  misc_feature (23)..(25): n is a, c, g, or t
ctacacgacgctcttccgatctnnnctgtacaactcatggartggctaaag

SEQ ID NO: 312 - DNA, 52 bp, Artificial Sequence
  primer
  misc_feature (23)..(26): n is a, c, g, or t
ctacacgacgctcttccgatctnnnncgtggttgctcatggartggctaaag

SEQ ID NO: 313 - DNA, 49 bp, Artificial Sequence
  primer
  misc_feature 23: n is a, c, g, or t
ctacacgacgctcttccgatctnaataacgtctcatggartggctaaag

SEQ ID NO: 314 - DNA, 50 bp, Artificial Sequence
  primer
  misc_feature (23)..(24): n is a, c, g, or t
ctacacgacgctcttccgatctnnttcttgaactcatggartggctaaag

SEQ ID NO: 315 - DNA, 51 bp, Artificial Sequence
  primer
  misc_feature (23)..(25): n is a, c, g, or t
ctacacgacgctcttccgatctnnnggcagatcctcatggartggctaaag

SEQ ID NO: 316 - DNA, 52 bp, Artificial Sequence
  primer
  misc_feature (23)..(26): n is a, c, g, or t
ctacacgacgctcttccgatctnnnnctatgttactcatggartggctaaag

SEQ ID NO: 317 - DNA, 49 bp, Artificial Sequence
  primer
  misc_feature 23: n is a, c, g, or t
ctacacgacgctcttccgatctngttgacgcctcatggartggctaaag

SEQ ID NO: 318 - DNA, 50 bp, Artificial Sequence
  primer
  misc_feature (23)..(24): n is a, c, g, or t
ctacacgacgctcttccgatctnnatctacgactcatggartggctaaag

SEQ ID NO: 319 - DNA, 51 bp, Artificial Sequence
  primer
  misc_feature (23)..(25): n is a, c, g, or t
ctacacgacgctcttccgatctnnnctcgacagctcatggartggctaaag

SEQ ID NO: 320 - DNA, 52 bp, Artificial Sequence
  primer
  misc_feature (23)..(26): n is a, c, g, or t
ctacacgacgctcttccgatctnnnngaggctgcctcatggartggctaaag

SEQ ID NO: 321 - DNA, 49 bp, Artificial Sequence
  primer
  misc_feature 23: n is a, c, g, or t
ctacacgacgctcttccgatctncctcgtagctcatggartggctaaag

SEQ ID NO: 322 - DNA, 50 bp, Artificial Sequence
  primer
  misc_feature (23)..(24): n is a, c, g, or t
ctacacgacgctcttccgatctnncataggcactcatggartggctaaag

SEQ ID NO: 323 - DNA, 51 bp, Artificial Sequence
  primer
  misc_feature (23)..(25): n is a, c, g, or t
ctacacgacgctcttccgatctnnnagatgaacctcatggartggctaaag

SEQ ID NO: 324 - DNA, 52 bp, Artificial Sequence
  primer
  misc_feature (23)..(26): n is a, c, g, or t
ctacacgacgctcttccgatctnnnnccgagtatctcatggartggctaaag

SEQ ID NO: 325 - DNA, 49 bp, Artificial Sequence
  primer
  misc_feature 23: n is a, c, g, or t
ctacacgacgctcttccgatctnaatattgactcatggartggctaaag

SEQ ID NO: 326 - DNA, 50 bp, Artificial Sequence
  primer
  misc_feature (23)..(24): n is a, c, g, or t
ctacacgacgctcttccgatctnngtataccgctcatggartggctaaag

SEQ ID NO: 327 - DNA, 51 bp, Artificial Sequence
  primer
  misc_feature (23)..(25): n is a, c, g, or t
ctacacgacgctcttccgatctnnngatccaacctcatggartggctaaag

SEQ ID NO: 328 - DNA, 52 bp, Artificial Sequence
  primer
  misc_feature (23)..(26): n is a, c, g, or t
ctacacgacgctcttccgatctnnnnagatacgcctcatggartggctaaag

SEQ ID NO: 329 - DNA, 49 bp, Artificial Sequence
  primer
  misc_feature 23: n is a, c, g, or t
ctacacgacgctcttccgatctnggtatcttctcatggartggctaaag

SEQ ID NO: 330 - DNA, 50 bp, Artificial Sequence
  primer
  misc_feature (23)..(24): n is a, c, g, or t
ctacacgacgctcttccgatctnncctctggcctcatggartggctaaag

SEQ ID NO: 331 - DNA, 49 bp, Artificial Sequence
  primer
  misc_feature 23: n is a, c, g, or t
ctacacgacgctcttccgatctnccattgtgctcatggartggctaaag

SEQ ID NO: 332 - DNA, 50 bp, Artificial Sequence
  primer
  misc_feature (23)..(24): n is a, c, g, or t
ctacacgacgctcttccgatctnnactacggtctcatggartggctaaag

SEQ ID NO: 333 - DNA, 51 bp, Artificial Sequence
  primer
  misc_feature (23)..(25): n is a, c, g, or t
ctacacgacgctcttccgatctnnnaagtgctactcatggartggctaaag

SEQ ID NO: 334 - DNA, 52 bp, Artificial Sequence
  primer
  misc_feature (23)..(26): n is a, c, g, or t
ctacacgacgctcttccgatctnnnngccgaacgctcatggartggctaaag

SEQ ID NO: 335 - DNA, 49 bp, Artificial Sequence
  primer
  misc_feature 23: n is a, c, g, or t
ctacacgacgctcttccgatctntgtccacgctcatggartggctaaag

SEQ ID NO: 336 - DNA, 50 bp, Artificial Sequence
  primer
  misc_feature (23)..(24): n is a, c, g, or t
ctacacgacgctcttccgatctnngacacactctcatggartggctaaag

SEQ ID NO: 337 - DNA, 51 bp, Artificial Sequence
  primer
  misc_feature (23)..(25): n is a, c, g, or t
ctacacgacgctcttccgatctnnnaatatgctctcatggartggctaaag

SEQ ID NO: 338 - DNA, 52 bp, Artificial Sequence
  primer
  misc_feature (23)..(26): n is a, c, g, or t
ctacacgacgctcttccgatctnnnnttctcatactcatggartggctaaag

SEQ ID NO: 339 - DNA, 49 bp, Artificial Sequence
  primer
  misc_feature 23: n is a, c, g, or t
ctacacgacgctcttccgatctntctgtgatctcatggartggctaaag

SEQ ID NO: 340 - DNA, 50 bp, Artificial Sequence
  primer
  misc_feature (23)..(24): n is a, c, g, or t
ctacacgacgctcttccgatctnnccgaacttctcatggartggctaaag

SEQ ID NO: 341 - DNA, 51 bp, Artificial Sequence
  primer
  misc_feature (23)..(25): n is a, c, g, or t
ctacacgacgctcttccgatctnnngtctaacactcatggartggctaaag

SEQ ID NO: 342 - DNA, 52 bp, Artificial Sequence
  primer
  misc_feature (23)..(26): n is a, c, g, or t
ctacacgacgctcttccgatctnnnngacgccatctcatggartggctaaag

SEQ ID NO: 343 - DNA, 49 bp, Artificial Sequence
  primer
  misc_feature 23: n is a, c, g, or t
ctacacgacgctcttccgatctngccaatgtctcatggartggctaaag

SEQ ID NO: 344 - DNA, 50 bp, Artificial Sequence
  primer
  misc_feature (23)..(24): n is a, c, g, or t
ctacacgacgctcttccgatctnnccaacgtcctcatggartggctaaag

SEQ ID NO: 345 - DNA, 51 bp, Artificial Sequence
  primer
  misc_feature (23)..(25): n is a, c, g, or t
ctacacgacgctcttccgatctnnngtagataactcatggartggctaaag

SEQ ID NO: 346 - DNA, 52 bp, Artificial Sequence
  primer
  misc_feature (23)..(26): n is a, c, g, or t
ctacacgacgctcttccgatctnnnncttacggcctcatggartggctaaag

SEQ ID NO: 347 - DNA, 49 bp, Artificial Sequence
  primer
  misc_feature 23: n is a, c, g, or t
ctacacgacgctcttccgatctnccaagtgcctcatggartggctaaag

SEQ ID NO: 348 - DNA, 50 bp, Artificial Sequence
  primer
  misc_feature (23)..(24): n is a, c, g, or t
ctacacgacgctcttccgatctnnctaactcactcatggartggctaaag

SEQ ID NO: 349 - DNA, 51 bp, Artificial Sequence
  primer
  misc_feature (23)..(25): n is a, c, g, or t
ctacacgacgctcttccgatctnnnaatatctgctcatggartggctaaag

SEQ ID NO: 350 - DNA, 52 bp, Artificial Sequence
  primer
  misc_feature (23)..(26): n is a, c, g, or t
ctacacgacgctcttccgatctnnnnttatatcactcatggartggctaaag

SEQ ID NO: 351 - DNA, 49 bp, Artificial Sequence
  primer
  misc_feature 23: n is a, c, g, or t
ctacacgacgctcttccgatctnctgcggatctcatggartggctaaag

SEQ ID NO: 352 - DNA, 50 bp, Artificial Sequence
  primer
  misc_feature (23)..(24): n is a, c, g, or t
ctacacgacgctcttccgatctnngcggcttgctcatggartggctaaag

SEQ ID NO: 353 - DNA, 51 bp, Artificial Sequence
  primer
  misc_feature (23)..(25): n is a, c, g, or t
ctacacgacgctcttccgatctnnngagttgatctcatggartggctaaag

SEQ ID NO: 354 - DNA, 52 bp, Artificial Sequence
  primer
  misc_feature (23)..(26): n is a, c, g, or t
ctacacgacgctcttccgatctnnnngcactgagctcatggartggctaaag

SEQ ID NO: 355 - DNA, 49 bp, Artificial Sequence
  primer
  misc_feature 23: n is a, c, g, or t
ctacacgacgctcttccgatctngaccacctctcatggartggctaaag

SEQ ID NO: 356 - DNA, 49 bp, Artificial Sequence
  primer
  misc_feature 23: n is a, c, g, or t
ctacacgacgctcttccgatctnaatagcaactcatggartggctaaag

SEQ ID NO: 357 - DNA, 49 bp, Artificial Sequence
  primer
  misc_feature 23: n is a, c, g, or t
ctacacgacgctcttccgatctncctaccggctcatggartggctaaag

SEQ ID NO: 358 - DNA, 50 bp, Artificial Sequence
  primer
  misc_feature (23)..(24): n is a, c, g, or t
ctacacgacgctcttccgatctnnggaggatgctcatggartggctaaag

SEQ ID NO: 359 - DNA, 51 bp, Artificial Sequence
  primer
  misc_feature (23)..(25): n is a, c, g, or t
ctacacgacgctcttccgatctnnncgctgaatctcatggartggctaaag

SEQ ID NO: 360 - DNA, 52 bp, Artificial Sequence
  primer
  misc_feature (23)..(26): n is a, c, g, or t
ctacacgacgctcttccgatctnnnntgtgacgactcatggartggctaaag

SEQ ID NO: 361 - DNA, 49 bp, Artificial Sequence
  primer
  misc_feature 23: n is a, c, g, or t
ctacacgacgctcttccgatctnaatagattctcatggartggctaaag

SEQ ID NO: 362 - DNA, 50 bp, Artificial Sequence
  primer
  misc_feature (23)..(24): n is a, c, g, or t
ctacacgacgctcttccgatctnnttagcgcactcatggartggctaaag

SEQ ID NO: 363 - DNA, 51 bp, Artificial Sequence
  primer
  misc_feature (23)..(25): n is a, c, g, or t
ctacacgacgctcttccgatctnnngcggccgtctcatggartggctaaag

SEQ ID NO: 364 - DNA, 52 bp, Artificial Sequence
  primer
  misc_feature (23)..(26): n is a, c, g, or t
ctacacgacgctcttccgatctnnnncagtaaccctcatggartggctaaag

SEQ ID NO: 365 - DNA, 49 bp, Artificial Sequence
  primer
  misc_feature 23: n is a, c, g, or t
ctacacgacgctcttccgatctngcctagtactcatggartggctaaag

SEQ ID NO: 366 - DNA, 50 bp, Artificial Sequence
  primer
  misc_feature (23)..(24): n is a, c, g, or t
ctacacgacgctcttccgatctnncacggcgcctcatggartggctaaag

SEQ ID NO: 367 - DNA, 51 bp, Artificial Sequence
  primer
  misc_feature (23)..(25): n is a, c, g, or t
ctacacgacgctcttccgatctnnnggtgcagactcatggartggctaaag

SEQ ID NO: 368 - DNA, 52 bp, Artificial Sequence
  primer
  misc_feature (23)..(26): n is a, c, g, or t
ctacacgacgctcttccgatctnnnntcgctgacctcatggartggctaaag

SEQ ID NO: 369 - DNA, 49 bp, Artificial Sequence
  primer
  misc_feature 23: n is a, c, g, or t
ctacacgacgctcttccgatctncagccagtctcatggartggctaaag

SEQ ID NO: 370 - DNA, 50 bp, Artificial Sequence
  primer
  misc_feature (23)..(24): n is a, c, g, or t
ctacacgacgctcttccgatctnncgtcaaccctcatggartggctaaag

SEQ ID NO: 371 - DNA, 49 bp, Artificial Sequence
  primer
  misc_feature 23: n is a, c, g, or t
ctacacgacgctcttccgatctngccggcgactcatggartggctaaag

SEQ ID NO: 372 - DNA, 50 bp, Artificial Sequence
  primer
  misc_feature (23)..(24): n is a, c, g, or t
ctacacgacgctcttccgatctnngcctccggctcatggartggctaaag

SEQ ID NO: 373 - DNA, 51 bp, Artificial Sequence
  primer
  misc_feature (23)..(25): n is a, c, g, or t
ctacacgacgctcttccgatctnnnaatagtccctcatggartggctaaag

SEQ ID NO: 374 - DNA, 52 bp, Artificial Sequence
  primer
  misc_feature (23)..(26): n is a, c, g, or t
ctacacgacgctcttccgatctnnnnttagacgtctcatggartggctaaag

SEQ ID NO: 375 - DNA, 49 bp, Artificial Sequence
  primer
  misc_feature 23: n is a, c, g, or t
ctacacgacgctcttccgatctngtggactactcatggartggctaaag

SEQ ID NO: 376 - DNA, 50 bp, Artificial Sequence
  primer
  misc_feature (23)..(24): n is a, c, g, or t
ctacacgacgctcttccgatctnncacggacgctcatggartggctaaag

SEQ ID NO: 377 - DNA, 51 bp, Artificial Sequence
  primer
  misc_feature (23)..(25): n is a, c, g, or t
ctacacgacgctcttccgatctnnncactagagctcatggartggctaaag

SEQ ID NO: 378 - DNA, 52 bp, Artificial Sequence
  primer
  misc_feature (23)..(26): n is a, c, g, or t
ctacacgacgctcttccgatctnnnngcagatggctcatggartggctaaag

SEQ ID NO: 379 - DNA, 49 bp, Artificial Sequence
  primer
  misc_feature 23: n is a, c, g, or t
ctacacgacgctcttccgatctnctctcacgctcatggartggctaaag

SEQ ID NO: 380 - DNA, 50 bp, Artificial Sequence
  primer
  misc_feature (23)..(24): n is a, c, g, or t
ctacacgacgctcttccgatctnnggaatcacctcatggartggctaaag

SEQ ID NO: 381 - DNA, 51 bp, Artificial Sequence
  primer
  misc_feature (23)..(25): n is a, c, g, or t
ctacacgacgctcttccgatctnnncgttgacgctcatggartggctaaag

SEQ ID NO: 382 - DNA, 52 bp, Artificial Sequence
  primer
  misc_feature (23)..(26): n is a, c, g, or t
ctacacgacgctcttccgatctnnnncatcaggtctcatggartggctaaag

SEQ ID NO: 383 - DNA, 49 bp, Artificial Sequence
  primer
  misc_feature 23: n is a, c, g, or t
ctacacgacgctcttccgatctncgttgtaactcatggartggctaaag

SEQ ID NO: 384 - DNA, 50 bp, Artificial Sequence
  primer
  misc_feature (23)..(24): n is a, c, g, or t
ctacacgacgctcttccgatctnnggcacggtctcatggartggctaaag

SEQ ID NO: 385 - DNA, 48 bp, Artificial Sequence
  primer
  misc_feature 23: n is a, c, g, or t
ctacacgacgctcttccgatctnccaatactgccttctccatcttctg

SEQ ID NO: 386 - DNA, 49 bp, Artificial Sequence
  primer
  misc_feature (23)..(24): n is a, c, g, or t
ctacacgacgctcttccgatctnntcgcgcatgccttctccatcttctg

SEQ ID NO: 387 - DNA, 50 bp, Artificial Sequence
  primer
  misc_feature (23)..(25): n is a, c, g, or t
ctacacgacgctcttccgatctnnngtgtgaacgccttctccatcttctg

SEQ ID NO: 388 - DNA, 51 bp, Artificial Sequence
  primer
  misc_feature (23)..(26): n is a, c, g, or t
ctacacgacgctcttccgatctnnnnggtggcacgccttctccatcttctg

SEQ ID NO: 389 - DNA, 48 bp, Artificial Sequence
  primer
  misc_feature 23: n is a, c, g, or t
ctacacgacgctcttccgatctntaggtgctgccttctccatcttctg

SEQ ID NO: 390 - DNA, 49 bp, Artificial Sequence
  primer
  misc_feature (23)..(24): n is a, c, g, or t
ctacacgacgctcttccgatctnngagcggttgccttctccatcttctg

SEQ ID NO: 391 - DNA, 50 bp, Artificial Sequence
  primer
  misc_feature (23)..(25): n is a, c, g, or t
ctacacgacgctcttccgatctnnnaggattaggccttctccatcttctg

SEQ ID NO: 392 - DNA, 51 bp, Artificial Sequence
  primer
  misc_feature (23)..(26): n is a, c, g, or t
ctacacgacgctcttccgatctnnnngtgagccagccttctccatcttctg

SEQ ID NO: 393 - DNA, 48 bp, Artificial Sequence
  primer
  misc_feature 23: n is a, c, g, or t
ctacacgacgctcttccgatctnaattatgcgccttctccatcttctg

SEQ ID NO: 394 - DNA, 49 bp, Artificial Sequence
  primer
  misc_feature (23)..(24): n is a, c, g, or t
ctacacgacgctcttccgatctnnttacgccggccttctccatcttctg

SEQ ID NO: 395 - DNA, 50 bp, Artificial Sequence
  primer
  misc_feature (23)..(25): n is a, c, g, or t
ctacacgacgctcttccgatctnnngtagtgatgccttctccatcttctg

SEQ ID NO: 396 - DNA, 51 bp, Artificial Sequence
  primer
  misc_feature (23)..(26): n is a, c, g, or t
ctacacgacgctcttccgatctnnnntggttgcagccttctccatcttctg

SEQ ID NO: 397 - DNA, 48 bp, Artificial Sequence
  primer
  misc_feature 23: n is a, c, g, or t
ctacacgacgctcttccgatctngtccgaccgccttctccatcttctg

SEQ ID NO: 398 - DNA, 49 bp, Artificial Sequence
  primer
  misc_feature (23)..(24): n is a, c, g, or t
ctacacgacgctcttccgatctnngccagccggccttctccatcttctg

SEQ ID NO: 399 - DNA, 50 bp, Artificial Sequence
  primer
  misc_feature (23)..(25): n is a, c, g, or t
ctacacgacgctcttccgatctnnnctcgtgtcgccttctccatcttctg

SEQ ID NO: 400 - DNA, 51 bp, Artificial Sequence
  primer
  misc_feature (23)..(26): n is a, c, g, or t
ctacacgacgctcttccgatctnnnngccgtggcgccttctccatcttctg

SEQ ID NO: 401 - DNA, 48 bp, Artificial Sequence
  primer
  misc_feature 23: n is a, c, g, or t
ctacacgacgctcttccgatctngtagccacgccttctccatcttctg

SEQ ID NO: 402 - DNA, 49 bp, Artificial Sequence
  primer
  misc_feature (23)..(24): n is a, c, g, or t
ctacacgacgctcttccgatctnngacttatagccttctccatcttctg

SEQ ID NO: 403 - DNA, 50 bp, Artificial Sequence
  primer
  misc_feature (23)..(25): n is a, c, g, or t
ctacacgacgctcttccgatctnnngaacgtcggccttctccatcttctg

SEQ ID NO: 404 - DNA, 51 bp, Artificial Sequence
  primer
  misc_feature (23)..(26): n is a, c, g, or t
ctacacgacgctcttccgatctnnnnatgcgtaggccttctccatcttctg

SEQ ID NO: 405 - DNA, 48 bp, Artificial Sequence
  primer
  misc_feature 23: n is a, c, g, or t
ctacacgacgctcttccgatctnaattagatgccttctccatcttctg

SEQ ID NO: 406 - DNA, 49 bp, Artificial Sequence
  primer
  misc_feature (23)..(24): n is a, c, g, or t
ctacacgacgctcttccgatctnnttacgatagccttctccatcttctg

SEQ ID NO: 407 - DNA, 50 bp, Artificial Sequence
  primer
  misc_feature (23)..(25): n is a, c, g, or t
ctacacgacgctcttccgatctnnnctgtacaagccttctccatcttctg

SEQ ID NO: 408 - DNA, 51 bp, Artificial Sequence
  primer
  misc_feature (23)..(26): n is a, c, g, or t
ctacacgacgctcttccgatctnnnncgtggttggccttctccatcttctg

SEQ ID NO: 409 - DNA, 48 bp, Artificial Sequence
  primer
  misc_feature 23: n is a, c, g, or t
ctacacgacgctcttccgatctnaataacgtgccttctccatcttctg

SEQ ID NO: 410 - DNA, 49 bp, Artificial Sequence
  primer
  misc_feature (23)..(24): n is a, c, g, or t
ctacacgacgctcttccgatctnnttcttgaagccttctccatcttctg

SEQ ID NO: 411 - DNA, 50 bp, Artificial Sequence
  primer
  misc_feature (23)..(25): n is a, c, g, or t
ctacacgacgctcttccgatctnnnggcagatcgccttctccatcttctg

SEQ ID NO: 412 - DNA, 51 bp, Artificial Sequence
  primer
  misc_feature (23)..(26): n is a, c, g, or t
ctacacgacgctcttccgatctnnnnctatgttagccttctccatcttctg

SEQ ID NO: 413 - DNA, 48 bp, Artificial Sequence
  primer
  misc_feature 23: n is a, c, g, or t
ctacacgacgctcttccgatctngttgacgcgccttctccatcttctg

SEQ ID NO: 414 - DNA, 49 bp, Artificial Sequence
  primer
  misc_feature (23)..(24): n is a, c, g, or t
ctacacgacgctcttccgatctnnatctacgagccttctccatcttctg

SEQ ID NO: 415 - DNA, 50 bp, Artificial Sequence
  primer
  misc_feature (23)..(25): n is a, c, g, or t
ctacacgacgctcttccgatctnnnctcgacaggccttctccatcttctg

SEQ ID NO: 416 - DNA, 51 bp, Artificial Sequence
  primer
  misc_feature (23)..(26): n is a, c, g, or t
ctacacgacgctcttccgatctnnnngaggctgcgccttctccatcttctg

SEQ ID NO: 417 - DNA, 48 bp, Artificial Sequence
  primer
  misc_feature 23: n is a, c, g, or t
ctacacgacgctcttccgatctncctcgtaggccttctccatcttctg

SEQ ID NO: 418 - DNA, 49 bp, Artificial Sequence
  primer
  misc_feature (23)..(24): n is a, c, g, or t
ctacacgacgctcttccgatctnncataggcagccttctccatcttctg

SEQ ID NO: 419 - DNA, 50 bp, Artificial Sequence
  primer
  misc_feature (23)..(25): n is a, c, g, or t
ctacacgacgctcttccgatctnnnagatgaacgccttctccatcttctg

SEQ ID NO: 420 - DNA, 51 bp, Artificial Sequence
  primer
  misc_feature (23)..(26): n is a, c, g, or t
ctacacgacgctcttccgatctnnnnccgagtatgccttctccatcttctg

SEQ ID NO: 421 - DNA, 48 bp, Artificial Sequence
  primer
  misc_feature 23: n is a, c, g, or t
ctacacgacgctcttccgatctnaatattgagccttctccatcttctg

SEQ ID NO: 422 - DNA, 49 bp, Artificial Sequence
  primer
  misc_feature (23)..(24): n is a, c, g, or t
ctacacgacgctcttccgatctnngtataccggccttctccatcttctg

SEQ ID NO: 423 - DNA, 50 bp, Artificial Sequence
  primer
  misc_feature (23)..(25): n is a, c, g, or t
ctacacgacgctcttccgatctnnngatccaacgccttctccatcttctg

SEQ ID NO: 424 - DNA, 51 bp, Artificial Sequence
  primer
  misc_feature (23)..(26): n is a, c, g, or t
ctacacgacgctcttccgatctnnnnagatacgcgccttctccatcttctg

SEQ ID NO: 425 - DNA, 48 bp, Artificial Sequence
  primer
  misc_feature 23: n is a, c, g, or t
ctacacgacgctcttccgatctnggtatcttgccttctccatcttctg

SEQ ID NO: 426 - DNA, 49 bp, Artificial Sequence
  primer
  misc_feature (23)..(24): n is a, c, g, or t
ctacacgacgctcttccgatctnncctctggcgccttctccatcttctg

SEQ ID NO: 427 - DNA, 48 bp, Artificial Sequence
  primer
  misc_feature 23: n is a, c, g, or t
ctacacgacgctcttccgatctnccattgtggccttctccatcttctg

SEQ ID NO: 428 - DNA, 49 bp, Artificial Sequence
  primer
  misc_feature (23)..(24): n is a, c, g, or t
ctacacgacgctcttccgatctnnactacggtgccttctccatcttctg

SEQ ID NO: 429 - DNA, 50 bp, Artificial Sequence
  primer
  misc_feature (23)..(25): n is a, c, g, or t
ctacacgacgctcttccgatctnnnaagtgctagccttctccatcttctg

SEQ ID NO: 430 - DNA, 51 bp, Artificial Sequence
  primer
  misc_feature (23)..(26): n is a, c, g, or t
ctacacgacgctcttccgatctnnnngccgaacggccttctccatcttctg

SEQ ID NO: 431 - DNA, 48 bp, Artificial Sequence
  primer
  misc_feature 23: n is a, c, g, or t
ctacacgacgctcttccgatctntgtccacggccttctccatcttctg

SEQ ID NO: 432 - DNA, 49 bp, Artificial Sequence
  primer
  misc_feature (23)..(24): n is a, c, g, or t
ctacacgacgctcttccgatctnngacacactgccttctccatcttctg

SEQ ID NO: 433 - DNA, 50 bp, Artificial Sequence
  primer
  misc_feature (23)..(25): n is a, c, g, or t
ctacacgacgctcttccgatctnnnaatatgctgccttctccatcttctg

SEQ ID NO: 434 - DNA, 51 bp, Artificial Sequence
  primer
  misc_feature (23)..(26): n is a, c, g, or t
ctacacgacgctcttccgatctnnnnttctcatagccttctccatcttctg

SEQ ID NO: 435 - DNA, 48 bp, Artificial Sequence
  primer
  misc_feature 23: n is a, c, g, or t
ctacacgacgctcttccgatctntctgtgatgccttctccatcttctg

SEQ ID NO: 436 - DNA, 49 bp, Artificial Sequence
  primer
  misc_feature (23)..(24): n is a, c, g, or t
ctacacgacgctcttccgatctnnccgaacttgccttctccatcttctg

SEQ ID NO: 437 - DNA, 50 bp, Artificial Sequence
  primer
  misc_feature (23)..(25): n is a, c, g, or t
ctacacgacgctcttccgatctnnngtctaacagccttctccatcttctg

SEQ ID NO: 438 - DNA, 51 bp, Artificial Sequence
  primer
  misc_feature (23)..(26): n is a, c, g, or t
ctacacgacgctcttccgatctnnnngacgccatgccttctccatcttctg

SEQ ID NO: 439 - DNA, 48 bp, Artificial Sequence
  primer
  misc_feature 23: n is a, c, g, or t
ctacacgacgctcttccgatctngccaatgtgccttctccatcttctg

SEQ ID NO: 440 - DNA, 49 bp, Artificial Sequence
  primer
  misc_feature (23)..(24): n is a, c, g, or t
ctacacgacgctcttccgatctnnccaacgtcgccttctccatcttctg

SEQ ID NO: 441 - DNA, 50 bp, Artificial Sequence
  primer
  misc_feature (23)..(25): n is a, c, g, or t
ctacacgacgctcttccgatctnnngtagataagccttctccatcttctg

SEQ ID NO: 442 - DNA, 51 bp, Artificial Sequence
  primer
  misc_feature (23)..(26): n is a, c, g, or t
ctacacgacgctcttccgatctnnnncttacggcgccttctccatcttctg

SEQ ID NO: 443 - DNA, 48 bp, Artificial Sequence
  primer
  misc_feature 23: n is a, c, g, or t
ctacacgacgctcttccgatctnccaagtgcgccttctccatcttctg

SEQ ID NO: 444 - DNA, 49 bp, Artificial Sequence
  primer
  misc_feature (23)..(24): n is a, c, g, or t
ctacacgacgctcttccgatctnnctaactcagccttctccatcttctg

SEQ ID NO: 445 - DNA, 50 bp, Artificial Sequence
  primer
  misc_feature (23)..(25): n is a, c, g, or t
ctacacgacgctcttccgatctnnnaatatctggccttctccatcttctg

SEQ ID NO: 446 - DNA, 51 bp, Artificial Sequence
  primer
  misc_feature (23)..(26): n is a, c, g, or t
ctacacgacgctcttccgatctnnnnttatatcagccttctccatcttctg

SEQ ID NO: 447 - DNA, 48 bp, Artificial Sequence
  primer
  misc_feature 23: n is a, c, g, or t
ctacacgacgctcttccgatctnctgcggatgccttctccatcttctg

SEQ ID NO: 448 - DNA, 49 bp, Artificial Sequence
  primer
  misc_feature (23)..(24): n is a, c, g, or t
ctacacgacgctcttccgatctnngcggcttggccttctccatcttctg

SEQ ID NO: 449 - DNA, 50 bp, Artificial Sequence
  primer
  misc_feature (23)..(25): n is a, c, g, or t
ctacacgacgctcttccgatctnnngagttgatgccttctccatcttctg

SEQ ID NO: 450 - DNA, 51 bp, Artificial Sequence
  primer
  misc_feature (23)..(26): n is a, c, g, or t
ctacacgacgctcttccgatctnnnngcactgaggccttctccatcttctg

SEQ ID NO: 451 - DNA, 48 bp, Artificial Sequence
  primer
  misc_feature 23: n is a, c, g, or t
ctacacgacgctcttccgatctngaccacctgccttctccatcttctg

SEQ ID NO: 452 - DNA, 48 bp, Artificial Sequence
  primer
  misc_feature 23: n is a, c, g, or t
ctacacgacgctcttccgatctnaatagcaagccttctccatcttctg

SEQ ID NO: 453 - DNA, 48 bp, Artificial Sequence
  primer
  misc_feature 23: n is a, c, g, or t
ctacacgacgctcttccgatctncctaccgggccttctccatcttctg

SEQ ID NO: 454 - DNA, 49 bp, Artificial Sequence
  primer
  misc_feature (23)..(24): n is a, c, g, or t
ctacacgacgctcttccgatctnnggaggatggccttctccatcttctg

SEQ ID NO: 455 - DNA, 50 bp, Artificial Sequence
  primer
  misc_feature (23)..(25): n is a, c, g, or t
ctacacgacgctcttccgatctnnncgctgaatgccttctccatcttctg

SEQ ID NO: 456 - DNA, 51 bp, Artificial Sequence
  primer
  misc_feature (23)..(26): n is a, c, g, or t
ctacacgacgctcttccgatctnnnntgtgacgagccttctccatcttctg

SEQ ID NO: 457 - DNA, 48 bp, Artificial Sequence
  primer
  misc_feature 23: n is a, c, g, or t
ctacacgacgctcttccgatctnaatagattgccttctccatcttctg

SEQ ID NO: 458 - DNA, 49 bp, Artificial Sequence
  primer
  misc_feature (23)..(24): n is a, c, g, or t
ctacacgacgctcttccgatctnnttagcgcagccttctccatcttctg

SEQ ID NO: 459 - DNA, 50 bp, Artificial Sequence
  primer
  misc_feature (23)..(25): n is a, c, g, or t
ctacacgacgctcttccgatctnnngcggccgtgccttctccatcttctg

SEQ ID NO: 460 - DNA, 51 bp, Artificial Sequence
  primer
  misc_feature (23)..(26): n is a, c, g, or t
ctacacgacgctcttccgatctnnnncagtaaccgccttctccatcttctg

SEQ ID NO: 461 - DNA, 48 bp, Artificial Sequence
  primer
  misc_feature 23: n is a, c, g, or t
ctacacgacgctcttccgatctngcctagtagccttctccatcttctg

SEQ ID NO: 462 - DNA, 49 bp, Artificial Sequence
  primer
  misc_feature (23)..(24): n is a, c, g, or t
ctacacgacgctcttccgatctnncacggcgcgccttctccatcttctg

SEQ ID NO: 463 - DNA, 50 bp, Artificial Sequence
  primer
  misc_feature (23)..(25): n is a, c, g, or t
ctacacgacgctcttccgatctnnnggtgcagagccttctccatcttctg

SEQ ID NO: 464 - DNA, 51 bp, Artificial Sequence
  primer
  misc_feature (23)..(26): n is a, c, g, or t
ctacacgacgctcttccgatctnnnntcgctgacgccttctccatcttctg

SEQ ID NO: 465 - DNA, 48 bp, Artificial Sequence
  primer
  misc_feature 23: n is a, c, g, or t
ctacacgacgctcttccgatctncagccagtgccttctccatcttctg

SEQ ID NO: 466 - DNA, 49 bp, Artificial Sequence
  primer
  misc_feature (23)..(24): n is a, c, g, or t
ctacacgacgctcttccgatctnncgtcaaccgccttctccatcttctg

SEQ ID NO: 467 - DNA, 48 bp, Artificial Sequence
  primer
  misc_feature 23: n is a, c, g, or t
ctacacgacgctcttccgatctngccggcgagccttctccatcttctg

SEQ ID NO: 468 - DNA, 49 bp, Artificial Sequence
  primer
  misc_feature (23)..(24): n is a, c, g, or t
ctacacgacgctcttccgatctnngcctccgggccttctccatcttctg

SEQ ID NO: 469 - DNA, 50 bp, Artificial Sequence
  primer
  misc_feature (23)..(25): n is a, c, g, or t
ctacacgacgctcttccgatctnnnaatagtccgccttctccatcttctg

SEQ ID NO: 470 - DNA, 51 bp, Artificial Sequence
  primer
  misc_feature (23)..(26): n is a, c, g, or t
ctacacgacgctcttccgatctnnnnttagacgtgccttctccatcttctg

SEQ ID NO: 471 - DNA, 48 bp, Artificial Sequence
  primer
  misc_feature 23: n is a, c, g, or t
ctacacgacgctcttccgatctngtggactagccttctccatcttctg

SEQ ID NO: 472 - DNA, 49 bp, Artificial Sequence
  primer
  misc_feature (23)..(24): n is a, c, g, or t
ctacacgacgctcttccgatctnncacggacggccttctccatcttctg

SEQ ID NO: 473 - DNA, 50 bp, Artificial Sequence
  primer
  misc_feature (23)..(25): n is a, c, g, or t
ctacacgacgctcttccgatctnnncactagaggccttctccatcttctg

SEQ ID NO: 474 - DNA, 51 bp, Artificial Sequence
  primer
  misc_feature (23)..(26): n is a, c, g, or t
ctacacgacgctcttccgatctnnnngcagatgggccttctccatcttctg

SEQ ID NO: 475 - DNA, 48 bp, Artificial Sequence
  primer
  misc_feature 23: n is a, c, g, or t
ctacacgacgctcttccgatctnctctcacggccttctccatcttctg

SEQ ID NO: 476 - DNA, 49 bp, Artificial Sequence
  primer
  misc_feature (23)..(24): n is a, c, g, or t
ctacacgacgctcttccgatctnnggaatcacgccttctccatcttctg

SEQ ID NO: 477 - DNA, 50 bp, Artificial Sequence
  primer
  misc_feature (23)..(25): n is a, c, g, or t
ctacacgacgctcttccgatctnnncgttgacggccttctccatcttctg

SEQ ID NO: 478 - DNA, 51 bp, Artificial Sequence
  primer
  misc_feature (23)..(26): n is a, c, g, or t
ctacacgacgctcttccgatctnnnncatcaggtgccttctccatcttctg

SEQ ID NO: 479 - DNA, 48 bp, Artificial Sequence
  primer
  misc_feature 23: n is a, c, g, or t
ctacacgacgctcttccgatctncgttgtaagccttctccatcttctg

SEQ ID NO: 480 - DNA, 49 bp, Artificial Sequence
  primer
  misc_feature (23)..(24): n is a, c, g, or t
ctacacgacgctcttccgatctnnggcacggtgccttctccatcttctg

SEQ ID NO: 481 - DNA, 48 bp, Artificial Sequence
  primer
  misc_feature 23: n is a, c, g, or t
ctacacgacgctcttccgatctnaattaatgtcctccggcccctgaat

SEQ ID NO: 482 - DNA, 49 bp, Artificial Sequence
  primer
  misc_feature (23)..(24): n is a, c, g, or t
ctacacgacgctcttccgatctnnttaattcctcctccggcccctgaat

SEQ ID NO: 483 - DNA, 48 bp, Artificial Sequence
  primer
  misc_feature 23: n is a, c, g, or t
ctacacgacgctcttccgatctnccaatacttcctccggcccctgaat

SEQ ID NO: 484 - DNA, 49 bp, Artificial Sequence
  primer
  misc_feature (23)..(24): n is a, c, g, or t
ctacacgacgctcttccgatctnntcgcgcattcctccggcccctgaat

SEQ ID NO: 485 - DNA, 50 bp, Artificial Sequence
  primer
  misc_feature (23)..(25): n is a, c, g, or t
ctacacgacgctcttccgatctnnngtgtgaactcctccggcccctgaat

SEQ ID NO: 486 - DNA, 51 bp, Artificial Sequence
  primer
  misc_feature (23)..(26): n is a, c, g, or t
ctacacgacgctcttccgatctnnnnggtggcactcctccggcccctgaat

SEQ ID NO: 487 - DNA, 48 bp, Artificial Sequence
  primer
  misc_feature 23: n is a, c, g, or t
ctacacgacgctcttccgatctntaggtgcttcctccggcccctgaat

SEQ ID NO: 488 - DNA, 49 bp, Artificial Sequence
  primer
  misc_feature (23)..(24): n is a, c, g, or t
ctacacgacgctcttccgatctnngagcggtttcctccggcccctgaat

SEQ ID NO: 489 - DNA, 50 bp, Artificial Sequence
  primer
  misc_feature (23)..(25): n is a, c, g, or t
ctacacgacgctcttccgatctnnnaggattagtcctccggcccctgaat

SEQ ID NO: 490 - DNA, 51 bp, Artificial Sequence
  primer
  misc_feature (23)..(26): n is a, c, g, or t
ctacacgacgctcttccgatctnnnngtgagccatcctccggcccctgaat

SEQ ID NO: 491 - DNA, 48 bp, Artificial Sequence
  primer
  misc_feature 23: n is a, c, g, or t
ctacacgacgctcttccgatctnaattatgctcctccggcccctgaat

SEQ ID NO: 492 - DNA, 49 bp, Artificial Sequence
  primer
  misc_feature (23)..(24): n is a, c, g, or t
ctacacgacgctcttccgatctnnttacgccgtcctccggcccctgaat

SEQ ID NO: 493 - DNA, 50 bp, Artificial Sequence
  primer
  misc_feature (23)..(25): n is a, c, g, or t
ctacacgacgctcttccgatctnnngtagtgattcctccggcccctgaat

SEQ ID NO: 494 - DNA, 51 bp, Artificial Sequence
  primer
  misc_feature (23)..(26): n is a, c, g, or t
ctacacgacgctcttccgatctnnnntggttgcatcctccggcccctgaat

SEQ ID NO: 495 - DNA, 48 bp, Artificial Sequence
  primer
  misc_feature 23: n is a, c, g, or t
ctacacgacgctcttccgatctngtccgacctcctccggcccctgaat

SEQ ID NO: 496 - DNA, 66 bp, Artificial Sequence
  primer
gtgactggagttcagacgtgtgctcttccgatctagcttggttctggttactgccagttgaatctg

SEQ ID NO: 497 - DNA, 66 bp, Artificial Sequence
  primer
gtgactggagttcagacgtgtgctcttccgatctagcttatgtctggttactgccagttgaatctg

SEQ ID NO: 498 - DNA, 66 bp, Artificial Sequence
  primer
gtgactggagttcagacgtgtgctcttccgatctataacgactctggttactgccagttgaatctg

SEQ ID NO: 499 - DNA, 66 bp, Artificial Sequence
  primer
gtgactggagttcagacgtgtgctcttccgatctgatggagttctggttactgccagttgaatctg

SEQ ID NO: 500 - DNA, 66 bp, Artificial Sequence
  primer
gtgactggagttcagacgtgtgctcttccgatcttgatctaatctggttactgccagttgaatctg

SEQ ID NO: 501 - DNA, 66 bp, Artificial Sequence
  primer
gtgactggagttcagacgtgtgctcttccgatctagctatattctggttactgccagttgaatctg

SEQ ID NO: 502 - DNA, 66 bp, Artificial Sequence
  primer
gtgactggagttcagacgtgtgctcttccgatctagcagagatctggttactgccagttgaatctg

SEQ ID NO: 503 - DNA, 66 bp, Artificial Sequence
  primer
gtgactggagttcagacgtgtgctcttccgatctgacgtaagtctggttactgccagttgaatctg

SEQ ID NO: 504 - DNA, 66 bp, Artificial Sequence
  primer
gtgactggagttcagacgtgtgctcttccgatctaggcctgatctggttactgccagttgaatctg

SEQ ID NO: 505 - DNA, 66 bp, Artificial Sequence
  primer
gtgactggagttcagacgtgtgctcttccgatcttaagattatctggttactgccagttgaatctg

SEQ ID NO: 506 - DNA, 66 bp, Artificial Sequence
  primer
gtgactggagttcagacgtgtgctcttccgatctaggcgaattctggttactgccagttgaatctg

SEQ ID NO: 507 - DNA, 66 bp, Artificial Sequence
  primer
gtgactggagttcagacgtgtgctcttccgatctttgttctttctggttactgccagttgaatctg

SEQ ID NO: 508 - DNA, 66 bp, Artificial Sequence
  primer
gtgactggagttcagacgtgtgctcttccgatcttactcctgtctggttactgccagttgaatctg

SEQ ID NO: 509 - DNA, 66 bp, Artificial Sequence
  primer
gtgactggagttcagacgtgtgctcttccgatctgactggcgtctggttactgccagttgaatctg

SEQ ID NO: 510 - DNA, 66 bp, Artificial Sequence
  primer
gtgactggagttcagacgtgtgctcttccgatctatatatactctggttactgccagttgaatctg

SEQ ID NO: 511 - DNA, 66 bp, Artificial Sequence
  primer
gtgactggagttcagacgtgtgctcttccgatcttagatcggtctggttactgccagttgaatctg

SEQ ID NO: 512 - DNA, 66 bp, Artificial Sequence
  primer
gtgactggagttcagacgtgtgctcttccgatctaggcaagctctggttactgccagttgaatctg

SEQ ID NO: 513 - DNA, 66 bp, Artificial Sequence
  primer
gtgactggagttcagacgtgtgctcttccgatcttccaggtatctggttactgccagttgaatctg

SEQ ID NO: 514 - DNA, 66 bp, Artificial Sequence
  primer
gtgactggagttcagacgtgtgctcttccgatctaggtcaagtctggttactgccagttgaatctg

SEQ ID NO: 515 - DNA, 66 bp, Artificial Sequence
  primer
gtgactggagttcagacgtgtgctcttccgatcttacactggtctggttactgccagttgaatctg

SEQ ID NO: 516 - DNA, 66 bp, Artificial Sequence
  primer
gtgactggagttcagacgtgtgctcttccgatcttccttgcgtctggttactgccagttgaatctg

SEQ ID NO: 517 - DNA, 66 bp, Artificial Sequence
  primer
gtgactggagttcagacgtgtgctcttccgatctaggacctctctggttactgccagttgaatctg

SEQ ID NO: 518 - DNA, 66 bp, Artificial Sequence
  primer
gtgactggagttcagacgtgtgctcttccgatcttaagcatttctggttactgccagttgaatctg

SEQ ID NO: 519 - DNA, 66 bp, Artificial Sequence
  primer
gtgactggagttcagacgtgtgctcttccgatctaggatatttctggttactgccagttgaatctg

SEQ ID NO: 520 - DNA, 66 bp, Artificial Sequence
  primer
gtgactggagttcagacgtgtgctcttccgatctaatcgttatctggttactgccagttgaatctg

SEQ ID NO: 521 - DNA, 66 bp, Artificial Sequence
  primer
gtgactggagttcagacgtgtgctcttccgatctgtctacattctggttactgccagttgaatctg

SEQ ID NO: 522 - DNA, 66 bp, Artificial Sequence
  primer
gtgactggagttcagacgtgtgctcttccgatctcgctgctctctggttactgccagttgaatctg

SEQ ID NO: 523 - DNA, 66 bp, Artificial Sequence
  primer
gtgactggagttcagacgtgtgctcttccgatctgatcaacatctggttactgccagttgaatctg

SEQ ID NO: 524 - DNA, 66 bp, Artificial Sequence
  primer
gtgactggagttcagacgtgtgctcttccgatctcgaaggactctggttactgccagttgaatctg

SEQ ID NO: 525 - DNA, 66 bp, Artificial Sequence
  primer
gtgactggagttcagacgtgtgctcttccgatctgatgccggtctggttactgccagttgaatctg

SEQ ID NO: 526 - DNA, 66 bp, Artificial Sequence
  primer
gtgactggagttcagacgtgtgctcttccgatctctacgaagtctggttactgccagttgaatctg

SEQ ID NO: 527 - DNA, 66 bp, Artificial Sequence
  primer
gtgactggagttcagacgtgtgctcttccgatctgatgcgtctctggttactgccagttgaatctg

SEQ ID NO: 528 - DNA, 66 bp, Artificial Sequence
  primer
gtgactggagttcagacgtgtgctcttccgatctctacggcatctggttactgccagttgaatctg

SEQ ID NO: 529 - DNA, 66 bp, Artificial Sequence
  primer
gtgactggagttcagacgtgtgctcttccgatctgattcctttctggttactgccagttgaatctg

SEQ ID NO: 530 - DNA, 66 bp, Artificial Sequence
  primer
gtgactggagttcagacgtgtgctcttccgatctctactcgatctggttactgccagttgaatctg

SEQ ID NO: 531 - DNA, 66 bp, Artificial Sequence
  primer
gtgactggagttcagacgtgtgctcttccgatctgattcgagtctggttactgccagttgaatctg

SEQ ID NO: 532 - DNA, 66 bp, Artificial Sequence
  primer
gtgactggagttcagacgtgtgctcttccgatctaatcggcgtctggttactgccagttgaatctg

SEQ ID NO: 533 - DNA, 66 bp, Artificial Sequence
  primer
gtgactggagttcagacgtgtgctcttccgatctttcgccgatctggttactgccagttgaatctg

SEQ ID NO: 534 - DNA, 66 bp, Artificial Sequence
  primer
gtgactggagttcagacgtgtgctcttccgatctctggcctctctggttactgccagttgaatctg

SEQ ID NO: 535 - DNA, 66 bp, Artificial Sequence
  primer
gtgactggagttcagacgtgtgctcttccgatctgaacttattctggttactgccagttgaatctg

SEQ ID NO: 536 - DNA, 66 bp, Artificial Sequence
  primer
gtgactggagttcagacgtgtgctcttccgatctcgtattggtctggttactgccagttgaatctg

SEQ ID NO: 537 - DNA, 66 bp, Artificial Sequence
  primer
gtgactggagttcagacgtgtgctcttccgatctgaagcacatctggttactgccagttgaatctg

SEQ ID NO: 538 - DNA, 66 bp, Artificial Sequence
  primer
gtgactggagttcagacgtgtgctcttccgatctcttaatactctggttactgccagttgaatctg

SEQ ID NO: 539 - DNA, 66 bp, Artificial Sequence
  primer
gtgactggagttcagacgtgtgctcttccgatctgaagtctttctggttactgccagttgaatctg

SEQ ID NO: 540 - DNA, 66 bp, Artificial Sequence
  primer
gtgactggagttcagacgtgtgctcttccgatctgaagaggctctggttactgccagttgaatctg

SEQ ID NO: 541 - DNA, 66 bp, Artificial Sequence
  primer
gtgactggagttcagacgtgtgctcttccgatctcggataactctggttactgccagttgaatctg

SEQ ID NO: 542 - DNA, 66 bp, Artificial Sequence
  primer
gtgactggagttcagacgtgtgctcttccgatctgaatctggtctggttactgccagttgaatctg

SEQ ID NO: 543 - DNA, 66 bp, Artificial Sequence
  primer
gtgactggagttcagacgtgtgctcttccgatctctgattgatctggttactgccagttgaatctg

SEQ ID NO: 544 - DNA, 66 bp, Artificial Sequence
  primer
gtgactggagttcagacgtgtgctcttccgatctaatccgtttctggttactgccagttgaatctg

SEQ ID NO: 545 - DNA, 66 bp, Artificial Sequence
  primer
gtgactggagttcagacgtgtgctcttccgatcttgcgtacatctggttactgccagttgaatctg

SEQ ID NO: 546 - DNA, 66 bp, Artificial Sequence
  primer
gtgactggagttcagacgtgtgctcttccgatctgaatcaattctggttactgccagttgaatctg

SEQ ID NO: 547 - DNA, 66 bp, Artificial Sequence
  primer
gtgactggagttcagacgtgtgctcttccgatcttgagtcagtctggttactgccagttgaatctg

SEQ ID NO: 548 - DNA, 66 bp, Artificial Sequence
  primer
gtgactggagttcagacgtgtgctcttccgatctgaatgctctctggttactgccagttgaatctg

SEQ ID NO: 549 - DNA, 66 bp, Artificial Sequence
  primer
gtgactggagttcagacgtgtgctcttccgatctgaatatcctctggttactgccagttgaatctg

SEQ ID NO: 550 - DNA, 66 bp, Artificial Sequence
  primer
gtgactggagttcagacgtgtgctcttccgatctcttatgaatctggttactgccagttgaatctg

SEQ ID NO: 551 - DNA, 66 bp, Artificial Sequence
  primer
gtgactggagttcagacgtgtgctcttccgatcttcggcacctctggttactgccagttgaatctg

SEQ ID NO: 552 - DNA, 66 bp, Artificial Sequence
  primer
gtgactggagttcagacgtgtgctcttccgatctaagaagcgtctggttactgccagttgaatctg

SEQ ID NO: 553 - DNA, 66 bp, Artificial Sequence
  primer
gtgactggagttcagacgtgtgctcttccgatctctcacgattctggttactgccagttgaatctg

SEQ ID NO: 554 - DNA, 66 bp, Artificial Sequence
  primer
gtgactggagttcagacgtgtgctcttccgatcttcggtcgatctggttactgccagttgaatctg

SEQ ID NO: 555 - DNA, 66 bp, Artificial Sequence
  primer
gtgactggagttcagacgtgtgctcttccgatcttcggtaagtctggttactgccagttgaatctg

SEQ ID NO: 556 - DNA, 66 bp, Artificial Sequence
  primer
gtgactggagttcagacgtgtgctcttccgatctaagatacatctggttactgccagttgaatctg

SEQ ID NO: 557 - DNA, 66 bp, Artificial Sequence
  primer
gtgactggagttcagacgtgtgctcttccgatctgtcgctgttctggttactgccagttgaatctg

SEQ ID NO: 558 - DNA, 66 bp, Artificial Sequence
  primer
gtgactggagttcagacgtgtgctcttccgatcttcggatgttctggttactgccagttgaatctg

SEQ ID NO: 559 - DNA, 66 bp, Artificial Sequence
  primer
gtgactggagttcagacgtgtgctcttccgatctcgagccggtctggttactgccagttgaatctg

SEQ ID NO: 560 - DNA, 66 bp, Artificial Sequence
  primer
gtgactggagttcagacgtgtgctcttccgatctcgattatctctggttactgccagttgaatctg

SEQ ID NO: 561 - DNA, 66 bp, Artificial Sequence
  primer
gtgactggagttcagacgtgtgctcttccgatcttcgaagcttctggttactgccagttgaatctg

SEQ ID NO: 562 - DNA, 66 bp, Artificial Sequence
  primer
gtgactggagttcagacgtgtgctcttccgatctctatcatttctggttactgccagttgaatctg

SEQ ID NO: 563 - DNA, 66 bp, Artificial Sequence
  primer
gtgactggagttcagacgtgtgctcttccgatctaagttatctctggttactgccagttgaatctg

SEQ ID NO: 564 - DNA, 66 bp, Artificial Sequence
  primer
gtgactggagttcagacgtgtgctcttccgatctcgaacggatctggttactgccagttgaatctg

SEQ ID NO: 565 - DNA, 66 bp, Artificial Sequence
  primer
gtgactggagttcagacgtgtgctcttccgatctctactgactctggttactgccagttgaatctg

SEQ ID NO: 566 - DNA, 66 bp, Artificial Sequence
  primer
gtgactggagttcagacgtgtgctcttccgatcttcttaagttctggttactgccagttgaatctg

SEQ ID NO: 567 - DNA, 66 bp, Artificial Sequence
  primer
gtgactggagttcagacgtgtgctcttccgatctttagagtctctggttactgccagttgaatctg

SEQ ID NO: 568 - DNA, 66 bp, Artificial Sequence
  primer
gtgactggagttcagacgtgtgctcttccgatctaagacgaatctggttactgccagttgaatctg

SEQ ID NO: 569 - DNA, 66 bp, Artificial Sequence
  primer
gtgactggagttcagacgtgtgctcttccgatctttattatgtctggttactgccagttgaatctg

SEQ ID NO: 570 - DNA, 66 bp, Artificial Sequence
  primer
gtgactggagttcagacgtgtgctcttccgatctcgctattatctggttactgccagttgaatctg

SEQ ID NO: 571 - DNA, 66 bp, Artificial Sequence
  primer
gtgactggagttcagacgtgtgctcttccgatcttctatcagtctggttactgccagttgaatctg

SEQ ID NO: 572 - DNA, 66 bp, Artificial Sequence
  primer
gtgactggagttcagacgtgtgctcttccgatctcggtggtatctggttactgccagttgaatctg

SEQ ID NO: 573 - DNA, 66 bp, Artificial Sequence
  primer
gtgactggagttcagacgtgtgctcttccgatcttcaccaattctggttactgccagttgaatctg

SEQ ID NO: 574 - DNA, 66 bp, Artificial Sequence
  primer
gtgactggagttcagacgtgtgctcttccgatctctggaagctctggttactgccagttgaatctg

SEQ ID NO: 575 - DNA, 66 bp, Artificial Sequence
  primer
gtgactggagttcagacgtgtgctcttccgatctcgtaagagtctggttactgccagttgaatctg

SEQ ID NO: 576 - DNA, 66 bp, Artificial Sequence
  primer
gtgactggagttcagacgtgtgctcttccgatctaagagagctctggttactgccagttgaatctg

SEQ ID NO: 577 - DNA, 66 bp, Artificial Sequence
  primer
gtgactggagttcagacgtgtgctcttccgatcttcaacgagtctggttactgccagttgaatctg

SEQ ID NO: 578 - DNA, 66 bp, Artificial Sequence
  primer
gtgactggagttcagacgtgtgctcttccgatcttgcgagactctggttactgccagttgaatctg

SEQ ID NO: 579 - DNA, 66 bp, Artificial Sequence
  primer
gtgactggagttcagacgtgtgctcttccgatctcctggtgttctggttactgccagttgaatctg

SEQ ID NO: 580 - DNA, 66 bp, Artificial Sequence
  primer
gtgactggagttcagacgtgtgctcttccgatctaagtaagttctggttactgccagttgaatctg

SEQ ID NO: 581 - DNA, 66 bp, Artificial Sequence
  primer
gtgactggagttcagacgtgtgctcttccgatcttgactgaatctggttactgccagttgaatctg

SEQ ID NO: 582 - DNA, 66 bp, Artificial Sequence
  primer
gtgactggagttcagacgtgtgctcttccgatctaagactgttctggttactgccagttgaatctg

SEQ ID NO: 583 - DNA, 66 bp, Artificial Sequence
  primer
gtgactggagttcagacgtgtgctcttccgatctcaatgatgtctggttactgccagttgaatctg

SEQ ID NO: 584 - DNA, 66 bp, Artificial Sequence
  primer
gtgactggagttcagacgtgtgctcttccgatctcacagtaatctggttactgccagttgaatctg

SEQ ID NO: 585 - DNA, 66 bp, Artificial Sequence
  primer
gtgactggagttcagacgtgtgctcttccgatcttggtcatttctggttactgccagttgaatctg

SEQ ID NO: 586 - DNA, 66 bp, Artificial Sequence
  primer
gtgactggagttcagacgtgtgctcttccgatctcaaccgtgtctggttactgccagttgaatctg

SEQ ID NO: 587 - DNA, 66 bp, Artificial Sequence
  primer
gtgactggagttcagacgtgtgctcttccgatcttggtgcactctggttactgccagttgaatctg

SEQ ID NO: 588 - DNA, 66 bp, Artificial Sequence
  primer
gtgactggagttcagacgtgtgctcttccgatctccacaatgtctggttactgccagttgaatctg

SEQ ID NO: 589 - DNA, 66 bp, Artificial Sequence
  primer
gtgactggagttcagacgtgtgctcttccgatcttgtgtgcctctggttactgccagttgaatctg

SEQ ID NO: 590 - DNA, 66 bp, Artificial Sequence
  primer
gtgactggagttcagacgtgtgctcttccgatctcaccacggtctggttactgccagttgaatctg

SEQ ID NO: 591 - DNA, 66 bp, Artificial Sequence
  primer
gtgactggagttcagacgtgtgctcttccgatcttgtgttaatctggttactgccagttgaatctg

SEQ ID NO: 592 - DNA, 63 bp, Artificial Sequence
  primer
gtgactggagttcagacgtgtgctcttccgatctagcttggttgtagcacgattgcagcattg

SEQ ID NO: 593 - DNA, 63 bp, Artificial Sequence
  primer
gtgactggagttcagacgtgtgctcttccgatctagcttatgtgtagcacgattgcagcattg

SEQ ID NO: 594 - DNA, 63 bp, Artificial Sequence
  primer
gtgactggagttcagacgtgtgctcttccgatctataacgactgtagcacgattgcagcattg

SEQ ID NO: 595 - DNA, 63 bp, Artificial Sequence
  primer
gtgactggagttcagacgtgtgctcttccgatctgatggagttgtagcacgattgcagcattg

SEQ ID NO: 596 - DNA, 63 bp, Artificial Sequence
  primer
gtgactggagttcagacgtgtgctcttccgatcttgatctaatgtagcacgattgcagcattg

SEQ ID NO: 597 - DNA, 63 bp, Artificial Sequence
  primer
gtgactggagttcagacgtgtgctcttccgatctagctatattgtagcacgattgcagcattg

SEQ ID NO: 598 - DNA, 63 bp, Artificial Sequence
  primer
gtgactggagttcagacgtgtgctcttccgatctagcagagatgtagcacgattgcagcattg

SEQ ID NO: 599 - DNA, 63 bp, Artificial Sequence
  primer
gtgactggagttcagacgtgtgctcttccgatctgacgtaagtgtagcacgattgcagcattg

SEQ ID NO: 600 - DNA, 63 bp, Artificial Sequence
  primer
gtgactggagttcagacgtgtgctcttccgatctaggcctgatgtagcacgattgcagcattg

SEQ ID NO: 601 - DNA, 63 bp, Artificial Sequence
  primer
gtgactggagttcagacgtgtgctcttccgatcttaagattatgtagcacgattgcagcattg

SEQ ID NO: 602 - DNA, 63 bp, Artificial Sequence
  primer
gtgactggagttcagacgtgtgctcttccgatctaggcgaattgtagcacgattgcagcattg

SEQ ID NO: 603 - DNA, 63 bp, Artificial Sequence
  primer
gtgactggagttcagacgtgtgctcttccgatctttgttctttgtagcacgattgcagcattg

SEQ ID NO: 604 - DNA, 63 bp, Artificial Sequence
  primer
gtgactggagttcagacgtgtgctcttccgatcttactcctgtgtagcacgattgcagcattg

SEQ ID NO: 605 - DNA, 63 bp, Artificial Sequence
  primer
gtgactggagttcagacgtgtgctcttccgatctgactggcgtgtagcacgattgcagcattg

SEQ ID NO: 606 - DNA, 63 bp, Artificial Sequence
  primer
gtgactggagttcagacgtgtgctcttccgatctatatatactgtagcacgattgcagcattg

SEQ ID NO: 607 - DNA, 63 bp, Artificial Sequence
  primer
gtgactggagttcagacgtgtgctcttccgatcttagatcggtgtagcacgattgcagcattg

SEQ ID NO: 608 - DNA, 63 bp, Artificial Sequence
  primer
gtgactggagttcagacgtgtgctcttccgatctaggcaagctgtagcacgattgcagcattg

SEQ ID NO: 609 - DNA, 63 bp, Artificial Sequence
  primer
gtgactggagttcagacgtgtgctcttccgatcttccaggtatgtagcacgattgcagcattg

SEQ ID NO: 610 - DNA, 63 bp, Artificial Sequence
  primer
gtgactggagttcagacgtgtgctcttccgatctaggtcaagtgtagcacgattgcagcattg

SEQ ID NO: 611 - DNA, 63 bp, Artificial Sequence
  primer
gtgactggagttcagacgtgtgctcttccgatcttacactggtgtagcacgattgcagcattg

SEQ ID NO: 612 - DNA, 63 bp, Artificial Sequence
  primer
gtgactggagttcagacgtgtgctcttccgatcttccttgcgtgtagcacgattgcagcattg

SEQ ID NO: 613 - DNA, 63 bp, Artificial Sequence
  primer
gtgactggagttcagacgtgtgctcttccgatctaggacctctgtagcacgattgcagcattg

SEQ ID NO: 614 - DNA, 63 bp, Artificial Sequence
  primer
gtgactggagttcagacgtgtgctcttccgatcttaagcatttgtagcacgattgcagcattg

SEQ ID NO: 615 - DNA, 63 bp, Artificial Sequence
  primer
gtgactggagttcagacgtgtgctcttccgatctaggatatttgtagcacgattgcagcattg

SEQ ID NO: 616 - DNA, 63 bp, Artificial Sequence
  primer
gtgactggagttcagacgtgtgctcttccgatctaatcgttatgtagcacgattgcagcattg

SEQ ID NO: 617 - DNA, 63 bp, Artificial Sequence
  primer
gtgactggagttcagacgtgtgctcttccgatctgtctacattgtagcacgattgcagcattg

SEQ ID NO: 618 - DNA, 63 bp, Artificial Sequence
  primer
gtgactggagttcagacgtgtgctcttccgatctcgctgctctgtagcacgattgcagcattg

SEQ ID NO: 619 - DNA, 63 bp, Artificial Sequence
  primer
gtgactggagttcagacgtgtgctcttccgatctgatcaacatgtagcacgattgcagcattg

SEQ ID NO: 620 - DNA, 63 bp, Artificial Sequence
  primer
gtgactggagttcagacgtgtgctcttccgatctcgaaggactgtagcacgattgcagcattg

SEQ ID NO: 621 - DNA, 63 bp, Artificial Sequence
  primer
gtgactggagttcagacgtgtgctcttccgatctgatgccggtgtagcacgattgcagcattg

SEQ ID NO: 622 - DNA, 63 bp, Artificial Sequence
  primer
gtgactggagttcagacgtgtgctcttccgatctctacgaagtgtagcacgattgcagcattg

SEQ ID NO: 623 - DNA, 63 bp, Artificial Sequence
  primer
gtgactggagttcagacgtgtgctcttccgatctgatgcgtctgtagcacgattgcagcattg

SEQ ID NO: 624 - DNA, 63 bp, Artificial Sequence
  primer
gtgactggagttcagacgtgtgctcttccgatctctacggcatgtagcacgattgcagcattg

SEQ ID NO: 625 - DNA, 63 bp, Artificial Sequence
  primer
gtgactggagttcagacgtgtgctcttccgatctgattcctttgtagcacgattgcagcattg

SEQ ID NO: 626 - DNA, 63 bp, Artificial Sequence
  primer
gtgactggagttcagacgtgtgctcttccgatctctactcgatgtagcacgattgcagcattg

SEQ ID NO: 627 - DNA, 63 bp, Artificial Sequence
  primer
gtgactggagttcagacgtgtgctcttccgatctgattcgagtgtagcacgattgcagcattg

SEQ ID NO: 628 - DNA, 63 bp, Artificial Sequence
  primer
gtgactggagttcagacgtgtgctcttccgatctaatcggcgtgtagcacgattgcagcattg

SEQ ID NO: 629 - DNA, 63 bp, Artificial Sequence
  primer
gtgactggagttcagacgtgtgctcttccgatctttcgccgatgtagcacgattgcagcattg

SEQ ID NO: 630 - DNA, 63 bp, Artificial Sequence
  primer
gtgactggagttcagacgtgtgctcttccgatctctggcctctgtagcacgattgcagcattg

SEQ ID NO: 631 - DNA, 63 bp, Artificial Sequence
  primer
gtgactggagttcagacgtgtgctcttccgatctgaacttattgtagcacgattgcagcattg

SEQ ID NO: 632 - DNA, 63 bp, Artificial Sequence
  primer
gtgactggagttcagacgtgtgctcttccgatctcgtattggtgtagcacgattgcagcattg

SEQ ID NO: 633 - DNA, 63 bp, Artificial Sequence
  primer
gtgactggagttcagacgtgtgctcttccgatctgaagcacatgtagcacgattgcagcattg

SEQ ID NO: 634 - DNA, 63 bp, Artificial Sequence
  primer
gtgactggagttcagacgtgtgctcttccgatctcttaatactgtagcacgattgcagcattg

SEQ ID NO: 635 - DNA, 63 bp, Artificial Sequence
  primer
gtgactggagttcagacgtgtgctcttccgatctgaagtctttgtagcacgattgcagcattg

SEQ ID NO: 636 - DNA, 63 bp, Artificial Sequence
  primer
gtgactggagttcagacgtgtgctcttccgatctgaagaggctgtagcacgattgcagcattg

SEQ ID NO: 637 - DNA, 63 bp, Artificial Sequence
  primer
gtgactggagttcagacgtgtgctcttccgatctcggataactgtagcacgattgcagcattg

SEQ ID NO: 638 - DNA, 63 bp, Artificial Sequence
  primer
gtgactggagttcagacgtgtgctcttccgatctgaatctggtgtagcacgattgcagcattg

SEQ ID NO: 639 - DNA, 63 bp, Artificial Sequence
  primer
gtgactggagttcagacgtgtgctcttccgatctctgattgatgtagcacgattgcagcattg

SEQ ID NO: 640 - DNA, 63 bp, Artificial Sequence
  primer
gtgactggagttcagacgtgtgctcttccgatctaatccgtttgtagcacgattgcagcattg

SEQ ID NO: 641 - DNA, 63 bp, Artificial Sequence
  primer
gtgactggagttcagacgtgtgctcttccgatcttgcgtacatgtagcacgattgcagcattg

SEQ ID NO: 642 - DNA, 63 bp, Artificial Sequence
  primer
gtgactggagttcagacgtgtgctcttccgatctgaatcaattgtagcacgattgcagcattg

SEQ ID NO: 643 - DNA, 63 bp, Artificial Sequence
  primer
gtgactggagttcagacgtgtgctcttccgatcttgagtcagtgtagcacgattgcagcattg

SEQ ID NO: 644 - DNA, 63 bp, Artificial Sequence
  primer
gtgactggagttcagacgtgtgctcttccgatctgaatgctctgtagcacgattgcagcattg

SEQ ID NO: 645 - DNA, 63 bp, Artificial Sequence
  primer
gtgactggagttcagacgtgtgctcttccgatctgaatatcctgtagcacgattgcagcattg

SEQ ID NO: 646 - DNA, 63 bp, Artificial Sequence
  primer
gtgactggagttcagacgtgtgctcttccgatctcttatgaatgtagcacgattgcagcattg

SEQ ID NO: 647 - DNA, 63 bp, Artificial Sequence
  primer
gtgactggagttcagacgtgtgctcttccgatcttcggcacctgtagcacgattgcagcattg

SEQ ID NO: 648 - DNA, 63 bp, Artificial Sequence
  primer
gtgactggagttcagacgtgtgctcttccgatctaagaagcgtgtagcacgattgcagcattg

SEQ ID NO: 649 - DNA, 63 bp, Artificial Sequence
  primer
gtgactggagttcagacgtgtgctcttccgatctctcacgattgtagcacgattgcagcattg

SEQ ID NO: 650 - DNA, 63 bp, Artificial Sequence
  primer
gtgactggagttcagacgtgtgctcttccgatcttcggtcgatgtagcacgattgcagcattg

SEQ ID NO: 651 - DNA, 63 bp, Artificial Sequence
  primer
gtgactggagttcagacgtgtgctcttccgatcttcggtaagtgtagcacgattgcagcattg

SEQ ID NO: 652 - DNA, 63 bp, Artificial Sequence
  primer
gtgactggagttcagacgtgtgctcttccgatctaagatacatgtagcacgattgcagcattg

SEQ ID NO: 653 - DNA, 63 bp, Artificial Sequence
  primer
gtgactggagttcagacgtgtgctcttccgatctgtcgctgttgtagcacgattgcagcattg

SEQ ID NO: 654 - DNA, 63 bp, Artificial Sequence
  primer
gtgactggagttcagacgtgtgctcttccgatcttcggatgttgtagcacgattgcagcattg

SEQ ID NO: 655 - DNA, 63 bp, Artificial Sequence
  primer
gtgactggagttcagacgtgtgctcttccgatctcgagccggtgtagcacgattgcagcattg

SEQ ID NO: 656 - DNA, 63 bp, Artificial Sequence
  primer
gtgactggagttcagacgtgtgctcttccgatctcgattatctgtagcacgattgcagcattg

SEQ ID NO: 657 - DNA, 63 bp, Artificial Sequence
  primer
gtgactggagttcagacgtgtgctcttccgatcttcgaagcttgtagcacgattgcagcattg

SEQ ID NO: 658 - DNA, 63 bp, Artificial Sequence
  primer
gtgactggagttcagacgtgtgctcttccgatctctatcatttgtagcacgattgcagcattg

SEQ ID NO: 659 - DNA, 63 bp, Artificial Sequence
  primer
gtgactggagttcagacgtgtgctcttccgatctaagttatctgtagcacgattgcagcattg

SEQ ID NO: 660 - DNA, 63 bp, Artificial Sequence
  primer
gtgactggagttcagacgtgtgctcttccgatctcgaacggatgtagcacgattgcagcattg

SEQ ID NO: 661 - DNA, 63 bp, Artificial Sequence
  primer
gtgactggagttcagacgtgtgctcttccgatctctactgactgtagcacgattgcagcattg

SEQ ID NO: 662 - DNA, 63 bp, Artificial Sequence
  primer
gtgactggagttcagacgtgtgctcttccgatcttcttaagttgtagcacgattgcagcattg

SEQ ID NO: 663 - DNA, 63 bp, Artificial Sequence
  primer
gtgactggagttcagacgtgtgctcttccgatctttagagtctgtagcacgattgcagcattg

SEQ ID NO: 664 - DNA, 63 bp, Artificial Sequence
  primer
gtgactggagttcagacgtgtgctcttccgatctaagacgaatgtagcacgattgcagcattg

SEQ ID NO: 665 - DNA, 63 bp, Artificial Sequence
  primer
gtgactggagttcagacgtgtgctcttccgatctttattatgtgtagcacgattgcagcattg

SEQ ID NO: 666 - DNA, 63 bp, Artificial Sequence
  primer
gtgactggagttcagacgtgtgctcttccgatctcgctattatgtagcacgattgcagcattg

SEQ ID NO: 667 - DNA, 63 bp, Artificial Sequence
  primer
gtgactggagttcagacgtgtgctcttccgatcttctatcagtgtagcacgattgcagcattg

SEQ ID NO: 668 - DNA, 63 bp, Artificial Sequence
  primer
gtgactggagttcagacgtgtgctcttccgatctcggtggtatgtagcacgattgcagcattg

SEQ ID NO: 669 - DNA, 63 bp, Artificial Sequence
  primer
gtgactggagttcagacgtgtgctcttccgatcttcaccaattgtagcacgattgcagcattg

SEQ ID NO: 670 - DNA, 63 bp, Artificial Sequence
  primer
gtgactggagttcagacgtgtgctcttccgatctctggaagctgtagcacgattgcagcattg

SEQ ID NO: 671 - DNA, 63 bp, Artificial Sequence
  primer
gtgactggagttcagacgtgtgctcttccgatctcgtaagagtgtagcacgattgcagcattg

SEQ ID NO: 672 - DNA, 63 bp, Artificial Sequence
  primer
gtgactggagttcagacgtgtgctcttccgatctaagagagctgtagcacgattgcagcattg

SEQ ID NO: 673 - DNA, 63 bp, Artificial Sequence
  primer
gtgactggagttcagacgtgtgctcttccgatcttcaacgagtgtagcacgattgcagcattg

SEQ ID NO: 674 - DNA, 63 bp, Artificial Sequence
  primer
gtgactggagttcagacgtgtgctcttccgatcttgcgagactgtagcacgattgcagcattg

SEQ ID NO: 675 - DNA, 63 bp, Artificial Sequence
  primer
gtgactggagttcagacgtgtgctcttccgatctcctggtgttgtagcacgattgcagcattg

SEQ ID NO: 676 - DNA, 63 bp, Artificial Sequence
  primer
gtgactggagttcagacgtgtgctcttccgatctaagtaagttgtagcacgattgcagcattg

SEQ ID NO: 677 - DNA, 63 bp, Artificial Sequence
  primer
gtgactggagttcagacgtgtgctcttccgatcttgactgaatgtagcacgattgcagcattg

SEQ ID NO: 678 - DNA, 63 bp, Artificial Sequence
  primer
gtgactggagttcagacgtgtgctcttccgatctaagactgttgtagcacgattgcagcattg

SEQ ID NO: 679 - DNA, 63 bp, Artificial Sequence
  primer
gtgactggagttcagacgtgtgctcttccgatctcaatgatgtgtagcacgattgcagcattg

SEQ ID NO: 680 - DNA, 63 bp, Artificial Sequence
  primer
gtgactggagttcagacgtgtgctcttccgatctcacagtaatgtagcacgattgcagcattg

SEQ ID NO: 681 - DNA, 63 bp, Artificial Sequence
  primer
gtgactggagttcagacgtgtgctcttccgatcttggtcatttgtagcacgattgcagcattg

SEQ ID NO: 682 - DNA, 63 bp, Artificial Sequence
  primer
gtgactggagttcagacgtgtgctcttccgatctcaaccgtgtgtagcacgattgcagcattg

SEQ ID NO: 683 - DNA, 63 bp, Artificial Sequence
  primer
gtgactggagttcagacgtgtgctcttccgatcttggtgcactgtagcacgattgcagcattg

SEQ ID NO: 684 - DNA, 63 bp, Artificial Sequence
  primer
gtgactggagttcagacgtgtgctcttccgatctccacaatgtgtagcacgattgcagcattg

SEQ ID NO: 685 - DNA, 63 bp, Artificial Sequence
  primer
gtgactggagttcagacgtgtgctcttccgatcttgtgtgcctgtagcacgattgcagcattg

SEQ ID NO: 686 - DNA, 63 bp, Artificial Sequence
  primer
gtgactggagttcagacgtgtgctcttccgatctcaccacggtgtagcacgattgcagcattg

SEQ ID NO: 687 - DNA, 63 bp, Artificial Sequence
  primer
gtgactggagttcagacgtgtgctcttccgatcttgtgttaatgtagcacgattgcagcattg

SEQ ID NO: 688 - DNA, 64 bp, Artificial Sequence
  primer
gtgactggagttcagacgtgtgctcttccgatctagcttggtggcaaatgctttcgctctggtc

SEQ ID NO: 689 - DNA, 64 bp, Artificial Sequence
  primer
gtgactggagttcagacgtgtgctcttccgatctagcttatgggcaaatgctttcgctctggtc

SEQ ID NO: 690 - DNA, 64 bp, Artificial Sequence
  primer
gtgactggagttcagacgtgtgctcttccgatctataacgacggcaaatgctttcgctctggtc

SEQ ID NO: 691 - DNA, 64 bp, Artificial Sequence
  primer
gtgactggagttcagacgtgtgctcttccgatctgatggagtggcaaatgctttcgctctggtc

SEQ ID NO: 692 - DNA, 64 bp, Artificial Sequence
  primer
gtgactggagttcagacgtgtgctcttccgatcttgatctaaggcaaatgctttcgctctggtc

SEQ ID NO: 693 - DNA, 64 bp, Artificial Sequence
  primer
gtgactggagttcagacgtgtgctcttccgatctagctatatggcaaatgctttcgctctggtc

SEQ ID NO: 694 - DNA, 64 bp, Artificial Sequence
  primer
gtgactggagttcagacgtgtgctcttccgatctagcagagaggcaaatgctttcgctctggtc

SEQ ID NO: 695 - DNA, 64 bp, Artificial Sequence
  primer
gtgactggagttcagacgtgtgctcttccgatctgacgtaagggcaaatgctttcgctctggtc

SEQ ID NO: 696 - DNA, 64 bp, Artificial Sequence
  primer
gtgactggagttcagacgtgtgctcttccgatctaggcctgaggcaaatgctttcgctctggtc

SEQ ID NO: 697 - DNA, 64 bp, Artificial Sequence
  primer
gtgactggagttcagacgtgtgctcttccgatcttaagattaggcaaatgctttcgctctggtc

SEQ ID NO: 698 - DNA, 64 bp, Artificial Sequence
  primer
gtgactggagttcagacgtgtgctcttccgatctaggcgaatggcaaatgctttcgctctggtc

SEQ ID NO: 699 - DNA, 64 bp, Artificial Sequence
  primer
gtgactggagttcagacgtgtgctcttccgatctttgttcttggcaaatgctttcgctctggtc

SEQ ID NO: 700 - DNA, 64 bp, Artificial Sequence
  primer
gtgactggagttcagacgtgtgctcttccgatcttactcctgggcaaatgctttcgctctggtc

SEQ ID NO: 701 - DNA, 64 bp, Artificial Sequence
  primer
gtgactggagttcagacgtgtgctcttccgatctgactggcgggcaaatgctttcgctctggtc

SEQ ID NO: 702 - DNA, 64 bp, Artificial Sequence
  primer
gtgactggagttcagacgtgtgctcttccgatctatatatacggcaaatgctttcgctctggtc

SEQ ID NO: 703 - DNA, 64 bp, Artificial Sequence
  primer
gtgactggagttcagacgtgtgctcttccgatcttagatcggggcaaatgctttcgctctggtc

SEQ ID NO: 704 - DNA, 64 bp, Artificial Sequence
  primer
gtgactggagttcagacgtgtgctcttccgatctaggcaagcggcaaatgctttcgctctggtc

SEQ ID NO: 705 - DNA, 64 bp, Artificial Sequence
  primer
gtgactggagttcagacgtgtgctcttccgatcttccaggtaggcaaatgctttcgctctggtc

SEQ ID NO: 706 - DNA, 64 bp, Artificial Sequence
  primer
gtgactggagttcagacgtgtgctcttccgatctaggtcaagggcaaatgctttcgctctggtc

SEQ ID NO: 707 - DNA, 64 bp, Artificial Sequence
  primer
gtgactggagttcagacgtgtgctcttccgatcttacactggggcaaatgctttcgctctggtc

SEQ ID NO: 708 - DNA, 64 bp, Artificial Sequence
  primer
gtgactggagttcagacgtgtgctcttccgatcttccttgcgggcaaatgctttcgctctggtc

SEQ ID NO: 709 - DNA, 64 bp, Artificial Sequence
  primer
gtgactggagttcagacgtgtgctcttccgatctaggacctcggcaaatgctttcgctctggtc

SEQ ID NO: 710 - DNA, 64 bp, Artificial Sequence
  primer
gtgactggagttcagacgtgtgctcttccgatcttaagcattggcaaatgctttcgctctggtc

SEQ ID NO: 711 - DNA, 64 bp, Artificial Sequence
  primer
gtgactggagttcagacgtgtgctcttccgatctaggatattggcaaatgctttcgctctggtc

SEQ ID NO: 712 - DNA, 64 bp, Artificial Sequence
  primer
gtgactggagttcagacgtgtgctcttccgatctaatcgttaggcaaatgctttcgctctggtc

SEQ ID NO: 713 - DNA, 64 bp, Artificial Sequence
  primer
gtgactggagttcagacgtgtgctcttccgatctgtctacatggcaaatgctttcgctctggtc

SEQ ID NO: 714 - DNA, 64 bp, Artificial Sequence
  primer
gtgactggagttcagacgtgtgctcttccgatctcgctgctcggcaaatgctttcgctctggtc

SEQ ID NO: 715 - DNA, 64 bp, Artificial Sequence
  primer
gtgactggagttcagacgtgtgctcttccgatctgatcaacaggcaaatgctttcgctctggtc

SEQ ID NO: 716 - DNA, 64 bp, Artificial Sequence
  primer
gtgactggagttcagacgtgtgctcttccgatctcgaaggacggcaaatgctttcgctctggtc

SEQ ID NO: 717 - DNA, 64 bp, Artificial Sequence
  primer
gtgactggagttcagacgtgtgctcttccgatctgatgccggggcaaatgctttcgctctggtc

SEQ ID NO: 718 - DNA, 64 bp, Artificial Sequence
  primer
gtgactggagttcagacgtgtgctcttccgatctctacgaagggcaaatgctttcgctctggtc

SEQ ID NO: 719 - DNA, 64 bp, Artificial Sequence
  primer
gtgactggagttcagacgtgtgctcttccgatctgatgcgtcggcaaatgctttcgctctggtc

SEQ ID NO: 720 - DNA, 64 bp, Artificial Sequence
  primer
gtgactggagttcagacgtgtgctcttccgatctctacggcaggcaaatgctttcgctctggtc

SEQ ID NO: 721 - DNA, 64 bp, Artificial Sequence
  primer
gtgactggagttcagacgtgtgctcttccgatctgattccttggcaaatgctttcgctctggtc

SEQ ID NO: 722 - DNA, 64 bp, Artificial Sequence
  primer
gtgactggagttcagacgtgtgctcttccgatctctactcgaggcaaatgctttcgctctggtc

SEQ ID NO: 723 - DNA, 64 bp, Artificial Sequence
  primer
gtgactggagttcagacgtgtgctcttccgatctgattcgagggcaaatgctttcgctctggtc

SEQ ID NO: 724 - DNA, 64 bp, Artificial Sequence
  primer
gtgactggagttcagacgtgtgctcttccgatctaatcggcgggcaaatgctttcgctctggtc

SEQ ID NO: 725 - DNA, 64 bp, Artificial Sequence
  primer
gtgactggagttcagacgtgtgctcttccgatctttcgccgaggcaaatgctttcgctctggtc

SEQ ID NO: 726 - DNA, 64 bp, Artificial Sequence
  primer
gtgactggagttcagacgtgtgctcttccgatctctggcctcggcaaatgctttcgctctggtc

SEQ ID NO: 727 - DNA, 64 bp, Artificial Sequence
  primer
gtgactggagttcagacgtgtgctcttccgatctgaacttatggcaaatgctttcgctctggtc

SEQ ID NO: 728 - DNA, 64 bp, Artificial Sequence
  primer
gtgactggagttcagacgtgtgctcttccgatctcgtattggggcaaatgctttcgctctggtc

SEQ ID NO: 729 - DNA, 64 bp, Artificial Sequence
  primer
gtgactggagttcagacgtgtgctcttccgatctgaagcacaggcaaatgctttcgctctggtc

SEQ ID NO: 730 - DNA, 64 bp, Artificial Sequence
  primer
gtgactggagttcagacgtgtgctcttccgatctcttaatacggcaaatgctttcgctctggtc

SEQ ID NO: 731 - DNA, 64 bp, Artificial Sequence
  primer
gtgactggagttcagacgtgtgctcttccgatctgaagtcttggcaaatgctttcgctctggtc

SEQ ID NO: 732 - DNA, 64 bp, Artificial Sequence
  primer
gtgactggagttcagacgtgtgctcttccgatctgaagaggcggcaaatgctttcgctctggtc

SEQ ID NO: 733 - DNA, 64 bp, Artificial Sequence
  primer
gtgactggagttcagacgtgtgctcttccgatctcggataacggcaaatgctttcgctctggtc

SEQ ID NO: 734 - DNA, 64 bp, Artificial Sequence
  primer
gtgactggagttcagacgtgtgctcttccgatctgaatctggggcaaatgctttcgctctggtc

SEQ ID NO: 735 - DNA, 64 bp, Artificial Sequence
  primer
gtgactggagttcagacgtgtgctcttccgatctctgattgaggcaaatgctttcgctctggtc

SEQ ID NO: 736 - DNA, 64 bp, Artificial Sequence
  primer
gtgactggagttcagacgtgtgctcttccgatctaatccgttggcaaatgctttcgctctggtc

SEQ ID NO: 737 - DNA, 64 bp, Artificial Sequence
  primer
gtgactggagttcagacgtgtgctcttccgatcttgcgtacaggcaaatgctttcgctctggtc

SEQ ID NO: 738 - DNA, 64 bp, Artificial Sequence
  primer
gtgactggagttcagacgtgtgctcttccgatctgaatcaatggcaaatgctttcgctctggtc

SEQ ID NO: 739 - DNA, 64 bp, Artificial Sequence
  primer
gtgactggagttcagacgtgtgctcttccgatcttgagtcagggcaaatgctttcgctctggtc

SEQ ID NO: 740 - DNA, 64 bp, Artificial Sequence
  primer
gtgactggagttcagacgtgtgctcttccgatctgaatgctcggcaaatgctttcgctctggtc

SEQ ID NO: 741 - DNA, 64 bp, Artificial Sequence
  primer
gtgactggagttcagacgtgtgctcttccgatctgaatatccggcaaatgctttcgctctggtc

SEQ ID NO: 742 - DNA, 64 bp, Artificial Sequence
  primer
gtgactggagttcagacgtgtgctcttccgatctcttatgaaggcaaatgctttcgctctggtc

SEQ ID NO: 743 - DNA, 64 bp, Artificial Sequence
  primer
gtgactggagttcagacgtgtgctcttccgatcttcggcaccggcaaatgctttcgctctggtc

SEQ ID NO: 744 - DNA, 64 bp, Artificial Sequence
  primer
gtgactggagttcagacgtgtgctcttccgatctaagaagcgggcaaatgctttcgctctggtc

SEQ ID NO: 745 - DNA, 64 bp, Artificial Sequence
  primer
gtgactggagttcagacgtgtgctcttccgatctctcacgatggcaaatgctttcgctctggtc

SEQ ID NO: 746 - DNA, 64 bp, Artificial Sequence
  primer
gtgactggagttcagacgtgtgctcttccgatcttcggtcgaggcaaatgctttcgctctggtc

SEQ ID NO: 747 - DNA, 64 bp, Artificial Sequence
  primer
gtgactggagttcagacgtgtgctcttccgatcttcggtaagggcaaatgctttcgctctggtc

SEQ ID NO: 748 - DNA, 64 bp, Artificial Sequence
  primer
gtgactggagttcagacgtgtgctcttccgatctaagatacaggcaaatgctttcgctctggtc

SEQ ID NO: 749 - DNA, 64 bp, Artificial Sequence
  primer
gtgactggagttcagacgtgtgctcttccgatctgtcgctgtggcaaatgctttcgctctggtc

SEQ ID NO: 750 - DNA, 64 bp, Artificial Sequence
  primer
gtgactggagttcagacgtgtgctcttccgatcttcggatgtggcaaatgctttcgctctggtc

SEQ ID NO: 751 - DNA, 64 bp, Artificial Sequence
  primer
gtgactggagttcagacgtgtgctcttccgatctcgagccggggcaaatgctttcgctctggtc

SEQ ID NO: 752 - DNA, 64 bp, Artificial Sequence
  primer
gtgactggagttcagacgtgtgctcttccgatctcgattatcggcaaatgctttcgctctggtc

SEQ ID NO: 753 - DNA, 64 bp, Artificial Sequence
  primer
gtgactggagttcagacgtgtgctcttccgatcttcgaagctggcaaatgctttcgctctggtc

SEQ ID NO: 754 - DNA, 64 bp, Artificial Sequence
  primer
gtgactggagttcagacgtgtgctcttccgatctctatcattggcaaatgctttcgctctggtc

SEQ ID NO: 755 - DNA, 64 bp, Artificial Sequence
  primer
gtgactggagttcagacgtgtgctcttccgatctaagttatcggcaaatgctttcgctctggtc

SEQ ID NO: 756 - DNA, 64 bp, Artificial Sequence
  primer
gtgactggagttcagacgtgtgctcttccgatctcgaacggaggcaaatgctttcgctctggtc

SEQ ID NO: 757 - DNA, 64 bp, Artificial Sequence
  primer
gtgactggagttcagacgtgtgctcttccgatctctactgacggcaaatgctttcgctctggtc

SEQ ID NO: 758 - DNA, 64 bp, Artificial Sequence
  primer
gtgactggagttcagacgtgtgctcttccgatcttcttaagtggcaaatgctttcgctctggtc

SEQ ID NO: 759 - DNA, 64 bp, Artificial Sequence
  primer
gtgactggagttcagacgtgtgctcttccgatctttagagtcggcaaatgctttcgctctggtc

SEQ ID NO: 760 - DNA, 64 bp, Artificial Sequence
  primer
gtgactggagttcagacgtgtgctcttccgatctaagacgaaggcaaatgctttcgctctggtc

SEQ ID NO: 761 - DNA, 64 bp, Artificial Sequence
  primer
gtgactggagttcagacgtgtgctcttccgatctttattatgggcaaatgctttcgctctggtc

SEQ ID NO: 762 - DNA, 64 bp, Artificial Sequence
  primer
gtgactggagttcagacgtgtgctcttccgatctcgctattaggcaaatgctttcgctctggtc

SEQ ID NO: 763 - DNA, 64 bp, Artificial Sequence
  primer
gtgactggagttcagacgtgtgctcttccgatcttctatcagggcaaatgctttcgctctggtc

SEQ ID NO: 764 - DNA, 64 bp, Artificial Sequence
  primer
gtgactggagttcagacgtgtgctcttccgatctcggtggtaggcaaatgctttcgctctggtc

SEQ ID NO: 765 - DNA, 64 bp, Artificial Sequence
  primer
gtgactggagttcagacgtgtgctcttccgatcttcaccaatggcaaatgctttcgctctggtc

SEQ ID NO: 766 - DNA, 64 bp, Artificial Sequence
  primer
gtgactggagttcagacgtgtgctcttccgatctctggaagcggcaaatgctttcgctctggtc

SEQ ID NO: 767 - DNA, 64 bp, Artificial Sequence
  primer
gtgactggagttcagacgtgtgctcttccgatctcgtaagagggcaaatgctttcgctctggtc

SEQ ID NO: 768 - DNA, 64 bp, Artificial Sequence
  primer
gtgactggagttcagacgtgtgctcttccgatctaagagagcggcaaatgctttcgctctggtc

SEQ ID NO: 769 - DNA, 64 bp, Artificial Sequence
  primer
gtgactggagttcagacgtgtgctcttccgatcttcaacgagggcaaatgctttcgctctggtc

SEQ ID NO: 770 - DNA, 64 bp, Artificial Sequence
  primer
gtgactggagttcagacgtgtgctcttccgatcttgcgagacggcaaatgctttcgctctggtc

SEQ ID NO: 771 - DNA, 64 bp, Artificial Sequence
  primer
gtgactggagttcagacgtgtgctcttccgatctcctggtgtggcaaatgctttcgctctggtc

SEQ ID NO: 772 - DNA, 64 bp, Artificial Sequence
  primer
gtgactggagttcagacgtgtgctcttccgatctaagtaagtggcaaatgctttcgctctggtc

SEQ ID NO: 773 - DNA, 64 bp, Artificial Sequence
  primer
gtgactggagttcagacgtgtgctcttccgatcttgactgaaggcaaatgctttcgctctggtc

SEQ ID NO: 774 - DNA, 64 bp, Artificial Sequence
  primer
gtgactggagttcagacgtgtgctcttccgatctaagactgtggcaaatgctttcgctctggtc

SEQ ID NO: 775 - DNA, 64 bp, Artificial Sequence
  primer
gtgactggagttcagacgtgtgctcttccgatctcaatgatgggcaaatgctttcgctctggtc

SEQ ID NO: 776 - DNA, 64 bp, Artificial Sequence
  primer
gtgactggagttcagacgtgtgctcttccgatctcacagtaaggcaaatgctttcgctctggtc

SEQ ID NO: 777 - DNA, 64 bp, Artificial Sequence
  primer
gtgactggagttcagacgtgtgctcttccgatcttggtcattggcaaatgctttcgctctggtc

SEQ ID NO: 778 - DNA, 64 bp, Artificial Sequence
  primer
gtgactggagttcagacgtgtgctcttccgatctcaaccgtgggcaaatgctttcgctctggtc

SEQ ID NO: 779 - DNA, 64 bp, Artificial Sequence
  primer
gtgactggagttcagacgtgtgctcttccgatcttggtgcacggcaaatgctttcgctctggtc

SEQ ID NO: 780 - DNA, 64 bp, Artificial Sequence
  primer
gtgactggagttcagacgtgtgctcttccgatctccacaatgggcaaatgctttcgctctggtc

SEQ ID NO: 781 - DNA, 64 bp, Artificial Sequence
  primer
gtgactggagttcagacgtgtgctcttccgatcttgtgtgccggcaaatgctttcgctctggtc

SEQ ID NO: 782 - DNA, 64 bp, Artificial Sequence
  primer
gtgactggagttcagacgtgtgctcttccgatctcaccacggggcaaatgctttcgctctggtc

SEQ ID NO: 783 - DNA, 64 bp, Artificial Sequence
  primer
gtgactggagttcagacgtgtgctcttccgatcttgtgttaaggcaaatgctttcgctctggtc

SEQ ID NO: 784 - DNA, 65 bp, Artificial Sequence
  primer
  misc_feature 51: n is a, c, g, or t
gtgactggagttcagacgtgtgctcttccgatctagcttggttggacaaancgtctacgctgcag

SEQ ID NO: 785 - DNA, 65 bp, Artificial Sequence
  primer
  misc_feature 51: n is a, c, g, or t
gtgactggagttcagacgtgtgctcttccgatctagcttatgtggacaaancgtctacgctgcag

SEQ ID NO: 786 - DNA, 65 bp, Artificial Sequence
  primer
  misc_feature 51: n is a, c, g, or t
gtgactggagttcagacgtgtgctcttccgatctataacgactggacaaancgtctacgctgcag

SEQ ID NO: 787 - DNA, 65 bp, Artificial Sequence
  primer
  misc_feature 51: n is a, c, g, or t
gtgactggagttcagacgtgtgctcttccgatctgatggagttggacaaancgtctacgctgcag

SEQ ID NO: 788 - DNA, 65 bp, Artificial Sequence
  primer
  misc_feature 51: n is a, c, g, or t
gtgactggagttcagacgtgtgctcttccgatcttgatctaatggacaaancgtctacgctgcag

SEQ ID NO: 789 - DNA, 65 bp, Artificial Sequence
  primer
  misc_feature 51: n is a, c, g, or t
gtgactggagttcagacgtgtgctcttccgatctagctatattggacaaancgtctacgctgcag

SEQ ID NO: 790 - DNA, 65 bp, Artificial Sequence
  primer
  misc_feature 51: n is a, c, g, or t
gtgactggagttcagacgtgtgctcttccgatctagcagagatggacaaancgtctacgctgcag

SEQ ID NO: 791 - DNA, 65 bp, Artificial Sequence
  primer
  misc_feature 51: n is a, c, g, or t
gtgactggagttcagacgtgtgctcttccgatctgacgtaagtggacaaancgtctacgctgcag

SEQ ID NO: 792 - DNA, 65 bp, Artificial Sequence
  primer
  misc_feature 51: n is a, c, g, or t
gtgactggagttcagacgtgtgctcttccgatctaggcctgatggacaaancgtctacgctgcag

SEQ ID NO: 793 - DNA, 65 bp, Artificial Sequence
  primer
  misc_feature 51: n is a, c, g, or t
gtgactggagttcagacgtgtgctcttccgatcttaagattatggacaaancgtctacgctgcag

SEQ ID NO: 794 - DNA, 65 bp, Artificial Sequence
  primer
  misc_feature 51: n is a, c, g, or t
gtgactggagttcagacgtgtgctcttccgatctaggcgaattggacaaancgtctacgctgcag

SEQ ID NO: 795 - DNA, 65 bp, Artificial Sequence
  primer
  misc_feature 51: n is a, c, g, or t
gtgactggagttcagacgtgtgctcttccgatctttgttctttggacaaancgtctacgctgcag

SEQ ID NO: 796 - DNA, 65 bp, Artificial Sequence
  primer
  misc_feature 51: n is a, c, g, or t
gtgactggagttcagacgtgtgctcttccgatcttactcctgtggacaaancgtctacgctgcag

SEQ ID NO: 797 - DNA, 65 bp, Artificial Sequence
  primer
  misc_feature 51: n is a, c, g, or t
gtgactggagttcagacgtgtgctcttccgatctgactggcgtggacaaancgtctacgctgcag

SEQ ID NO: 798 - DNA, 65 bp, Artificial Sequence
  primer
  misc_feature 51: n is a, c, g, or t
gtgactggagttcagacgtgtgctcttccgatctatatatactggacaaancgtctacgctgcag

SEQ ID NO: 799 - DNA, 65 bp, Artificial Sequence
  primer
  misc_feature 51: n is a, c, g, or t
gtgactggagttcagacgtgtgctcttccgatcttagatcggtggacaaancgtctacgctgcag

SEQ ID NO: 800 - DNA, 65 bp, Artificial Sequence
  primer
  misc_feature 51: n is a, c, g, or t
gtgactggagttcagacgtgtgctcttccgatctaggcaagctggacaaancgtctacgctgcag

SEQ ID NO: 801 - DNA, 65 bp, Artificial Sequence
  primer
  misc_feature 51: n is a, c, g, or t
gtgactggagttcagacgtgtgctcttccgatcttccaggtatggacaaancgtctacgctgcag

SEQ ID NO: 802 - DNA, 65 bp, Artificial Sequence
  primer
  misc_feature 51: n is a, c, g, or t
gtgactggagttcagacgtgtgctcttccgatctaggtcaagtggacaaancgtctacgctgcag

SEQ ID NO: 803 - DNA, 65 bp, Artificial Sequence
  primer
  misc_feature 51: n is a, c, g, or t
gtgactggagttcagacgtgtgctcttccgatcttacactggtggacaaancgtctacgctgcag

SEQ ID NO: 804 - DNA, 65 bp, Artificial Sequence
  primer
  misc_feature 51: n is a, c, g, or t
gtgactggagttcagacgtgtgctcttccgatcttccttgcgtggacaaancgtctacgctgcag

SEQ ID NO: 805 - DNA, 65 bp, Artificial Sequence
  primer
  misc_feature 51: n is a, c, g, or t
gtgactggagttcagacgtgtgctcttccgatctaggacctctggacaaancgtctacgctgcag

SEQ ID NO: 806 - DNA, 65 bp, Artificial Sequence
  primer
  misc_feature 51: n is a, c, g, or t
gtgactggagttcagacgtgtgctcttccgatcttaagcatttggacaaancgtctacgctgcag

SEQ ID NO: 807 - DNA, 65 bp, Artificial Sequence
  primer
  misc_feature 51: n is a, c, g, or t
gtgactggagttcagacgtgtgctcttccgatctaggatatttggacaaancgtctacgctgcag

SEQ ID NO: 808 - DNA, 65 bp, Artificial Sequence
  primer
  misc_feature 51: n is a, c, g, or t
gtgactggagttcagacgtgtgctcttccgatctaatcgttatggacaaancgtctacgctgcag

SEQ ID NO: 809 - DNA, 65 bp, Artificial Sequence
  primer
  misc_feature 51: n is a, c, g, or t
gtgactggagttcagacgtgtgctcttccgatctgtctacattggacaaancgtctacgctgcag

SEQ ID NO: 810 - DNA, 65 bp, Artificial Sequence
  primer
  misc_feature 51: n is a, c, g, or t
gtgactggagttcagacgtgtgctcttccgatctcgctgctctggacaaancgtctacgctgcag

SEQ ID NO: 811 - DNA, 65 bp, Artificial Sequence
  primer
  misc_feature 51: n is a, c, g, or t
gtgactggagttcagacgtgtgctcttccgatctgatcaacatggacaaancgtctacgctgcag

SEQ ID NO: 812 - DNA, 65 bp, Artificial Sequence
  primer
  misc_feature 51: n is a, c, g, or t
gtgactggagttcagacgtgtgctcttccgatctcgaaggactggacaaancgtctacgctgcag

SEQ ID NO: 813 - DNA, 65 bp, Artificial Sequence
  primer
  misc_feature 51: n is a, c, g, or t
gtgactggagttcagacgtgtgctcttccgatctgatgccggtggacaaancgtctacgctgcag

SEQ ID NO: 814 - DNA, 65 bp, Artificial Sequence
  primer
  misc_feature 51: n is a, c, g, or t
gtgactggagttcagacgtgtgctcttccgatctctacgaagtggacaaancgtctacgctgcag

SEQ ID NO: 815 - DNA, 65 bp, Artificial Sequence
  primer
  misc_feature 51: n is a, c, g, or t
gtgactggagttcagacgtgtgctcttccgatctgatgcgtctggacaaancgtctacgctgcag

SEQ ID NO: 816 - DNA, 65 bp, Artificial Sequence
  primer
  misc_feature 51: n is a, c, g, or t
gtgactggagttcagacgtgtgctcttccgatctctacggcatggacaaancgtctacgctgcag

SEQ ID NO: 817 - DNA, 65 bp, Artificial Sequence
  primer
  misc_feature 51: n is a, c, g, or t
gtgactggagttcagacgtgtgctcttccgatctgattcctttggacaaancgtctacgctgcag

SEQ ID NO: 818 - DNA, 65 bp, Artificial Sequence
  primer
  misc_feature 51: n is a, c, g, or t
gtgactggagttcagacgtgtgctcttccgatctctactcgatggacaaancgtctacgctgcag

SEQ ID NO: 819 - DNA, 65 bp, Artificial Sequence
  primer
  misc_feature 51: n is a, c, g, or t
gtgactggagttcagacgtgtgctcttccgatctgattcgagtggacaaancgtctacgctgcag

SEQ ID NO: 820 - DNA, 65 bp, Artificial Sequence
  primer
  misc_feature 51: n is a, c, g, or t
gtgactggagttcagacgtgtgctcttccgatctaatcggcgtggacaaancgtctacgctgcag

SEQ ID NO: 821 - DNA, 65 bp, Artificial Sequence
  primer
  misc_feature 51: n is a, c, g, or t
gtgactggagttcagacgtgtgctcttccgatctttcgccgatggacaaancgtctacgctgcag

SEQ ID NO: 822 - DNA, 65 bp, Artificial Sequence
  primer
  misc_feature 51: n is a, c, g, or t
gtgactggagttcagacgtgtgctcttccgatctctggcctctggacaaancgtctacgctgcag

SEQ ID NO: 823 - DNA, 65 bp, Artificial Sequence
  primer
  misc_feature 51: n is a, c, g, or t
gtgactggagttcagacgtgtgctcttccgatctgaacttattggacaaancgtctacgctgcag

SEQ ID NO: 824 - DNA, 65 bp, Artificial Sequence
  primer
  misc_feature 51: n is a, c, g, or t
gtgactggagttcagacgtgtgctcttccgatctcgtattggtggacaaancgtctacgctgcag

SEQ ID NO: 825 - DNA, 65 bp, Artificial Sequence
  primer
  misc_feature 51: n is a, c, g, or t
gtgactggagttcagacgtgtgctcttccgatctgaagcacatggacaaancgtctacgctgcag

SEQ ID NO: 826 - DNA, 65 bp, Artificial Sequence
  primer
  misc_feature 51: n is a, c, g, or t
gtgactggagttcagacgtgtgctcttccgatctcttaatactggacaaancgtctacgctgcag

SEQ ID NO: 827 - DNA, 65 bp, Artificial Sequence
  primer
  misc_feature 51: n is a, c, g, or t
gtgactggagttcagacgtgtgctcttccgatctgaagtctttggacaaancgtctacgctgcag

SEQ ID NO: 828 - DNA, 65 bp, Artificial Sequence
  primer
  misc_feature 51: n is a, c, g, or t
gtgactggagttcagacgtgtgctcttccgatctgaagaggctggacaaancgtctacgctgcag

SEQ ID NO: 829 - DNA, 65 bp, Artificial Sequence
  primer
  misc_feature 51: n is a, c, g, or t
gtgactggagttcagacgtgtgctcttccgatctcggataactggacaaancgtctacgctgcag

SEQ ID NO: 830 - DNA, 65 bp, Artificial Sequence
  primer
  misc_feature 51: n is a, c, g, or t
gtgactggagttcagacgtgtgctcttccgatctgaatctggtggacaaancgtctacgctgcag

SEQ ID NO: 831 - DNA, 65 bp, Artificial Sequence
  primer
  misc_feature 51: n is a, c, g, or t
gtgactggagttcagacgtgtgctcttccgatctctgattgatggacaaancgtctacgctgcag

SEQ ID NO: 832 - DNA, 65 bp, Artificial Sequence
  primer
  misc_feature 51: n is a, c, g, or t
gtgactggagttcagacgtgtgctcttccgatctaatccgtttggacaaancgtctacgctgcag

SEQ ID NO: 833 - DNA, 65 bp, Artificial Sequence
  primer
  misc_feature 51: n is a, c, g, or t
gtgactggagttcagacgtgtgctcttccgatcttgcgtacatggacaaancgtctacgctgcag

SEQ ID NO: 834 - DNA, 65 bp, Artificial Sequence
  primer
  misc_feature 51: n is a, c, g, or t
gtgactggagttcagacgtgtgctcttccgatctgaatcaattggacaaancgtctacgctgcag

SEQ ID NO: 835 - DNA, 65 bp, Artificial Sequence
  primer
  misc_feature 51: n is a, c, g, or t
gtgactggagttcagacgtgtgctcttccgatcttgagtcagtggacaaancgtctacgctgcag

SEQ ID NO: 836 - DNA, 65 bp, Artificial Sequence
  primer
  misc_feature 51: n is a, c, g, or t
gtgactggagttcagacgtgtgctcttccgatctgaatgctctggacaaancgtctacgctgcag

SEQ ID NO: 837 - DNA, 65 bp, Artificial Sequence
  primer
  misc_feature 51: n is a, c, g, or t
gtgactggagttcagacgtgtgctcttccgatctgaatatcctggacaaancgtctacgctgcag

SEQ ID NO: 838 - DNA, 65 bp, Artificial Sequence
  primer
  misc_feature 51: n is a, c, g, or t
gtgactggagttcagacgtgtgctcttccgatctcttatgaatggacaaancgtctacgctgcag

SEQ ID NO: 839 - DNA, 65 bp, Artificial Sequence
  primer
  misc_feature 51: n is a, c, g, or t
gtgactggagttcagacgtgtgctcttccgatcttcggcacctggacaaancgtctacgctgcag

SEQ ID NO: 840 - DNA, 65 bp, Artificial Sequence
  primer
  misc_feature 51: n is a, c, g, or t
gtgactggagttcagacgtgtgctcttccgatctaagaagcgtggacaaancgtctacgctgcag

SEQ ID NO: 841 - DNA, 65 bp, Artificial Sequence
  primer
  misc_feature 51: n is a, c, g, or t
gtgactggagttcagacgtgtgctcttccgatctctcacgattggacaaancgtctacgctgcag

SEQ ID NO: 842 - DNA, 65 bp, Artificial Sequence
  primer
  misc_feature 51: n is a, c, g, or t
gtgactggagttcagacgtgtgctcttccgatcttcggtcgatggacaaancgtctacgctgcag

SEQ ID NO: 843 - DNA, 65 bp, Artificial Sequence
  primer
  misc_feature 51: n is a, c, g, or t
gtgactggagttcagacgtgtgctcttccgatcttcggtaagtggacaaancgtctacgctgcag

SEQ ID NO: 844 - DNA, 65 bp, Artificial Sequence
  primer
  misc_feature 51: n is a, c, g, or t
gtgactggagttcagacgtgtgctcttccgatctaagatacatggacaaancgtctacgctgcag

SEQ ID NO: 845 - DNA, 65 bp, Artificial Sequence
  primer
  misc_feature 51: n is a, c, g, or t
gtgactggagttcagacgtgtgctcttccgatctgtcgctgttggacaaancgtctacgctgcag

SEQ ID NO: 846 - DNA, 65 bp, Artificial Sequence
  primer
  misc_feature 51: n is a, c, g, or t
gtgactggagttcagacgtgtgctcttccgatcttcggatgttggacaaancgtctacgctgcag

SEQ ID NO: 847 - DNA, 65 bp, Artificial Sequence
  primer
  misc_feature 51: n is a, c, g, or t
gtgactggagttcagacgtgtgctcttccgatctcgagccggtggacaaancgtctacgctgcag

SEQ ID NO: 848 - DNA, 65 bp, Artificial Sequence
  primer
  misc_feature 51: n is a, c, g, or t
gtgactggagttcagacgtgtgctcttccgatctcgattatctggacaaancgtctacgctgcag

SEQ ID NO: 849 - DNA, 65 bp, Artificial Sequence
  primer
  misc_feature 51: n is a, c, g, or t
gtgactggagttcagacgtgtgctcttccgatcttcgaagcttggacaaancgtctacgctgcag

SEQ ID NO: 850 - DNA, 65 bp, Artificial Sequence
  primer
  misc_feature 51: n is a, c, g, or t
gtgactggagttcagacgtgtgctcttccgatctctatcatttggacaaancgtctacgctgcag

SEQ ID NO: 851 - DNA, 65 bp, Artificial Sequence
  primer
  misc_feature 51: n is a, c, g, or t
gtgactggagttcagacgtgtgctcttccgatctaagttatctggacaaancgtctacgctgcag

SEQ ID NO: 852 - DNA, 65 bp, Artificial Sequence
  primer
  misc_feature 51: n is a, c, g, or t
gtgactggagttcagacgtgtgctcttccgatctcgaacggatggacaaancgtctacgctgcag

SEQ ID NO: 853 - DNA, 65 bp, Artificial Sequence
  primer
  misc_feature 51: n is a, c, g, or t
gtgactggagttcagacgtgtgctcttccgatctctactgactggacaaancgtctacgctgcag

SEQ ID NO: 854 - DNA, 65 bp, Artificial Sequence
  primer
  misc_feature 51: n is a, c, g, or t
gtgactggagttcagacgtgtgctcttccgatcttcttaagttggacaaancgtctacgctgcag

SEQ ID NO: 855 - DNA, 65 bp, Artificial Sequence
  primer
  misc_feature 51: n is a, c, g, or t
gtgactggagttcagacgtgtgctcttccgatctttagagtctggacaaancgtctacgctgcag

SEQ ID NO: 856 - DNA, 65 bp, Artificial Sequence
  primer
  misc_feature 51: n is a, c, g, or t
gtgactggagttcagacgtgtgctcttccgatctaagacgaatggacaaancgtctacgctgcag

SEQ ID NO: 857 - DNA, 65 bp, Artificial Sequence
  primer
  misc_feature 51: n is a, c, g, or t
gtgactggagttcagacgtgtgctcttccgatctttattatgtggacaaancgtctacgctgcag

SEQ ID NO: 858 - DNA, 65 bp, Artificial Sequence
  primer
  misc_feature 51: n is a, c, g, or t
gtgactggagttcagacgtgtgctcttccgatctcgctattatggacaaancgtctacgctgcag

SEQ ID NO: 859 - DNA, 65 bp, Artificial Sequence
  primer
  misc_feature 51: n is a, c, g, or t
gtgactggagttcagacgtgtgctcttccgatcttctatcagtggacaaancgtctacgctgcag

SEQ ID NO: 860 - DNA, 65 bp, Artificial Sequence
  primer
  misc_feature 51: n is a, c, g, or t
gtgactggagttcagacgtgtgctcttccgatctcggtggtatggacaaancgtctacgctgcag

SEQ ID NO: 861 - DNA, 65 bp, Artificial Sequence
  primer
  misc_feature 51: n is a, c, g, or t
gtgactggagttcagacgtgtgctcttccgatcttcaccaattggacaaancgtctacgctgcag

SEQ ID NO: 862 - DNA, 65 bp, Artificial Sequence
  primer
  misc_feature 51: n is a, c, g, or t
gtgactggagttcagacgtgtgctcttccgatctctggaagctggacaaancgtctacgctgcag

SEQ ID NO: 863 - DNA, 65 bp, Artificial Sequence
  primer
  misc_feature 51: n is a, c, g, or t
gtgactggagttcagacgtgtgctcttccgatctcgtaagagtggacaaancgtctacgctgcag

SEQ ID NO: 864 - DNA, 65 bp, Artificial Sequence
  primer
  misc_feature 51: n is a, c, g, or t
gtgactggagttcagacgtgtgctcttccgatctaagagagctggacaaancgtctacgctgcag

SEQ ID NO: 865 - DNA, 65 bp, Artificial Sequence
  primer
  misc_feature 51: n is a, c, g, or t
gtgactggagttcagacgtgtgctcttccgatcttcaacgagtggacaaancgtctacgctgcag

SEQ ID NO: 866 - DNA, 65 bp, Artificial Sequence
  primer
  misc_feature 51: n is a, c, g, or t
gtgactggagttcagacgtgtgctcttccgatcttgcgagactggacaaancgtctacgctgcag

SEQ ID NO: 867 - DNA, 65 bp, Artificial Sequence
  primer
  misc_feature 51: n is a, c, g, or t
gtgactggagttcagacgtgtgctcttccgatctcctggtgttggacaaancgtctacgctgcag

SEQ ID NO: 868 - DNA, 65 bp, Artificial Sequence
  primer
  misc_feature 51: n is a, c, g, or t
gtgactggagttcagacgtgtgctcttccgatctaagtaagttggacaaancgtctacgctgcag

SEQ ID NO: 869 - DNA, 65 bp, Artificial Sequence
  primer
  misc_feature 51: n is a, c, g, or t
gtgactggagttcagacgtgtgctcttccgatcttgactgaatggacaaancgtctacgctgcag

SEQ ID NO: 870 - DNA, 65 bp, Artificial Sequence
  primer
  misc_feature 51: n is a, c, g, or t
gtgactggagttcagacgtgtgctcttccgatctaagactgttggacaaancgtctacgctgcag

SEQ ID NO: 871 - DNA, 65 bp, Artificial Sequence
  primer
  misc_feature 51: n is a, c, g, or t
gtgactggagttcagacgtgtgctcttccgatctcaatgatgtggacaaancgtctacgctgcag

SEQ ID NO: 872 - DNA, 65 bp, Artificial Sequence
  primer
  misc_feature 51: n is a, c, g, or t
gtgactggagttcagacgtgtgctcttccgatctcacagtaatggacaaancgtctacgctgcag

SEQ ID NO: 873 - DNA, 65 bp, Artificial Sequence
  primer
  misc_feature 51: n is a, c, g, or t
gtgactggagttcagacgtgtgctcttccgatcttggtcatttggacaaancgtctacgctgcag

SEQ ID NO: 874 - DNA, 65 bp, Artificial Sequence
  primer
  misc_feature 51: n is a, c, g, or t
gtgactggagttcagacgtgtgctcttccgatctcaaccgtgtggacaaancgtctacgctgcag

SEQ ID NO: 875 - DNA, 65 bp, Artificial Sequence
  primer
  misc_feature 51: n is a, c, g, or t
gtgactggagttcagacgtgtgctcttccgatcttggtgcactggacaaancgtctacgctgcag

SEQ ID NO: 876 - DNA, 65 bp, Artificial Sequence
  primer
  misc_feature 51: n is a, c, g, or t
gtgactggagttcagacgtgtgctcttccgatctccacaatgtggacaaancgtctacgctgcag

SEQ ID NO: 877 - DNA, 65 bp, Artificial Sequence
  primer
  misc_feature 51: n is a, c, g, or t
gtgactggagttcagacgtgtgctcttccgatcttgtgtgcctggacaaancgtctacgctgcag

SEQ ID NO: 878 - DNA, 65 bp, Artificial Sequence
  primer
  misc_feature 51: n is a, c, g, or t
gtgactggagttcagacgtgtgctcttccgatctcaccacggtggacaaancgtctacgctgcag

SEQ ID NO: 879 - DNA, 65 bp, Artificial Sequence
  primer
  misc_feature 51: n is a, c, g, or t
gtgactggagttcagacgtgtgctcttccgatcttgtgttaatggacaaancgtctacgctgcag

SEQ ID NO: 880 - DNA, 60 bp, Artificial Sequence
  primer
gtgactggagttcagacgtgtgctcttccgatctagcttggtgtcgctgtttggagacac

SEQ ID NO: 881 - DNA, 60 bp, Artificial Sequence
  primer
gtgactggagttcagacgtgtgctcttccgatctagcttatggtcgctgtttggagacac

SEQ ID NO: 882 - DNA, 60 bp, Artificial Sequence
  primer
gtgactggagttcagacgtgtgctcttccgatctataacgacgtcgctgtttggagacac

SEQ ID NO: 883 - DNA, 60 bp, Artificial Sequence
  primer
gtgactggagttcagacgtgtgctcttccgatctgatggagtgtcgctgtttggagacac

SEQ ID NO: 884 - DNA, 60 bp, Artificial Sequence
  primer
gtgactggagttcagacgtgtgctcttccgatcttgatctaagtcgctgtttggagacac

SEQ ID NO: 885 - DNA, 60 bp, Artificial Sequence
  primer
gtgactggagttcagacgtgtgctcttccgatctagctatatgtcgctgtttggagacac

SEQ ID NO: 886 - DNA, 60 bp, Artificial Sequence
  primer
gtgactggagttcagacgtgtgctcttccgatctagcagagagtcgctgtttggagacac

SEQ ID NO: 887 - DNA, 60 bp, Artificial Sequence
  primer
gtgactggagttcagacgtgtgctcttccgatctgacgtaaggtcgctgtttggagacac

SEQ ID NO: 888 - DNA, 60 bp, Artificial Sequence
  primer
gtgactggagttcagacgtgtgctcttccgatctaggcctgagtcgctgtttggagacac

SEQ ID NO: 889 - DNA, 60 bp, Artificial Sequence
  primer
gtgactggagttcagacgtgtgctcttccgatcttaagattagtcgctgtttggagacac

SEQ ID NO: 890 - DNA, 60 bp, Artificial Sequence
  primer
gtgactggagttcagacgtgtgctcttccgatctaggcgaatgtcgctgtttggagacac

SEQ ID NO: 891 - DNA, 60 bp, Artificial Sequence
  primer
gtgactggagttcagacgtgtgctcttccgatctttgttcttgtcgctgtttggagacac

SEQ ID NO: 892 - DNA, 60 bp, Artificial Sequence
  primer
gtgactggagttcagacgtgtgctcttccgatcttactcctggtcgctgtttggagacac

SEQ ID NO: 893 - DNA, 60 bp, Artificial Sequence
  primer
gtgactggagttcagacgtgtgctcttccgatctgactggcggtcgctgtttggagacac

SEQ ID NO: 894 - DNA, 60 bp, Artificial Sequence
  primer
gtgactggagttcagacgtgtgctcttccgatctatatatacgtcgctgtttggagacac

SEQ ID NO: 895 - DNA, 60 bp, Artificial Sequence
  primer
gtgactggagttcagacgtgtgctcttccgatcttagatcgggtcgctgtttggagacac

SEQ ID NO: 896 - DNA, 60 bp, Artificial Sequence
  primer
gtgactggagttcagacgtgtgctcttccgatctaggcaagcgtcgctgtttggagacac

SEQ ID NO: 897 - DNA, 60 bp, Artificial Sequence
  primer
gtgactggagttcagacgtgtgctcttccgatcttccaggtagtcgctgtttggagacac

SEQ ID NO: 898 - DNA, 60 bp, Artificial Sequence
  primer
gtgactggagttcagacgtgtgctcttccgatctaggtcaaggtcgctgtttggagacac

SEQ ID NO: 899 - DNA, 60 bp, Artificial Sequence
  primer
gtgactggagttcagacgtgtgctcttccgatcttacactgggtcgctgtttggagacac

SEQ ID NO: 900 - DNA, 60 bp, Artificial Sequence
  primer
gtgactggagttcagacgtgtgctcttccgatcttccttgcggtcgctgtttggagacac

SEQ ID NO: 901 - DNA, 60 bp, Artificial Sequence
  primer
gtgactggagttcagacgtgtgctcttccgatctaggacctcgtcgctgtttggagacac

SEQ ID NO: 902 - DNA, 60 bp, Artificial Sequence
  primer
gtgactggagttcagacgtgtgctcttccgatcttaagcattgtcgctgtttggagacac

SEQ ID NO: 903 - DNA, 60 bp, Artificial Sequence
  primer
gtgactggagttcagacgtgtgctcttccgatctaggatattgtcgctgtttggagacac

SEQ ID NO: 904 - DNA, 60 bp, Artificial Sequence
  primer
gtgactggagttcagacgtgtgctcttccgatctaatcgttagtcgctgtttggagacac

SEQ ID NO: 905 - DNA, 60 bp, Artificial Sequence
  primer
gtgactggagttcagacgtgtgctcttccgatctgtctacatgtcgctgtttggagacac

SEQ ID NO: 906 - DNA, 60 bp, Artificial Sequence
  primer
gtgactggagttcagacgtgtgctcttccgatctcgctgctcgtcgctgtttggagacac

SEQ ID NO: 907 - DNA, 60 bp, Artificial Sequence
  primer
gtgactggagttcagacgtgtgctcttccgatctgatcaacagtcgctgtttggagacac

SEQ ID NO: 908 - DNA, 60 bp, Artificial Sequence
  primer
gtgactggagttcagacgtgtgctcttccgatctcgaaggacgtcgctgtttggagacac

SEQ ID NO: 909 - DNA, 60 bp, Artificial Sequence
  primer
gtgactggagttcagacgtgtgctcttccgatctgatgccgggtcgctgtttggagacac

SEQ ID NO: 910 - DNA, 60 bp, Artificial Sequence
  primer
gtgactggagttcagacgtgtgctcttccgatctctacgaaggtcgctgtttggagacac

SEQ ID NO: 911 - DNA, 60 bp, Artificial Sequence
  primer
gtgactggagttcagacgtgtgctcttccgatctgatgcgtcgtcgctgtttggagacac

SEQ ID NO: 912 - DNA, 60 bp, Artificial Sequence
  primer
gtgactggagttcagacgtgtgctcttccgatctctacggcagtcgctgtttggagacac

SEQ ID NO: 913 - DNA, 60 bp, Artificial Sequence
  primer
gtgactggagttcagacgtgtgctcttccgatctgattccttgtcgctgtttggagacac

SEQ ID NO: 914 - DNA, 60 bp, Artificial Sequence
  primer
gtgactggagttcagacgtgtgctcttccgatctctactcgagtcgctgtttggagacac

SEQ ID NO: 915 - DNA, 60 bp, Artificial Sequence
  primer
gtgactggagttcagacgtgtgctcttccgatctgattcgaggtcgctgtttggagacac

SEQ ID NO: 916 - DNA, 60 bp, Artificial Sequence
  primer
gtgactggagttcagacgtgtgctcttccgatctaatcggcggtcgctgtttggagacac

SEQ ID NO: 917 - DNA, 60 bp, Artificial Sequence
  primer
gtgactggagttcagacgtgtgctcttccgatctttcgccgagtcgctgtttggagacac

SEQ ID NO: 918 - DNA, 60 bp, Artificial Sequence
  primer
gtgactggagttcagacgtgtgctcttccgatctctggcctcgtcgctgtttggagacac

SEQ ID NO: 919 - DNA, 60 bp, Artificial Sequence
  primer
gtgactggagttcagacgtgtgctcttccgatctgaacttatgtcgctgtttggagacac

SEQ ID NO: 920 - DNA, 60 bp, Artificial Sequence
  primer
gtgactggagttcagacgtgtgctcttccgatctcgtattgggtcgctgtttggagacac

SEQ ID NO: 921 - DNA, 60 bp, Artificial Sequence
  primer
gtgactggagttcagacgtgtgctcttccgatctgaagcacagtcgctgtttggagacac

SEQ ID NO: 922 - DNA, 60 bp, Artificial Sequence
  primer
gtgactggagttcagacgtgtgctcttccgatctcttaatacgtcgctgtttggagacac

SEQ ID NO: 923 - DNA, 60 bp, Artificial Sequence
  primer
gtgactggagttcagacgtgtgctcttccgatctgaagtcttgtcgctgtttggagacac

SEQ ID NO: 924 - DNA, 60 bp, Artificial Sequence
  primer
gtgactggagttcagacgtgtgctcttccgatctgaagaggcgtcgctgtttggagacac

SEQ ID NO: 925 - DNA, 60 bp, Artificial Sequence
  primer
gtgactggagttcagacgtgtgctcttccgatctcggataacgtcgctgtttggagacac

SEQ ID NO: 926 - DNA, 60 bp, Artificial Sequence
  primer
gtgactggagttcagacgtgtgctcttccgatctgaatctgggtcgctgtttggagacac

SEQ ID NO: 927 - DNA, 60 bp, Artificial Sequence
  primer
gtgactggagttcagacgtgtgctcttccgatctctgattgagtcgctgtttggagacac

SEQ ID NO: 928 - DNA, 60 bp, Artificial Sequence
  primer
gtgactggagttcagacgtgtgctcttccgatctaatccgttgtcgctgtttggagacac

SEQ ID NO: 929 - DNA, 60 bp, Artificial Sequence
  primer
gtgactggagttcagacgtgtgctcttccgatcttgcgtacagtcgctgtttggagacac

SEQ ID NO: 930 - DNA, 60 bp, Artificial Sequence
  primer
gtgactggagttcagacgtgtgctcttccgatctgaatcaatgtcgctgtttggagacac

SEQ ID NO: 931 - DNA, 60 bp, Artificial Sequence
  primer
gtgactggagttcagacgtgtgctcttccgatcttgagtcaggtcgctgtttggagacac

SEQ ID NO: 932 - DNA, 60 bp, Artificial Sequence
  primer
gtgactggagttcagacgtgtgctcttccgatctgaatgctcgtcgctgtttggagacac

SEQ ID NO: 933 - DNA, 60 bp, Artificial Sequence
  primer
gtgactggagttcagacgtgtgctcttccgatctgaatatccgtcgctgtttggagacac

SEQ ID NO: 934 - DNA, 60 bp, Artificial Sequence
  primer
gtgactggagttcagacgtgtgctcttccgatctcttatgaagtcgctgtttggagacac

SEQ ID NO: 935 - DNA, 60 bp, Artificial Sequence
  primer
gtgactggagttcagacgtgtgctcttccgatcttcggcaccgtcgctgtttggagacac

SEQ ID NO: 936 - DNA, 60 bp, Artificial Sequence
  primer
gtgactggagttcagacgtgtgctcttccgatctaagaagcggtcgctgtttggagacac

SEQ ID NO: 937 - DNA, 60 bp, Artificial Sequence
  primer
gtgactggagttcagacgtgtgctcttccgatctctcacgatgtcgctgtttggagacac

SEQ ID NO: 938 - DNA, 60 bp, Artificial Sequence
  primer
gtgactggagttcagacgtgtgctcttccgatcttcggtcgagtcgctgtttggagacac

SEQ ID NO: 939 - DNA, 60 bp, Artificial Sequence
  primer
gtgactggagttcagacgtgtgctcttccgatcttcggtaaggtcgctgtttggagacac

SEQ ID NO: 940 - DNA, 60 bp, Artificial Sequence
  primer
gtgactggagttcagacgtgtgctcttccgatctaagatacagtcgctgtttggagacac

SEQ ID NO: 941 - DNA, 60 bp, Artificial Sequence
  primer
gtgactggagttcagacgtgtgctcttccgatctgtcgctgtgtcgctgtttggagacac

SEQ ID NO: 942 - DNA, 60 bp, Artificial Sequence
  primer
gtgactggagttcagacgtgtgctcttccgatcttcggatgtgtcgctgtttggagacac

SEQ ID NO: 943 - DNA, 60 bp, Artificial Sequence
  primer
gtgactggagttcagacgtgtgctcttccgatctcgagccgggtcgctgtttggagacac

SEQ ID NO: 944 - DNA, 60 bp, Artificial Sequence
  primer
gtgactggagttcagacgtgtgctcttccgatctcgattatcgtcgctgtttggagacac

SEQ ID NO: 945 - DNA, 60 bp, Artificial Sequence
  primer
gtgactggagttcagacgtgtgctcttccgatcttcgaagctgtcgctgtttggagacac

SEQ ID NO: 946 - DNA, 60 bp, Artificial Sequence
  primer
gtgactggagttcagacgtgtgctcttccgatctctatcattgtcgctgtttggagacac

SEQ ID NO: 947 - DNA, 60 bp, Artificial Sequence
  primer
gtgactggagttcagacgtgtgctcttccgatctaagttatcgtcgctgtttggagacac

SEQ ID NO: 948 - DNA, 60 bp, Artificial Sequence
  primer
gtgactggagttcagacgtgtgctcttccgatctcgaacggagtcgctgtttggagacac

SEQ ID NO: 949 - DNA, 60 bp, Artificial Sequence
  primer
gtgactggagttcagacgtgtgctcttccgatctctactgacgtcgctgtttggagacac

SEQ ID NO: 950 - DNA, 60 bp, Artificial Sequence
  primer
gtgactggagttcagacgtgtgctcttccgatcttcttaagtgtcgctgtttggagacac

SEQ ID NO: 951 - DNA, 60 bp, Artificial Sequence
  primer
gtgactggagttcagacgtgtgctcttccgatctttagagtcgtcgctgtttggagacac

SEQ ID NO: 952 - DNA, 60 bp, Artificial Sequence
  primer
gtgactggagttcagacgtgtgctcttccgatctaagacgaagtcgctgtttggagacac

SEQ ID NO: 953 - DNA, 60 bp, Artificial Sequence
  primer
gtgactggagttcagacgtgtgctcttccgatctttattatggtcgctgtttggagacac

SEQ ID NO: 954 - DNA, 60 bp, Artificial Sequence
  primer
gtgactggagttcagacgtgtgctcttccgatctcgctattagtcgctgtttggagacac

SEQ ID NO: 955 - DNA, 60 bp, Artificial Sequence
  primer
gtgactggagttcagacgtgtgctcttccgatcttctatcaggtcgctgtttggagacac

SEQ ID NO: 956 - DNA, 60 bp, Artificial Sequence
  primer
gtgactggagttcagacgtgtgctcttccgatctcggtggtagtcgctgtttggagacac

SEQ ID NO: 957 - DNA, 60 bp, Artificial Sequence
  primer
gtgactggagttcagacgtgtgctcttccgatcttcaccaatgtcgctgtttggagacac

SEQ ID NO: 958 - DNA, 60 bp, Artificial Sequence
  primer
gtgactggagttcagacgtgtgctcttccgatctctggaagcgtcgctgtttggagacac

SEQ ID NO: 959 - DNA, 60 bp, Artificial Sequence
  primer
gtgactggagttcagacgtgtgctcttccgatctcgtaagaggtcgctgtttggagacac

SEQ ID NO: 960 - DNA, 60 bp, Artificial Sequence
  primer
gtgactggagttcagacgtgtgctcttccgatctaagagagcgtcgctgtttggagacac

SEQ ID NO: 961 - DNA, 60 bp, Artificial Sequence
  primer
gtgactggagttcagacgtgtgctcttccgatcttcaacgaggtcgctgtttggagacac

SEQ ID NO: 962 - DNA, 60 bp, Artificial Sequence
  primer
gtgactggagttcagacgtgtgctcttccgatcttgcgagacgtcgctgtttggagacac

SEQ ID NO: 963 - DNA, 60 bp, Artificial Sequence
  primer
gtgactggagttcagacgtgtgctcttccgatctcctggtgtgtcgctgtttggagacac

SEQ ID NO: 964 - DNA, 60 bp, Artificial Sequence
  primer
gtgactggagttcagacgtgtgctcttccgatctaagtaagtgtcgctgtttggagacac

SEQ ID NO: 965 - DNA, 60 bp, Artificial Sequence
  primer
gtgactggagttcagacgtgtgctcttccgatcttgactgaagtcgctgtttggagacac

SEQ ID NO: 966 - DNA, 60 bp, Artificial Sequence
  primer
gtgactggagttcagacgtgtgctcttccgatctaagactgtgtcgctgtttggagacac

SEQ ID NO: 967 - DNA, 60 bp, Artificial Sequence
  primer
gtgactggagttcagacgtgtgctcttccgatctcaatgatggtcgctgtttggagacac

SEQ ID NO: 968 - DNA, 60 bp, Artificial Sequence
  primer
gtgactggagttcagacgtgtgctcttccgatctcacagtaagtcgctgtttggagacac

SEQ ID NO: 969 - DNA, 60 bp, Artificial Sequence
  primer
gtgactggagttcagacgtgtgctcttccgatcttggtcattgtcgctgtttggagacac

SEQ ID NO: 970 - DNA, 60 bp, Artificial Sequence
  primer
gtgactggagttcagacgtgtgctcttccgatctcaaccgtggtcgctgtttggagacac

SEQ ID NO: 971 - DNA, 60 bp, Artificial Sequence
  primer
gtgactggagttcagacgtgtgctcttccgatcttggtgcacgtcgctgtttggagacac

SEQ ID NO: 972 - DNA, 60 bp, Artificial Sequence
  primer
gtgactggagttcagacgtgtgctcttccgatctccacaatggtcgctgtttggagacac

SEQ ID NO: 973 - DNA, 60 bp, Artificial Sequence
  primer
gtgactggagttcagacgtgtgctcttccgatcttgtgtgccgtcgctgtttggagacac

SEQ ID NO: 974 - DNA, 60 bp, Artificial Sequence
  primer
gtgactggagttcagacgtgtgctcttccgatctcaccacgggtcgctgtttggagacac

SEQ ID NO: 975 - DNA, 60 bp, Artificial Sequence
  primer
gtgactggagttcagacgtgtgctcttccgatcttgtgttaagtcgctgtttggagacac

SEQ ID NO: 976 - DNA, 65 bp, Artificial Sequence
  primer
gtgactggagttcagacgtgtgctcttccgatctagcgctcggaaacacggacacccaaagtagt

SEQ ID NO: 977 - DNA, 65 bp, Artificial Sequence
  primer
gtgactggagttcagacgtgtgctcttccgatcttgcgcttcgaaacacggacacccaaagtagt

SEQ ID NO: 978 - DNA, 65 bp, Artificial Sequence
  primer
gtgactggagttcagacgtgtgctcttccgatctagcttggtgaaacacggacacccaaagtagt

SEQ ID NO: 979 - DNA, 65 bp, Artificial Sequence
  primer
gtgactggagttcagacgtgtgctcttccgatctagcttatggaaacacggacacccaaagtagt

SEQ ID NO: 980 - DNA, 65 bp, Artificial Sequence
  primer
gtgactggagttcagacgtgtgctcttccgatctataacgacgaaacacggacacccaaagtagt

SEQ ID NO: 981 - DNA, 65 bp, Artificial Sequence
  primer
gtgactggagttcagacgtgtgctcttccgatctgatggagtgaaacacggacacccaaagtagt

SEQ ID NO: 982 - DNA, 65 bp, Artificial Sequence
  primer
gtgactggagttcagacgtgtgctcttccgatcttgatctaagaaacacggacacccaaagtagt

SEQ ID NO: 983 - DNA, 65 bp, Artificial Sequence
  primer
gtgactggagttcagacgtgtgctcttccgatctagctatatgaaacacggacacccaaagtagt

SEQ ID NO: 984 - DNA, 65 bp, Artificial Sequence
  primer
gtgactggagttcagacgtgtgctcttccgatctagcagagagaaacacggacacccaaagtagt

SEQ ID NO: 985 - DNA, 65 bp, Artificial Sequence
  primer
gtgactggagttcagacgtgtgctcttccgatctgacgtaaggaaacacggacacccaaagtagt

SEQ ID NO: 986 - DNA, 65 bp, Artificial Sequence
  primer
gtgactggagttcagacgtgtgctcttccgatctaggcctgagaaacacggacacccaaagtagt

SEQ ID NO: 987 - DNA, 65 bp, Artificial Sequence
  primer
gtgactggagttcagacgtgtgctcttccgatcttaagattagaaacacggacacccaaagtagt

SEQ ID NO: 988 - DNA, 65 bp, Artificial Sequence
  primer
gtgactggagttcagacgtgtgctcttccgatctaggcgaatgaaacacggacacccaaagtagt

SEQ ID NO: 989 - DNA, 65 bp, Artificial Sequence
  primer
gtgactggagttcagacgtgtgctcttccgatctttgttcttgaaacacggacacccaaagtagt

SEQ ID NO: 990 - DNA, 65 bp, Artificial Sequence
  primer
gtgactggagttcagacgtgtgctcttccgatcttactcctggaaacacggacacccaaagtagt

SEQ ID NO: 991 - DNA, 22 bp, Artificial Sequence
  part of primer
ctacacgacgctcttccgatct

SEQ ID NO: 992 - DNA, 8 bp, Artificial Sequence
  part of primer
ccaatact

SEQ ID NO: 993 - DNA, 20 bp, Artificial Sequence
  part of primer
gaccccaaaatcagcgaaat

SEQ ID NO: 994 - DNA, 22 bp, Artificial Sequence
  part of primer
gggagccttgaatacaccaaaa

SEQ ID NO: 995 - DNA, 21 bp, Artificial Sequence
  part of primer
ggcattcgtattgcgccgcta

SEQ ID NO: 996 - DNA, 18 bp, Artificial Sequence
  part of primer
ctcatggartggctaaag

SEQ ID NO: 997 - DNA, 17 bp, Artificial Sequence
  part of primer
gccttctccatcttctg

SEQ ID NO: 998 - DNA, 17 bp, Artificial Sequence
  part of primer
tcctccggcccctgaat

SEQ ID NO: 999 - DNA, 34 bp, Artificial Sequence
  part of primer
gtgactggagttcagacgtgtgctcttccgatct

SEQ ID NO: 1000 - DNA, 8 bp, Artificial Sequence
  part of primer
agcttggt

SEQ ID NO: 1001 - DNA, 24 bp, Artificial Sequence
  part of primer
tctggttactgccagttgaatctg

SEQ ID NO: 1002 - DNA, 21 bp, Artificial Sequence
  part of primer
tgtagcacgattgcagcattg

SEQ ID NO: 1003 - DNA, 22 bp, Artificial Sequence
  part of primer
ggcaaatgctttcgctctggtc

SEQ ID NO: 1004 - DNA, 23 bp, Artificial Sequence
  part of primer
  misc_feature (9)..(9): n is a, c, g, or t
tggacaaancgtctacgctgcag

SEQ ID NO: 1005 - DNA, 18 bp, Artificial Sequence
  part of primer
gtcgctgtttggagacac

SEQ ID NO: 1006 - DNA, 23 bp, Artificial Sequence
  part of primer
gaaacacggacacccaaagtagt

SEQ ID NO: 1007 - DNA, 26 bp, Artificial Sequence
  primer part
catgtatagcatggaaccaagtaaca

SEQ ID NO: 1008 - DNA, 28 bp, Artificial Sequence
  primer part
cgttattaacaataagtagggactgggt

SEQ ID NO: 1009 - DNA, 32 bp, Artificial Sequence
  primer part
ccatcaatattcttaaacacaaattccctaag

SEQ ID NO: 1010 - DNA, 21 bp, Artificial Sequence
  primer part
cccacataataagctgcagca

SEQ ID NO: 1011 - DNA, 25 bp, Artificial Sequence
  primer part
ctacagtgaaggatttcaacgtaca

SEQ ID NO: 1012 - DNA, 27 bp, Artificial Sequence
  primer part
gcatagacattagtaaagcagagatca

SEQ ID NO: 1013 - DNA, 27 bp, Artificial Sequence
  primer part
caggtaattataattaccaccaacctt

SEQ ID NO: 1014 - DNA, 28 bp, Artificial Sequence
  primer part
agttcaaaagaaagtactactactctgt

SEQ ID NO: 1015 - DNA, 24 bp, Artificial Sequence
  primer part
ccaaattgttggaaaggcagaaac

SEQ ID NO: 1016 - DNA, 21 bp, Artificial Sequence
  primer part
gcatgaatagcaacagggact

SEQ ID NO: 1017 - DNA, 25 bp, Artificial Sequence
  primer part
gtctgataactagcgcatatacctg

SEQ ID NO: 1018 - DNA, 25 bp, Artificial Sequence
  primer part
gtacaatctactgatgtcttggtca

SEQ ID NO: 1019 - DNA, 23 bp, Artificial Sequence
  primer part
gtgcacaaatgaggtctctagca

SEQ ID NO: 1020 - DNA, 32 bp, Artificial Sequence
  primer part
gagattagacttcctaaacaatctatacaggt

SEQ ID NO: 1021 - DNA, 28 bp, Artificial Sequence
  primer part
ggggtactgctgttatgtctttaaaaga

SEQ ID NO: 1022 - DNA, 27 bp, Artificial Sequence
  primer part
ctgaggatctgaaaactttgtcagggt

SEQ ID NO: 1023 - DNA, 27 bp, Artificial Sequence
  primer part
cccctgcatacactaattctttcacac

SEQ ID NO: 1024 - DNA, 28 bp, Artificial Sequence
  primer part
ctgggtcttcgaatctaaagtagtacca

SEQ ID NO: 1025 - DNA, 32 bp, Artificial Sequence
  primer part
gcttccactgagaagtctaacataataagagg

SEQ ID NO: 1026 - DNA, 22 bp, Artificial Sequence
  primer part
ccctgttttccttcaaggtcca

SEQ ID NO: 1027 - DNA, 25 bp, Artificial Sequence
  primer part
gttggatggaaagtgagttcagagt

SEQ ID NO: 1028 - DNA, 27 bp, Artificial Sequence
  primer part
acctattggcaaatctaccaatggttc

SEQ ID NO: 1029 - DNA, 21 bp, Artificial Sequence
  primer part
gcgtgatctccctcagggttt

SEQ ID NO: 1030 - DNA, 26 bp, Artificial Sequence
  primer part
cgtacactttgtttctgagagagggt

SEQ ID NO: 1031 - DNA, 23 bp, Artificial Sequence
  primer part
cagatgctgtagactgtgcactt

SEQ ID NO: 1032 - DNA, 27 bp, Artificial Sequence
  primer part
cacttaaaagtggaaaatgatgcggaa

SEQ ID NO: 1033 - DNA, 25 bp, Artificial Sequence
  primer part
ggaagagaatcagcaactgtgttgc

SEQ ID NO: 1034 - DNA, 33 bp, Artificial Sequence
  primer part
caccaaccttagaatcaagattgttagaattcc

SEQ ID NO: 1035 - DNA, 23 bp, Artificial Sequence
  primer part
ccagatgattttacaggctgcgt

SEQ ID NO: 1036 - DNA, 31 bp, Artificial Sequence
  primer part
gtactactactctgtatggttggtaaccaac

SEQ ID NO: 1037 - DNA, 28 bp, Artificial Sequence
  primer part
gtctaatctcaaaccttttgagagagat

SEQ ID NO: 1038 - DNA, 24 bp, Artificial Sequence
  primer part
gaacacctgtgcctgttaaaccat

SEQ ID NO: 1039 - DNA, 22 bp, Artificial Sequence
  primer part
gcaccagcaactgtttgtggac

SEQ ID NO: 1040 - DNA, 28 bp, Artificial Sequence
  primer part
cagcaacctggttagaagtatttgttcc

SEQ ID NO: 1041 - DNA, 26 bp, Artificial Sequence
  primer part
cgtgatccacagacacttgagattct

SEQ ID NO: 1042 - DNA, 23 bp, Artificial Sequence
  primer part
cctgcaccaatgggtatgtcaca

SEQ ID NO: 1043 - DNA, 22 bp, Artificial Sequence
  primer part
gcaggctgtttaataggggctg

SEQ ID NO: 1044 - DNA, 29 bp, Artificial Sequence
  primer part
ggtcatagacactggtagaatttctgtgg

SEQ ID NO: 1045 - DNA, 28 bp, Artificial Sequence
  primer part
ggcagtttttgtacacaattaaaccgtg

SEQ ID NO: 1046 - DNA, 24 bp, Artificial Sequence
  primer part
tctagcagcaatatcaccaaggca